European Patent Specification EP 3 655 534 B1, published July 16, 2025. Title: COMPOSITIONS AND METHODS FOR TREATING beta-HEMOGLOBINOPATHIES. Applicant: CALIMMUNE, INC. BARTLETT, Jeffrey S. YAN, Ming AHLERS, Jeffrey Donal SYMONDS, Geoffrey. The sequence listing filed with the application follows.

SEQUENCE LISTING (69 sequences)

SEQ ID NO: 1 - DNA, 46 bp, Artificial Sequence
  Synthetic: shRNA targeting an HPRT gene
aggatatgcccttgactatttgtccgacatagtcaagggcatatcc

SEQ ID NO: 2 - DNA, 46 bp, Artificial Sequence
  Synthetic: shRNA targeting an HPRT gene
tcctatacgggaactgataaacaggctgtatcagttcccgtatagg

SEQ ID NO: 3 - DNA, 444 bp, Artificial Sequence
  Synthetic: sGbGm A gamma-globin translated sequence
atgggtcatttcacagaggaggacaaggctactatcacaagcctgtgggacaaggtgaatgtggaagatgctggaggagaaaccctgggaaggctcctggttgtctacccatggacccagaggttctttgacagctttggcaacctgtcctctgcctctgccatcatgggcaaccccaaagtcaaggcacatggcaagaaggtgctgacttccttgggagatgccataaagcacctggatgatctcaagggcacctttgcccagctgagtgaactgcactgtgacaagctgcatgtggatcctgagaacttcaagctcctgggcaacgtgctggtcaccgtgctggccattcactttggcaaagaattcacccctgaggtgcaggcttcctggcagaagatggtgactgcagtggccagtgccctgtcctccagataccactga

SEQ ID NO: 4 - protein, 147 aa, Artificial Sequence
  Synthetic: sGbGM  HGB1 amino acid sequece
MGHFTEEDKATITSLWDKVNVEDAGGETLGRLLVVYPWTQRFFDSFGNLSSASAIMGNPKVKAHGKKVLTSLGDAIKHLDDLKGTFAQLSELHCDKLHVDPENFKLLGNVLVTVLAIHFGKEFTPEVQASWQKMVTAVASALSSRYH

SEQ ID NO: 5 - DNA, 12088 bp, Artificial Sequence
  Synthetic: TL20c-7SKM1/sh734-rGbGM
ggccgcctcggccaaacagcccttgagtttaccactccctatcagtgatagagaaaagtgaaagtcgagtttaccactccctatcagtgatagagaaaagtgaaagtcgagtttaccactccctatcagtgatagagaaaagtgaaagtcgagtttaccactccctatcagtgatagagaaaagtgaaagtcgagtttaccagtccctatcagtgatagagaaaagtgaaagtcgagtttaccactccctatcagtgatagagaaaagtgaaagtcgagtttaccactccctatcagtgatagagaaaagtgaaagtcgagctcgccatgggaggcgtggcctgggcgggactggggagtggcgagccctcagatcctgcatataagcagctgctttttgcctgtactgggtctctctggttagaccagatctgagcctgggagctctctggctaactagggaacccactgcttaagcctcaataaagcttgccttgagtgcttcaagtagtgtgtgcccgtctgttgtgtgactctggtaactagagatccctcagacccttttagtcagtgtggaaaatctctagcagtggcgcccgaacagggacttgaaagcgaaagggaaaccagaggagctctctcgacgcaggactcggcttgctgaagcgcgcacggcaagaggcgaggggcggcgactggtgagtacgccaaaaattttgactagcggaggctagaaggagagagatgggtgcgagagcgtcagtattaagcgggggagaattagatcgcgatgggaaaaaattcggttaaggccagggggaaagaaaaaatataaattaaaacatatagtatgggcaagcagggagctagaacgattcgcagttaatactggcctgttagaaacatcagaaggctgtagacaaatactgggacagctacaaccatcccttcagacaggatcagaagaacttagatcattatataatacagtagcaaccctctattgtgtgcatcaaaggatagagataaaagacaccaaggaagctttagacaagatagaggaagagcaaaacaaaagtaagaaaaaagcacagcaagcagcaggatcttcagacctggaaattccctacaatccccaaagtcaaggagtagtagaatctatgaataaagaattaaagaaaattataggacaggtaagagatcaggctgaacatcttaagacagcagtacaaatggcagtattcatccacaattttaaaagaaaaggggggattggggggtacagtgcaggggaaagaatagtagacataatagcaacagacatacaaactaaagaattacaaaaacaaattacaaaaattcaaaattttcgggtttattacagggacagcagaaatccactttggaaaggaccagcaaagctcctctggaaaggtgaaggggcagtagtaatacaagataatagtgacataaaagtagtgccaagaagaaaagcaaagatcattagggattatggaaaacagatggcaggtgatgattgtgtggcaagtagacaggatgaggattagaacatggaaaagtttagtaaaacaccataaggaggagatatgagggacaattggagaagtgaattatataaatataaagtagtaaaaattgaaccattaggagtagcacccaccaaggcaaagagaagagtggtgcagagagaaaaaagagcagtgggaataggagctttgttccttgggttcttgggagcagcaggaagcactatgggcgcagcgtcaatgacgctgacggtacaggccagacaattattgtctggtatagtgcagcagcagaacaatttgctgagggctattgaggcgcaacagcatctgttgcaactcacagtctggggcatcaagcagctccaggcaagaatcctggctgtggaaagatacctaaaggatcaacagctcctggggatttggggttgctctggaaaactcatttgcaccactgctgtgccttggaatgctagttggagtaataaatctctggaacagatttggaatcacacgacctggatggagtgggacagagaaattaacaattacacaagcttaatacactccttaattgaagaatcgcaaaaccagcaagaaaagaatgaacaagaattattggaattagataaatgggcaagtttgtggaattggtttaacataacaaattggctgtggtatataaaattattcataatgatagtaggaggcttggtaggtttaagaatagtttttgctgtactttctatagtgaatagagttaggcagggatattcaccattatcgtttcagacccacctcccaaccccgaggggaccgagctcaagcttcgaagcggccgctcgacgtgcagtcgggctactgccccacccatagtaccggcattctggatagtgtcaaaacagccggaaatcaagtccgtttatctcaaactttagcattttgggaataaatgatatttgctatgctggttaaattagattttagttaaatttcctgctgaagctctagtacgataagtaacttgacctaagtgtaaagttgagatttccttcaggtttatatagcttgtgcgccgcctgggtacctcaggatatgcccttgactatttgtccgacatagtcaagggcatatccttttttacgcgtggggatcctctagagtcgagctcgcgaggatcatcaccggtgctagccggagccagaagcaccataagggacatgataagggagccagcagacctctgatctcttcctgaatgctaatcttaaacatcctgaggaagaatgggacttccatttggggtgggcctatgatagggtaataagacagtagtgaatatcaagctacaaaaagccccctttcaaattcttctcagtcctaacttttcatactaagcccagtccttccaaagcagactgtgaaagagtgatagttccgggagactagcaccggctagccgagcttggaacactttcccttcattaagaaccatccttgctactcagctgcaatcaatccagcccccaggtcttcactgaaccttttcccatctcttccaaaacatctgtttctgagaagtcctgtcctatagaggtctttcttcccaccggatttctcctacaccatttactcccacttgcagaactcccgtgtacaagtgtctttactgcttttatttgctcaacaaaatgcacatctcatataaaaataaatgaggagcatgcacacaccacaaacacaaacaggcatgcagaaatacacatacacacttccctcaatataaaccctttgtggctcatatatttaaaaagatgtaaaaaaaagagctgaagaaaatcatgtgtgatctctcagcagaatagatttattatttgtattgcttgcagaataaagcctatccttgaaagctctgaatcatgggcaagaggctcagtggtatctggaggacagggcactggccactgcagtcaccatcttctgccaggaagcctgcacctcaggggtgaattctttgccaaagtgaatggccagcacggtgaccagcacgttgcccaggagctgtgggaggaagataagaggtatgaacatgattagcaaaagggcctagcttggactcagaataatccagccttatcccaaccataaaataaaagcagaatggtagctggattgtagctgctattagcaatatgaaacctcttacatcagttacaatttatatgcagaaatatttatatgcagaaatattgctattgccttaacccagaaattatcactgttattctttagaatggtgcaaagaggcatgatacattgtatcattattgccctgaaagaaagagattagggaaagtattagaaataagataaacaaaaaagtatattaaaagaagaaagcattttttaaaattacaaatgcaaaattaccctgatttggtcaatatgtgtaccctgttacttctccccttcctatgacatgaacttaaccatagaaaagaaggggaaagaaaacatcaagggtcccatagactcaccttgaagttctcaggatccacatgcagcttgtcacagtgcagttcactcagctgggcaaaggtgcccttgagatcatccaggtgctttatggcatctcccaaggaagtcagcaccttcttgccatgtgccttgactttggggttgcccatgatggcagaggcagaggacaggttgccaaagctgtcaaagaacctctgggtccatgggtagacaaccaggagcctgtgagattgacaagaacagtttgacagtcagaaggtgccacaaatcctgagaagcaacctggacttttgccaggcacagggtccttccttccctcccttgtcctggtcaccagagcctaccttcccagggtttctcctccagcatcttccacattcaccttgtcccacaggcttgtgatagtagccttgtcctcctctgtgaaatgacccatggtgtctgtttgaggttgctagtgaacacagttgtgtcagaagcaaatgtaagcaatagatggctctgccctgacttttatgcccagccctggctcctgccctccctgctcctgggagtagattggccaaccctagggtgtggctccacagggtgaggtctaagtgatgacagccgtacctgtccttggctcttctggcactggcttaggagttggacttcaaaccctcagccctccctctaagatatatctcttggccccataccatcagtacaaattgctactaaaaacatcctcctttgcaagtgtatttacgacggtatcgatgtatgtgagcatgtgtcctctaacagcacaggccttttgccacctagctgtccaggggtgccttaaaatggcaaacaaggtttgttttcttttcctgttttcatgccttcctcttccatatccttgtttcatattaatacatgtgtatagatcctaaaaatctatacacatgtattaataaagcctgattctgccgcttctaggtatagaggccacctgcaagataaatatttgattcacaataactaatcattctatggcaattgataacaacaaatatatatatatatatatatatacgtatatgtgtatatatatatatatattcaggaaataatatattctagaatatgtcacattctgtctcaggcatccattttctttatgatgccgtttgaggtggagttttagtcaggtggtcagcttctccttttttttgccatctgccctgtaagcatcctgctggggacccagataggagtcatcactctaggctgagaacatctgggcacacaccctaagcctcagcatgactcatcatgactcagcattgctgtgcttgagccagaaggtttgcttagaaggttacacagaaccagaaggcgggggtggggcactgaccccgacaggggcctggccagaactgctcatgcttggactatgggaggtcactaatggagacacacagaaatgtaacaggaactaagggaattccggtgccctgcttaggagcttaatctttaatgaaagctaagctttcattaaaaaaagtctaaccagctgcattcgactttgactgcagcagctggttagaaggttctactggaggagggtcccagcccattgctaaattaacatcaggctctgagactggcagtatatctctaacagtggttgatgctatcttctggaacttgcctgctacattgagaccactgacccatacataggaagcccatagctctgtcctgaactgttaggccactggtccagagagtgtgcatctcctttgatcctcataataaccctatgagatagacacaattattactcttactttatagatgatgatcctgaaaacataggagtcaaggcacttgcccctagctgggggtataggggagcagtcccatgtagtagtagaatgaaaaatgctgctatgctgtgcctcccccacctttcccatgtctgccctctactcatggtctatctctcctggctcctgggagtcatggactccacccagcaccaccaacctgacctaaccacctatctgagcctgccagcctataacccatctgggccctgatagctggtggccagccctgaccccaccccaccctccctggaacctctgatagacacatctggcacaccagctcgcaaagtcaccgtgagggtcttgtgtttgctgagtcaaaattccttgaaatccaagtccttagagactcctgctcccaaatttacagtcatagacttcttcatggctgtctcctttatccacagaatgattcctttgcttcattgccccatccatctgatcctcctcatcagtgcagcacagggcccatgagcagtagctgcagagtctcacataggtctggcactgcctctgacatgtccgaccttaggcaaatgcttgactcttctgagctcggatcccttgagctcaggaggtcaaggctgcagtgagacatgatcttgccactgcactccagcctggacagcagagtgaaaccttgcctcacgaaacagaatacaaaaacaaacaaacaaaaaactgctccgcaatgcgcttccttgatgctctaccacataggtctgggtactttgtacacattatctcattgctgttcataattgttagattaattttgtaatattgatattattcctagaaagctgaggcctcaagatgataacttttattttctggacttgtaatagctttctcttgtattcaccatgttgtaactttcttagagtagtaacaatataaagttattgtgagtttttgcaaacacagcaaacacaacgacccatatagacattgatgtgaaattgtctattgtcaatttatgggaaaacaagtatgtactttttctactaagccattgaaacaggaataacagaacaagattgaaagaatacattttccgaaattacttgagtattatacaaagacaagcacgtggacctgggaggagggttattgtccatgactggtgtgtggagacaaatgcaggtttataatagatgggatggcatctagcgcaatgactttgccatcacttttagagagctcttgggggccccagtacacaagaggggacgcagggtatatgtagacatctcattctttttcttagtgtgagaataagaatagccatgacctgagtttatagacaatgagcccttttctctctcccactcagcagctatgagatggcttgccctgcctctctactaggctgactcactccaaggcccagcaatgggcagggctctgtcagggctttgatagcactatctgcagagccagggccgagaaggggtggactccagagactctccctcccattcccgagcagggtttgcttatttatgcatttaaatgatatatttattttaaaagaaataacaggagactgcccagccctggctgtgacatggaaactatgtagaatattttgggttccatttttttttccttctttcagttagaggaaaaggggctcactgcacatacactagacagaaagtcaggagctttgaatccaagcctgatcatttccatgtcatactgagaaagtccccacccttctctgagcctcagtttctctttttataagtaggagtctggagtaaatgatttccaatggctctcatttcaatacaaaatttccgtttattaaatgcatgagcttccgttactccaagactgagaaggaaattgaacctgagactcattgactggcaagatgtccccagaggctctcattcagcaataaaattctcaccttcacccaggcccactagtgtcagatttgcatgcgttaacgcggccgcatcgatgccgtagtacctttaagaccaatgacttacaaggcagctgtagatcttagccactttttaaaagaaaaggggggactggaagggctaattcactcccaaagaagacaagatccctgcaggcattcaaggccaggctggatgtggctctgggcagcctgggctgctggttgatgaccctgcacatagcagggggttggatctggatgagcactgtgctcctttgcaacccaggccgttctatgattctgtcattctaaatctctctttcagcctaaagctttttccccgtatccccccaggtgtctgcaggctcaaagagcagcgagaagcgttcagaggaaagcgatcccgtgccaccttccccgtgcccgggctgtccccgcacgctgccggctcggggatgcggggggagcgccggaccggagcggagccccgggcggctcgctgctgccccctagcgggggagggacgtaattacatccctgggggctttgggggggggctgtccccgtgagctccccagatctgctttttgcctgtactgggtctctctggttagaccagatctgagcctgggagctctctggctaactagggaacccactgcttaagcctcaataaagcttcagctgctcgagctagcagatctttttccctctgccaaaaattatggggacatcatgaagccccttgagcatctgacttctggctaataaaggaaatttattttcattgcaatagtgtgttggaattttttgtgtctctcactcggaaggacatatgggagggcaaatcatttaaaacatcagaatgagtatttggtttagagtttggcaacatatgcccatatgctggctgccatgaacaaaggttggctataaagaggtcatcagtatatgaaacagccccctgctgtccattccttattccatagaaaagccttgacttgaggttagattttttttatattttgttttgtgttatttttttctttaacatccctaaaattttccttacatgttttactagccagatttttcctcctctcctgactactcccagtcatagctgtccctcttctcttatggagatccctcgacctgcagcccaagcttggcgtaatcatggtcatagctgtttcctgtgtgaaattgttatccgctcacaattccacacaacatacgagccggaagcataaagtgtaaagcctggggtgcctaatgagtgagctaactcacattaattgcgttgcgctcactgcccgctttccagtcgggaaacctgtcgtgccagcggatccgcatctcaattagtcagcaaccatagtcccgcccctaactccgcccatcccgcccctaactccgcccagttccgcccattctccgccccatggctgactaattttttttatttatgcagaggccgaggccgcctcggcctctgagctattccagaagtagtgaggaggcttttttggaggcctaggcttttgcaaaaagctgtcgactgcagaggcctgcatgcaagcttggcgtaatcatggtcatagctgtttcctgtgtgaaattgttatccgctcacaattccacacaacatacgagccggaagcataaagtgtaaagcctggggtgcctaatgagtgagctaactcacattaattgcgttgcgctcactgcccgctttccagtcgggaaacctgtcgtgccagctgcattaatgaatcggccaacgcgcggggagaggcggtttgcgtattgggcgctcttccgcttcctcgctcactgactcgctgcgctcggtcgttcggctgcggcgagcggtatcagctcactcaaaggcggtaatacggttatccacagaatcaggggataacgcaggaaagaacatgtgagcaaaaggccagcaaaaggccaggaaccgtaaaaaggccgcgttgctggcgtttttccataggctccgcccccctgacgagcatcacaaaaatcgacgctcaagtcagaggtggcgaaacccgacaggactataaagataccaggcgtttccccctggaagctccctcgtgcgctctcctgttccgaccctgccgcttaccggatacctgtccgcctttctcccttcgggaagcgtggcgctttctcatagctcacgctgtaggtatctcagttcggtgtaggtcgttcgctccaagctgggctgtgtgcacgaaccccccgttcagcccgaccgctgcgccttatccggtaactatcgtcttgagtccaacccggtaagacacgacttatcgccactggcagcagccactggtaacaggattagcagagcgaggtatgtaggcggtgctacagagttcttgaagtggtggcctaactacggctacactagaagaacagtatttggtatctgcgctctgctgaagccagttaccttcggaaaaagagttggtagctcttgatccggcaaacaaaccaccgctggtagcggtggtttttttgtttgcaagcagcagattacgcgcagaaaaaaaggatctcaagaagatcctttgatcttttctacggggtctgacgctcagtggaacgaaaactcacgttaagggattttggtcatgagattatcaaaaaggatcttcacctagatccttttaaattaaaaatgaagttttaaatcaatctaaagtatatatgagtaaacttggtctgacagttaccaatgcttaatcagtgaggcacctatctcagcgatctgtctatttcgttcatccatagttgcctgactccccgtcgtgtagataactacgatacgggagggcttaccatctggccccagtgctgcaatgataccgcgagacccacgctcaccggctccagatttatcagcaataaaccagccagccggaagggccgagcgcagaagtggtcctgcaactttatccgcctccatccagtctattaattgttgccgggaagctagagtaagtagttcgccagttaatagtttgcgcaacgttgttgccattgctacaggcatcgtggtgtcacgctcgtcgtttggtatggcttcattcagctccggttcccaacgatcaaggcgagttacatgatcccccatgttgtgcaaaaaagcggttagctccttcggtcctccgatcgttgtcagaagtaagttggccgcagtgttatcactcatggttatggcagcactgcataattctcttactgtcatgccatccgtaagatgcttttctgtgactggtgagtactcaaccaagtcattctgagaatagtgtatgcggcgaccgagttgctcttgcccggcgtcaatacgggataataccgcgccacatagcagaactttaaaagtgctcatcattggaaaacgttcttcggggcgaaaactctcaaggatcttaccgctgttgagatccagttcgatgtaacccactcgtgcacccaactgatcttcagcatcttttactttcaccagcgtttctgggtgagcaaaaacaggaaggcaaaatgccgcaaaaaagggaataagggcgacacggaaatgttgaatactcatactcttcctttttcaatattattgaagcatttatcagggttattgtctcatgagcggatacatatttgaatgtatttagaaaaataaacaaataggggttccgcgcacatttccccgaaaagtgccacctgacgtctaagaaaccattattatcatgacattaacctataaaaataggcgtatcacgaggccctttcgtctcgcgcgtttcggtgatgacggtgaaaacctctgacacatgcagctcccggagacggtcacagcttgtctgtaagcggatgccgggagcagacaagcccgtcagggcgcgtcagcgggtgttggcgggtgtcggggctggcttaactatgcggcatcagagcagattgtactgagagtgcaccatatgcggtgtgaaataccgcacagatgcgtaaggagaaaataccgcatcaggcgccattcgccattcaggctgcgcaactgttgggaagggcgatcggtgcgggcctcttcgctattacgccagctggcgaaagggggatgtgctgcaaggcgattaagttgggtaacgccagggttttcccagtcacgacgttgtaaaacgacggccagtgaattc

SEQ ID NO: 6 - DNA, 12091 bp, Artificial Sequence
  Synthetic: TL20c-7SK/sh734-rGbGM
ggccgcctcggccaaacagcccttgagtttaccactccctatcagtgatagagaaaagtgaaagtcgagtttaccactccctatcagtgatagagaaaagtgaaagtcgagtttaccactccctatcagtgatagagaaaagtgaaagtcgagtttaccactccctatcagtgatagagaaaagtgaaagtcgagtttaccagtccctatcagtgatagagaaaagtgaaagtcgagtttaccactccctatcagtgatagagaaaagtgaaagtcgagtttaccactccctatcagtgatagagaaaagtgaaagtcgagctcgccatgggaggcgtggcctgggcgggactggggagtggcgagccctcagatcctgcatataagcagctgctttttgcctgtactgggtctctctggttagaccagatctgagcctgggagctctctggctaactagggaacccactgcttaagcctcaataaagcttgccttgagtgcttcaagtagtgtgtgcccgtctgttgtgtgactctggtaactagagatccctcagacccttttagtcagtgtggaaaatctctagcagtggcgcccgaacagggacttgaaagcgaaagggaaaccagaggagctctctcgacgcaggactcggcttgctgaagcgcgcacggcaagaggcgaggggcggcgactggtgagtacgccaaaaattttgactagcggaggctagaaggagagagatgggtgcgagagcgtcagtattaagcgggggagaattagatcgcgatgggaaaaaattcggttaaggccagggggaaagaaaaaatataaattaaaacatatagtatgggcaagcagggagctagaacgattcgcagttaatactggcctgttagaaacatcagaaggctgtagacaaatactgggacagctacaaccatcccttcagacaggatcagaagaacttagatcattatataatacagtagcaaccctctattgtgtgcatcaaaggatagagataaaagacaccaaggaagctttagacaagatagaggaagagcaaaacaaaagtaagaaaaaagcacagcaagcagcaggatcttcagacctggaaattccctacaatccccaaagtcaaggagtagtagaatctatgaataaagaattaaagaaaattataggacaggtaagagatcaggctgaacatcttaagacagcagtacaaatggcagtattcatccacaattttaaaagaaaaggggggattggggggtacagtgcaggggaaagaatagtagacataatagcaacagacatacaaactaaagaattacaaaaacaaattacaaaaattcaaaattttcgggtttattacagggacagcagaaatccactttggaaaggaccagcaaagctcctctggaaaggtgaaggggcagtagtaatacaagataatagtgacataaaagtagtgccaagaagaaaagcaaagatcattagggattatggaaaacagatggcaggtgatgattgtgtggcaagtagacaggatgaggattagaacatggaaaagtttagtaaaacaccataaggaggagatatgagggacaattggagaagtgaattatataaatataaagtagtaaaaattgaaccattaggagtagcacccaccaaggcaaagagaagagtggtgcagagagaaaaaagagcagtgggaataggagctttgttccttgggttcttgggagcagcaggaagcactatgggcgcagcgtcaatgacgctgacggtacaggccagacaattattgtctggtatagtgcagcagcagaacaatttgctgagggctattgaggcgcaacagcatctgttgcaactcacagtctggggcatcaagcagctccaggcaagaatcctggctgtggaaagatacctaaaggatcaacagctcctggggatttggggttgctctggaaaactcatttgcaccactgctgtgccttggaatgctagttggagtaataaatctctggaacagatttggaatcacacgacctggatggagtgggacagagaaattaacaattacacaagcttaatacactccttaattgaagaatcgcaaaaccagcaagaaaagaatgaacaagaattattggaattagataaatgggcaagtttgtggaattggtttaacataacaaattggctgtggtatataaaattattcataatgatagtaggaggcttggtaggtttaagaatagtttttgctgtactttctatagtgaatagagttaggcagggatattcaccattatcgtttcagacccacctcccaaccccgaggggaccgagctcaagcttcgaagcggccgcatcgacgtgcagtatttagcatgccccacccatctgcaaggcattctggatagtgtcaaaacagccggaaatcaagtccgtttatctcaaactttagcattttgggaataaatgatatttgctatgctggttaaattagattttagttaaatttcctgctgaagctctagtacgataagtaacttgacctaagtgtaaagttgagatttccttcaggtttatatagcttgtgcgccgcctgggtacctcaggatatgcccttgactatttgtccgacatagtcaagggcatatccttttttgtacgcgtggggatcctctagagtcgagctcgcgaggatcatcaccggtgctagccggagccagaagcaccataagggacatgataagggagccagcagacctctgatctcttcctgaatgctaatcttaaacatcctgaggaagaatgggacttccatttggggtgggcctatgatagggtaataagacagtagtgaatatcaagctacaaaaagccccctttcaaattcttctcagtcctaacttttcatactaagcccagtccttccaaagcagactgtgaaagagtgatagttccgggagactagcaccggctagccgagcttggaacactttcccttcattaagaaccatccttgctactcagctgcaatcaatccagcccccaggtcttcactgaaccttttcccatctcttccaaaacatctgtttctgagaagtcctgtcctatagaggtctttcttcccaccggatttctcctacaccatttactcccacttgcagaactcccgtgtacaagtgtctttactgcttttatttgctcaacaaaatgcacatctcatataaaaataaatgaggagcatgcacacaccacaaacacaaacaggcatgcagaaatacacatacacacttccctcaatataaaccctttgtggctcatatatttaaaaagatgtaaaaaaaagagctgaagaaaatcatgtgtgatctctcagcagaatagatttattatttgtattgcttgcagaataaagcctatccttgaaagctctgaatcatgggcaagaggctcagtggtatctggaggacagggcactggccactgcagtcaccatcttctgccaggaagcctgcacctcaggggtgaattctttgccaaagtgaatggccagcacggtgaccagcacgttgcccaggagctgtgggaggaagataagaggtatgaacatgattagcaaaagggcctagcttggactcagaataatccagccttatcccaaccataaaataaaagcagaatggtagctggattgtagctgctattagcaatatgaaacctcttacatcagttacaatttatatgcagaaatatttatatgcagaaatattgctattgccttaacccagaaattatcactgttattctttagaatggtgcaaagaggcatgatacattgtatcattattgccctgaaagaaagagattagggaaagtattagaaataagataaacaaaaaagtatattaaaagaagaaagcattttttaaaattacaaatgcaaaattaccctgatttggtcaatatgtgtaccctgttacttctccccttcctatgacatgaacttaaccatagaaaagaaggggaaagaaaacatcaagggtcccatagactcaccttgaagttctcaggatccacatgcagcttgtcacagtgcagttcactcagctgggcaaaggtgcccttgagatcatccaggtgctttatggcatctcccaaggaagtcagcaccttcttgccatgtgccttgactttggggttgcccatgatggcagaggcagaggacaggttgccaaagctgtcaaagaacctctgggtccatgggtagacaaccaggagcctgtgagattgacaagaacagtttgacagtcagaaggtgccacaaatcctgagaagcaacctggacttttgccaggcacagggtccttccttccctcccttgtcctggtcaccagagcctaccttcccagggtttctcctccagcatcttccacattcaccttgtcccacaggcttgtgatagtagccttgtcctcctctgtgaaatgacccatggtgtctgtttgaggttgctagtgaacacagttgtgtcagaagcaaatgtaagcaatagatggctctgccctgacttttatgcccagccctggctcctgccctccctgctcctgggagtagattggccaaccctagggtgtggctccacagggtgaggtctaagtgatgacagccgtacctgtccttggctcttctggcactggcttaggagttggacttcaaaccctcagccctccctctaagatatatctcttggccccataccatcagtacaaattgctactaaaaacatcctcctttgcaagtgtatttacgacggtatcgatgtatgtgagcatgtgtcctctaacagcacaggccttttgccacctagctgtccaggggtgccttaaaatggcaaacaaggtttgttttcttttcctgttttcatgccttcctcttccatatccttgtttcatattaatacatgtgtatagatcctaaaaatctatacacatgtattaataaagcctgattctgccgcttctaggtatagaggccacctgcaagataaatatttgattcacaataactaatcattctatggcaattgataacaacaaatatatatatatatatatatatacgtatatgtgtatatatatatatatattcaggaaataatatattctagaatatgtcacattctgtctcaggcatccattttctttatgatgccgtttgaggtggagttttagtcaggtggtcagcttctccttttttttgccatctgccctgtaagcatcctgctggggacccagataggagtcatcactctaggctgagaacatctgggcacacaccctaagcctcagcatgactcatcatgactcagcattgctgtgcttgagccagaaggtttgcttagaaggttacacagaaccagaaggcgggggtggggcactgaccccgacaggggcctggccagaactgctcatgcttggactatgggaggtcactaatggagacacacagaaatgtaacaggaactaagggaattccggtgccctgcttaggagcttaatctttaatgaaagctaagctttcattaaaaaaagtctaaccagctgcattcgactttgactgcagcagctggttagaaggttctactggaggagggtcccagcccattgctaaattaacatcaggctctgagactggcagtatatctctaacagtggttgatgctatcttctggaacttgcctgctacattgagaccactgacccatacataggaagcccatagctctgtcctgaactgttaggccactggtccagagagtgtgcatctcctttgatcctcataataaccctatgagatagacacaattattactcttactttatagatgatgatcctgaaaacataggagtcaaggcacttgcccctagctgggggtataggggagcagtcccatgtagtagtagaatgaaaaatgctgctatgctgtgcctcccccacctttcccatgtctgccctctactcatggtctatctctcctggctcctgggagtcatggactccacccagcaccaccaacctgacctaaccacctatctgagcctgccagcctataacccatctgggccctgatagctggtggccagccctgaccccaccccaccctccctggaacctctgatagacacatctggcacaccagctcgcaaagtcaccgtgagggtcttgtgtttgctgagtcaaaattccttgaaatccaagtccttagagactcctgctcccaaatttacagtcatagacttcttcatggctgtctcctttatccacagaatgattcctttgcttcattgccccatccatctgatcctcctcatcagtgcagcacagggcccatgagcagtagctgcagagtctcacataggtctggcactgcctctgacatgtccgaccttaggcaaatgcttgactcttctgagctcggatcccttgagctcaggaggtcaaggctgcagtgagacatgatcttgccactgcactccagcctggacagcagagtgaaaccttgcctcacgaaacagaatacaaaaacaaacaaacaaaaaactgctccgcaatgcgcttccttgatgctctaccacataggtctgggtactttgtacacattatctcattgctgttcataattgttagattaattttgtaatattgatattattcctagaaagctgaggcctcaagatgataacttttattttctggacttgtaatagctttctcttgtattcaccatgttgtaactttcttagagtagtaacaatataaagttattgtgagtttttgcaaacacagcaaacacaacgacccatatagacattgatgtgaaattgtctattgtcaatttatgggaaaacaagtatgtactttttctactaagccattgaaacaggaataacagaacaagattgaaagaatacattttccgaaattacttgagtattatacaaagacaagcacgtggacctgggaggagggttattgtccatgactggtgtgtggagacaaatgcaggtttataatagatgggatggcatctagcgcaatgactttgccatcacttttagagagctcttgggggccccagtacacaagaggggacgcagggtatatgtagacatctcattctttttcttagtgtgagaataagaatagccatgacctgagtttatagacaatgagcccttttctctctcccactcagcagctatgagatggcttgccctgcctctctactaggctgactcactccaaggcccagcaatgggcagggctctgtcagggctttgatagcactatctgcagagccagggccgagaaggggtggactccagagactctccctcccattcccgagcagggtttgcttatttatgcatttaaatgatatatttattttaaaagaaataacaggagactgcccagccctggctgtgacatggaaactatgtagaatattttgggttccatttttttttccttctttcagttagaggaaaaggggctcactgcacatacactagacagaaagtcaggagctttgaatccaagcctgatcatttccatgtcatactgagaaagtccccacccttctctgagcctcagtttctctttttataagtaggagtctggagtaaatgatttccaatggctctcatttcaatacaaaatttccgtttattaaatgcatgagcttccgttactccaagactgagaaggaaattgaacctgagactcattgactggcaagatgtccccagaggctctcattcagcaataaaattctcaccttcacccaggcccactagtgtcagatttgcatgcgttaacgcggccgcatcgatgccgtagtacctttaagaccaatgacttacaaggcagctgtagatcttagccactttttaaaagaaaaggggggactggaagggctaattcactcccaaagaagacaagatccctgcaggcattcaaggccaggctggatgtggctctgggcagcctgggctgctggttgatgaccctgcacatagcagggggttggatctggatgagcactgtgctcctttgcaacccaggccgttctatgattctgtcattctaaatctctctttcagcctaaagctttttccccgtatccccccaggtgtctgcaggctcaaagagcagcgagaagcgttcagaggaaagcgatcccgtgccaccttccccgtgcccgggctgtccccgcacgctgccggctcggggatgcggggggagcgccggaccggagcggagccccgggcggctcgctgctgccccctagcgggggagggacgtaattacatccctgggggctttgggggggggctgtccccgtgagctccccagatctgctttttgcctgtactgggtctctctggttagaccagatctgagcctgggagctctctggctaactagggaacccactgcttaagcctcaataaagcttcagctgctcgagctagcagatctttttccctctgccaaaaattatggggacatcatgaagccccttgagcatctgacttctggctaataaaggaaatttattttcattgcaatagtgtgttggaattttttgtgtctctcactcggaaggacatatgggagggcaaatcatttaaaacatcagaatgagtatttggtttagagtttggcaacatatgcccatatgctggctgccatgaacaaaggttggctataaagaggtcatcagtatatgaaacagccccctgctgtccattccttattccatagaaaagccttgacttgaggttagattttttttatattttgttttgtgttatttttttctttaacatccctaaaattttccttacatgttttactagccagatttttcctcctctcctgactactcccagtcatagctgtccctcttctcttatggagatccctcgacctgcagcccaagcttggcgtaatcatggtcatagctgtttcctgtgtgaaattgttatccgctcacaattccacacaacatacgagccggaagcataaagtgtaaagcctggggtgcctaatgagtgagctaactcacattaattgcgttgcgctcactgcccgctttccagtcgggaaacctgtcgtgccagcggatccgcatctcaattagtcagcaaccatagtcccgcccctaactccgcccatcccgcccctaactccgcccagttccgcccattctccgccccatggctgactaattttttttatttatgcagaggccgaggccgcctcggcctctgagctattccagaagtagtgaggaggcttttttggaggcctaggcttttgcaaaaagctgtcgactgcagaggcctgcatgcaagcttggcgtaatcatggtcatagctgtttcctgtgtgaaattgttatccgctcacaattccacacaacatacgagccggaagcataaagtgtaaagcctggggtgcctaatgagtgagctaactcacattaattgcgttgcgctcactgcccgctttccagtcgggaaacctgtcgtgccagctgcattaatgaatcggccaacgcgcggggagaggcggtttgcgtattgggcgctcttccgcttcctcgctcactgactcgctgcgctcggtcgttcggctgcggcgagcggtatcagctcactcaaaggcggtaatacggttatccacagaatcaggggataacgcaggaaagaacatgtgagcaaaaggccagcaaaaggccaggaaccgtaaaaaggccgcgttgctggcgtttttccataggctccgcccccctgacgagcatcacaaaaatcgacgctcaagtcagaggtggcgaaacccgacaggactataaagataccaggcgtttccccctggaagctccctcgtgcgctctcctgttccgaccctgccgcttaccggatacctgtccgcctttctcccttcgggaagcgtggcgctttctcatagctcacgctgtaggtatctcagttcggtgtaggtcgttcgctccaagctgggctgtgtgcacgaaccccccgttcagcccgaccgctgcgccttatccggtaactatcgtcttgagtccaacccggtaagacacgacttatcgccactggcagcagccactggtaacaggattagcagagcgaggtatgtaggcggtgctacagagttcttgaagtggtggcctaactacggctacactagaagaacagtatttggtatctgcgctctgctgaagccagttaccttcggaaaaagagttggtagctcttgatccggcaaacaaaccaccgctggtagcggtggtttttttgtttgcaagcagcagattacgcgcagaaaaaaaggatctcaagaagatcctttgatcttttctacggggtctgacgctcagtggaacgaaaactcacgttaagggattttggtcatgagattatcaaaaaggatcttcacctagatccttttaaattaaaaatgaagttttaaatcaatctaaagtatatatgagtaaacttggtctgacagttaccaatgcttaatcagtgaggcacctatctcagcgatctgtctatttcgttcatccatagttgcctgactccccgtcgtgtagataactacgatacgggagggcttaccatctggccccagtgctgcaatgataccgcgagacccacgctcaccggctccagatttatcagcaataaaccagccagccggaagggccgagcgcagaagtggtcctgcaactttatccgcctccatccagtctattaattgttgccgggaagctagagtaagtagttcgccagttaatagtttgcgcaacgttgttgccattgctacaggcatcgtggtgtcacgctcgtcgtttggtatggcttcattcagctccggttcccaacgatcaaggcgagttacatgatcccccatgttgtgcaaaaaagcggttagctccttcggtcctccgatcgttgtcagaagtaagttggccgcagtgttatcactcatggttatggcagcactgcataattctcttactgtcatgccatccgtaagatgcttttctgtgactggtgagtactcaaccaagtcattctgagaatagtgtatgcggcgaccgagttgctcttgcccggcgtcaatacgggataataccgcgccacatagcagaactttaaaagtgctcatcattggaaaacgttcttcggggcgaaaactctcaaggatcttaccgctgttgagatccagttcgatgtaacccactcgtgcacccaactgatcttcagcatcttttactttcaccagcgtttctgggtgagcaaaaacaggaaggcaaaatgccgcaaaaaagggaataagggcgacacggaaatgttgaatactcatactcttcctttttcaatattattgaagcatttatcagggttattgtctcatgagcggatacatatttgaatgtatttagaaaaataaacaaataggggttccgcgcacatttccccgaaaagtgccacctgacgtctaagaaaccattattatcatgacattaacctataaaaataggcgtatcacgaggccctttcgtctcgcgcgtttcggtgatgacggtgaaaacctctgacacatgcagctcccggagacggtcacagcttgtctgtaagcggatgccgggagcagacaagcccgtcagggcgcgtcagcgggtgttggcgggtgtcggggctggcttaactatgcggcatcagagcagattgtactgagagtgcaccatatgcggtgtgaaataccgcacagatgcgtaaggagaaaataccgcatcaggcgccattcgccattcaggctgcgcaactgttgggaagggcgatcggtgcgggcctcttcgctattacgccagctggcgaaagggggatgtgctgcaaggcgattaagttgggtaacgccagggttttcccagtcacgacgttgtaaaacgacggccagtgaattc

SEQ ID NO: 7 - DNA, 12088 bp, Artificial Sequence
  Synthetic: TL20c-r7SKM1/sh734-rGbGM
ggccgcctcggccaaacagcccttgagtttaccactccctatcagtgatagagaaaagtgaaagtcgagtttaccactccctatcagtgatagagaaaagtgaaagtcgagtttaccactccctatcagtgatagagaaaagtgaaagtcgagtttaccactccctatcagtgatagagaaaagtgaaagtcgagtttaccagtccctatcagtgatagagaaaagtgaaagtcgagtttaccactccctatcagtgatagagaaaagtgaaagtcgagtttaccactccctatcagtgatagagaaaagtgaaagtcgagctcgccatgggaggcgtggcctgggcgggactggggagtggcgagccctcagatcctgcatataagcagctgctttttgcctgtactgggtctctctggttagaccagatctgagcctgggagctctctggctaactagggaacccactgcttaagcctcaataaagcttgccttgagtgcttcaagtagtgtgtgcccgtctgttgtgtgactctggtaactagagatccctcagacccttttagtcagtgtggaaaatctctagcagtggcgcccgaacagggacttgaaagcgaaagggaaaccagaggagctctctcgacgcaggactcggcttgctgaagcgcgcacggcaagaggcgaggggcggcgactggtgagtacgccaaaaattttgactagcggaggctagaaggagagagatgggtgcgagagcgtcagtattaagcgggggagaattagatcgcgatgggaaaaaattcggttaaggccagggggaaagaaaaaatataaattaaaacatatagtatgggcaagcagggagctagaacgattcgcagttaatactggcctgttagaaacatcagaaggctgtagacaaatactgggacagctacaaccatcccttcagacaggatcagaagaacttagatcattatataatacagtagcaaccctctattgtgtgcatcaaaggatagagataaaagacaccaaggaagctttagacaagatagaggaagagcaaaacaaaagtaagaaaaaagcacagcaagcagcaggatcttcagacctggaaattccctacaatccccaaagtcaaggagtagtagaatctatgaataaagaattaaagaaaattataggacaggtaagagatcaggctgaacatcttaagacagcagtacaaatggcagtattcatccacaattttaaaagaaaaggggggattggggggtacagtgcaggggaaagaatagtagacataatagcaacagacatacaaactaaagaattacaaaaacaaattacaaaaattcaaaattttcgggtttattacagggacagcagaaatccactttggaaaggaccagcaaagctcctctggaaaggtgaaggggcagtagtaatacaagataatagtgacataaaagtagtgccaagaagaaaagcaaagatcattagggattatggaaaacagatggcaggtgatgattgtgtggcaagtagacaggatgaggattagaacatggaaaagtttagtaaaacaccataaggaggagatatgagggacaattggagaagtgaattatataaatataaagtagtaaaaattgaaccattaggagtagcacccaccaaggcaaagagaagagtggtgcagagagaaaaaagagcagtgggaataggagctttgttccttgggttcttgggagcagcaggaagcactatgggcgcagcgtcaatgacgctgacggtacaggccagacaattattgtctggtatagtgcagcagcagaacaatttgctgagggctattgaggcgcaacagcatctgttgcaactcacagtctggggcatcaagcagctccaggcaagaatcctggctgtggaaagatacctaaaggatcaacagctcctggggatttggggttgctctggaaaactcatttgcaccactgctgtgccttggaatgctagttggagtaataaatctctggaacagatttggaatcacacgacctggatggagtgggacagagaaattaacaattacacaagcttaatacactccttaattgaagaatcgcaaaaccagcaagaaaagaatgaacaagaattattggaattagataaatgggcaagtttgtggaattggtttaacataacaaattggctgtggtatataaaattattcataatgatagtaggaggcttggtaggtttaagaatagtttttgctgtactttctatagtgaatagagttaggcagggatattcaccattatcgtttcagacccacctcccaaccccgaggggaccgagctcaagcttcgaagcggccgcaaaaaaggatatgcccttgactatgtcggacaaatagtcaagggcatatcctgaggtacccaggcggcgcacaagctatataaacctgaaggaaatctcaactttacacttaggtcaagttacttatcgtactagagcttcagcaggaaatttaactaaaatctaatttaaccagcatagcaaatatcatttattcccaaaatgctaaagtttgagataaacggacttgatttccggctgttttgacactatccagaatgccggtactatgggtggggcagtagcccgactgcacgtcgaacgcgtggggatcctctagagtcgagctcgcgaggatcatcaccggtgctagccggagccagaagcaccataagggacatgataagggagccagcagacctctgatctcttcctgaatgctaatcttaaacatcctgaggaagaatgggacttccatttggggtgggcctatgatagggtaataagacagtagtgaatatcaagctacaaaaagccccctttcaaattcttctcagtcctaacttttcatactaagcccagtccttccaaagcagactgtgaaagagtgatagttccgggagactagcaccggctagccgagcttggaacactttcccttcattaagaaccatccttgctactcagctgcaatcaatccagcccccaggtcttcactgaaccttttcccatctcttccaaaacatctgtttctgagaagtcctgtcctatagaggtctttcttcccaccggatttctcctacaccatttactcccacttgcagaactcccgtgtacaagtgtctttactgcttttatttgctcaacaaaatgcacatctcatataaaaataaatgaggagcatgcacacaccacaaacacaaacaggcatgcagaaatacacatacacacttccctcaatataaaccctttgtggctcatatatttaaaaagatgtaaaaaaaagagctgaagaaaatcatgtgtgatctctcagcagaatagatttattatttgtattgcttgcagaataaagcctatccttgaaagctctgaatcatgggcaagaggctcagtggtatctggaggacagggcactggccactgcagtcaccatcttctgccaggaagcctgcacctcaggggtgaattctttgccaaagtgaatggccagcacggtgaccagcacgttgcccaggagctgtgggaggaagataagaggtatgaacatgattagcaaaagggcctagcttggactcagaataatccagccttatcccaaccataaaataaaagcagaatggtagctggattgtagctgctattagcaatatgaaacctcttacatcagttacaatttatatgcagaaatatttatatgcagaaatattgctattgccttaacccagaaattatcactgttattctttagaatggtgcaaagaggcatgatacattgtatcattattgccctgaaagaaagagattagggaaagtattagaaataagataaacaaaaaagtatattaaaagaagaaagcattttttaaaattacaaatgcaaaattaccctgatttggtcaatatgtgtaccctgttacttctccccttcctatgacatgaacttaaccatagaaaagaaggggaaagaaaacatcaagggtcccatagactcaccttgaagttctcaggatccacatgcagcttgtcacagtgcagttcactcagctgggcaaaggtgcccttgagatcatccaggtgctttatggcatctcccaaggaagtcagcaccttcttgccatgtgccttgactttggggttgcccatgatggcagaggcagaggacaggttgccaaagctgtcaaagaacctctgggtccatgggtagacaaccaggagcctgtgagattgacaagaacagtttgacagtcagaaggtgccacaaatcctgagaagcaacctggacttttgccaggcacagggtccttccttccctcccttgtcctggtcaccagagcctaccttcccagggtttctcctccagcatcttccacattcaccttgtcccacaggcttgtgatagtagccttgtcctcctctgtgaaatgacccatggtgtctgtttgaggttgctagtgaacacagttgtgtcagaagcaaatgtaagcaatagatggctctgccctgacttttatgcccagccctggctcctgccctccctgctcctgggagtagattggccaaccctagggtgtggctccacagggtgaggtctaagtgatgacagccgtacctgtccttggctcttctggcactggcttaggagttggacttcaaaccctcagccctccctctaagatatatctcttggccccataccatcagtacaaattgctactaaaaacatcctcctttgcaagtgtatttacgacggtatcgatgtatgtgagcatgtgtcctctaacagcacaggccttttgccacctagctgtccaggggtgccttaaaatggcaaacaaggtttgttttcttttcctgttttcatgccttcctcttccatatccttgtttcatattaatacatgtgtatagatcctaaaaatctatacacatgtattaataaagcctgattctgccgcttctaggtatagaggccacctgcaagataaatatttgattcacaataactaatcattctatggcaattgataacaacaaatatatatatatatatatatatacgtatatgtgtatatatatatatatattcaggaaataatatattctagaatatgtcacattctgtctcaggcatccattttctttatgatgccgtttgaggtggagttttagtcaggtggtcagcttctccttttttttgccatctgccctgtaagcatcctgctggggacccagataggagtcatcactctaggctgagaacatctgggcacacaccctaagcctcagcatgactcatcatgactcagcattgctgtgcttgagccagaaggtttgcttagaaggttacacagaaccagaaggcgggggtggggcactgaccccgacaggggcctggccagaactgctcatgcttggactatgggaggtcactaatggagacacacagaaatgtaacaggaactaagggaattccggtgccctgcttaggagcttaatctttaatgaaagctaagctttcattaaaaaaagtctaaccagctgcattcgactttgactgcagcagctggttagaaggttctactggaggagggtcccagcccattgctaaattaacatcaggctctgagactggcagtatatctctaacagtggttgatgctatcttctggaacttgcctgctacattgagaccactgacccatacataggaagcccatagctctgtcctgaactgttaggccactggtccagagagtgtgcatctcctttgatcctcataataaccctatgagatagacacaattattactcttactttatagatgatgatcctgaaaacataggagtcaaggcacttgcccctagctgggggtataggggagcagtcccatgtagtagtagaatgaaaaatgctgctatgctgtgcctcccccacctttcccatgtctgccctctactcatggtctatctctcctggctcctgggagtcatggactccacccagcaccaccaacctgacctaaccacctatctgagcctgccagcctataacccatctgggccctgatagctggtggccagccctgaccccaccccaccctccctggaacctctgatagacacatctggcacaccagctcgcaaagtcaccgtgagggtcttgtgtttgctgagtcaaaattccttgaaatccaagtccttagagactcctgctcccaaatttacagtcatagacttcttcatggctgtctcctttatccacagaatgattcctttgcttcattgccccatccatctgatcctcctcatcagtgcagcacagggcccatgagcagtagctgcagagtctcacataggtctggcactgcctctgacatgtccgaccttaggcaaatgcttgactcttctgagctcggatcccttgagctcaggaggtcaaggctgcagtgagacatgatcttgccactgcactccagcctggacagcagagtgaaaccttgcctcacgaaacagaatacaaaaacaaacaaacaaaaaactgctccgcaatgcgcttccttgatgctctaccacataggtctgggtactttgtacacattatctcattgctgttcataattgttagattaattttgtaatattgatattattcctagaaagctgaggcctcaagatgataacttttattttctggacttgtaatagctttctcttgtattcaccatgttgtaactttcttagagtagtaacaatataaagttattgtgagtttttgcaaacacagcaaacacaacgacccatatagacattgatgtgaaattgtctattgtcaatttatgggaaaacaagtatgtactttttctactaagccattgaaacaggaataacagaacaagattgaaagaatacattttccgaaattacttgagtattatacaaagacaagcacgtggacctgggaggagggttattgtccatgactggtgtgtggagacaaatgcaggtttataatagatgggatggcatctagcgcaatgactttgccatcacttttagagagctcttgggggccccagtacacaagaggggacgcagggtatatgtagacatctcattctttttcttagtgtgagaataagaatagccatgacctgagtttatagacaatgagcccttttctctctcccactcagcagctatgagatggcttgccctgcctctctactaggctgactcactccaaggcccagcaatgggcagggctctgtcagggctttgatagcactatctgcagagccagggccgagaaggggtggactccagagactctccctcccattcccgagcagggtttgcttatttatgcatttaaatgatatatttattttaaaagaaataacaggagactgcccagccctggctgtgacatggaaactatgtagaatattttgggttccatttttttttccttctttcagttagaggaaaaggggctcactgcacatacactagacagaaagtcaggagctttgaatccaagcctgatcatttccatgtcatactgagaaagtccccacccttctctgagcctcagtttctctttttataagtaggagtctggagtaaatgatttccaatggctctcatttcaatacaaaatttccgtttattaaatgcatgagcttccgttactccaagactgagaaggaaattgaacctgagactcattgactggcaagatgtccccagaggctctcattcagcaataaaattctcaccttcacccaggcccactagtgtcagatttgcatgcgttaacgcggccgcatcgatgccgtagtacctttaagaccaatgacttacaaggcagctgtagatcttagccactttttaaaagaaaaggggggactggaagggctaattcactcccaaagaagacaagatccctgcaggcattcaaggccaggctggatgtggctctgggcagcctgggctgctggttgatgaccctgcacatagcagggggttggatctggatgagcactgtgctcctttgcaacccaggccgttctatgattctgtcattctaaatctctctttcagcctaaagctttttccccgtatccccccaggtgtctgcaggctcaaagagcagcgagaagcgttcagaggaaagcgatcccgtgccaccttccccgtgcccgggctgtccccgcacgctgccggctcggggatgcggggggagcgccggaccggagcggagccccgggcggctcgctgctgccccctagcgggggagggacgtaattacatccctgggggctttgggggggggctgtccccgtgagctccccagatctgctttttgcctgtactgggtctctctggttagaccagatctgagcctgggagctctctggctaactagggaacccactgcttaagcctcaataaagcttcagctgctcgagctagcagatctttttccctctgccaaaaattatggggacatcatgaagccccttgagcatctgacttctggctaataaaggaaatttattttcattgcaatagtgtgttggaattttttgtgtctctcactcggaaggacatatgggagggcaaatcatttaaaacatcagaatgagtatttggtttagagtttggcaacatatgcccatatgctggctgccatgaacaaaggttggctataaagaggtcatcagtatatgaaacagccccctgctgtccattccttattccatagaaaagccttgacttgaggttagattttttttatattttgttttgtgttatttttttctttaacatccctaaaattttccttacatgttttactagccagatttttcctcctctcctgactactcccagtcatagctgtccctcttctcttatggagatccctcgacctgcagcccaagcttggcgtaatcatggtcatagctgtttcctgtgtgaaattgttatccgctcacaattccacacaacatacgagccggaagcataaagtgtaaagcctggggtgcctaatgagtgagctaactcacattaattgcgttgcgctcactgcccgctttccagtcgggaaacctgtcgtgccagcggatccgcatctcaattagtcagcaaccatagtcccgcccctaactccgcccatcccgcccctaactccgcccagttccgcccattctccgccccatggctgactaattttttttatttatgcagaggccgaggccgcctcggcctctgagctattccagaagtagtgaggaggcttttttggaggcctaggcttttgcaaaaagctgtcgactgcagaggcctgcatgcaagcttggcgtaatcatggtcatagctgtttcctgtgtgaaattgttatccgctcacaattccacacaacatacgagccggaagcataaagtgtaaagcctggggtgcctaatgagtgagctaactcacattaattgcgttgcgctcactgcccgctttccagtcgggaaacctgtcgtgccagctgcattaatgaatcggccaacgcgcggggagaggcggtttgcgtattgggcgctcttccgcttcctcgctcactgactcgctgcgctcggtcgttcggctgcggcgagcggtatcagctcactcaaaggcggtaatacggttatccacagaatcaggggataacgcaggaaagaacatgtgagcaaaaggccagcaaaaggccaggaaccgtaaaaaggccgcgttgctggcgtttttccataggctccgcccccctgacgagcatcacaaaaatcgacgctcaagtcagaggtggcgaaacccgacaggactataaagataccaggcgtttccccctggaagctccctcgtgcgctctcctgttccgaccctgccgcttaccggatacctgtccgcctttctcccttcgggaagcgtggcgctttctcatagctcacgctgtaggtatctcagttcggtgtaggtcgttcgctccaagctgggctgtgtgcacgaaccccccgttcagcccgaccgctgcgccttatccggtaactatcgtcttgagtccaacccggtaagacacgacttatcgccactggcagcagccactggtaacaggattagcagagcgaggtatgtaggcggtgctacagagttcttgaagtggtggcctaactacggctacactagaagaacagtatttggtatctgcgctctgctgaagccagttaccttcggaaaaagagttggtagctcttgatccggcaaacaaaccaccgctggtagcggtggtttttttgtttgcaagcagcagattacgcgcagaaaaaaaggatctcaagaagatcctttgatcttttctacggggtctgacgctcagtggaacgaaaactcacgttaagggattttggtcatgagattatcaaaaaggatcttcacctagatccttttaaattaaaaatgaagttttaaatcaatctaaagtatatatgagtaaacttggtctgacagttaccaatgcttaatcagtgaggcacctatctcagcgatctgtctatttcgttcatccatagttgcctgactccccgtcgtgtagataactacgatacgggagggcttaccatctggccccagtgctgcaatgataccgcgagacccacgctcaccggctccagatttatcagcaataaaccagccagccggaagggccgagcgcagaagtggtcctgcaactttatccgcctccatccagtctattaattgttgccgggaagctagagtaagtagttcgccagttaatagtttgcgcaacgttgttgccattgctacaggcatcgtggtgtcacgctcgtcgtttggtatggcttcattcagctccggttcccaacgatcaaggcgagttacatgatcccccatgttgtgcaaaaaagcggttagctccttcggtcctccgatcgttgtcagaagtaagttggccgcagtgttatcactcatggttatggcagcactgcataattctcttactgtcatgccatccgtaagatgcttttctgtgactggtgagtactcaaccaagtcattctgagaatagtgtatgcggcgaccgagttgctcttgcccggcgtcaatacgggataataccgcgccacatagcagaactttaaaagtgctcatcattggaaaacgttcttcggggcgaaaactctcaaggatcttaccgctgttgagatccagttcgatgtaacccactcgtgcacccaactgatcttcagcatcttttactttcaccagcgtttctgggtgagcaaaaacaggaaggcaaaatgccgcaaaaaagggaataagggcgacacggaaatgttgaatactcatactcttcctttttcaatattattgaagcatttatcagggttattgtctcatgagcggatacatatttgaatgtatttagaaaaataaacaaataggggttccgcgcacatttccccgaaaagtgccacctgacgtctaagaaaccattattatcatgacattaacctataaaaataggcgtatcacgaggccctttcgtctcgcgcgtttcggtgatgacggtgaaaacctctgacacatgcagctcccggagacggtcacagcttgtctgtaagcggatgccgggagcagacaagcccgtcagggcgcgtcagcgggtgttggcgggtgtcggggctggcttaactatgcggcatcagagcagattgtactgagagtgcaccatatgcggtgtgaaataccgcacagatgcgtaaggagaaaataccgcatcaggcgccattcgccattcaggctgcgcaactgttgggaagggcgatcggtgcgggcctcttcgctattacgccagctggcgaaagggggatgtgctgcaaggcgattaagttgggtaacgccagggttttcccagtcacgacgttgtaaaacgacggccagtgaattc

SEQ ID NO: 8 - DNA, 12091 bp, Artificial Sequence
  Synthetic: TL20c-r7SK/sh734-rGbGM
ggccgcctcggccaaacagcccttgagtttaccactccctatcagtgatagagaaaagtgaaagtcgagtttaccactccctatcagtgatagagaaaagtgaaagtcgagtttaccactccctatcagtgatagagaaaagtgaaagtcgagtttaccactccctatcagtgatagagaaaagtgaaagtcgagtttaccagtccctatcagtgatagagaaaagtgaaagtcgagtttaccactccctatcagtgatagagaaaagtgaaagtcgagtttaccactccctatcagtgatagagaaaagtgaaagtcgagctcgccatgggaggcgtggcctgggcgggactggggagtggcgagccctcagatcctgcatataagcagctgctttttgcctgtactgggtctctctggttagaccagatctgagcctgggagctctctggctaactagggaacccactgcttaagcctcaataaagcttgccttgagtgcttcaagtagtgtgtgcccgtctgttgtgtgactctggtaactagagatccctcagacccttttagtcagtgtggaaaatctctagcagtggcgcccgaacagggacttgaaagcgaaagggaaaccagaggagctctctcgacgcaggactcggcttgctgaagcgcgcacggcaagaggcgaggggcggcgactggtgagtacgccaaaaattttgactagcggaggctagaaggagagagatgggtgcgagagcgtcagtattaagcgggggagaattagatcgcgatgggaaaaaattcggttaaggccagggggaaagaaaaaatataaattaaaacatatagtatgggcaagcagggagctagaacgattcgcagttaatactggcctgttagaaacatcagaaggctgtagacaaatactgggacagctacaaccatcccttcagacaggatcagaagaacttagatcattatataatacagtagcaaccctctattgtgtgcatcaaaggatagagataaaagacaccaaggaagctttagacaagatagaggaagagcaaaacaaaagtaagaaaaaagcacagcaagcagcaggatcttcagacctggaaattccctacaatccccaaagtcaaggagtagtagaatctatgaataaagaattaaagaaaattataggacaggtaagagatcaggctgaacatcttaagacagcagtacaaatggcagtattcatccacaattttaaaagaaaaggggggattggggggtacagtgcaggggaaagaatagtagacataatagcaacagacatacaaactaaagaattacaaaaacaaattacaaaaattcaaaattttcgggtttattacagggacagcagaaatccactttggaaaggaccagcaaagctcctctggaaaggtgaaggggcagtagtaatacaagataatagtgacataaaagtagtgccaagaagaaaagcaaagatcattagggattatggaaaacagatggcaggtgatgattgtgtggcaagtagacaggatgaggattagaacatggaaaagtttagtaaaacaccataaggaggagatatgagggacaattggagaagtgaattatataaatataaagtagtaaaaattgaaccattaggagtagcacccaccaaggcaaagagaagagtggtgcagagagaaaaaagagcagtgggaataggagctttgttccttgggttcttgggagcagcaggaagcactatgggcgcagcgtcaatgacgctgacggtacaggccagacaattattgtctggtatagtgcagcagcagaacaatttgctgagggctattgaggcgcaacagcatctgttgcaactcacagtctggggcatcaagcagctccaggcaagaatcctggctgtggaaagatacctaaaggatcaacagctcctggggatttggggttgctctggaaaactcatttgcaccactgctgtgccttggaatgctagttggagtaataaatctctggaacagatttggaatcacacgacctggatggagtgggacagagaaattaacaattacacaagcttaatacactccttaattgaagaatcgcaaaaccagcaagaaaagaatgaacaagaattattggaattagataaatgggcaagtttgtggaattggtttaacataacaaattggctgtggtatataaaattattcataatgatagtaggaggcttggtaggtttaagaatagtttttgctgtactttctatagtgaatagagttaggcagggatattcaccattatcgtttcagacccacctcccaaccccgaggggaccgagctcaagcttcgaagcggccgcacaaaaaaggatatgcccttgactatgtcggacaaatagtcaagggcatatcctgaggtacccaggcggcgcacaagctatataaacctgaaggaaatctcaactttacacttaggtcaagttacttatcgtactagagcttcagcaggaaatttaactaaaatctaatttaaccagcatagcaaatatcatttattcccaaaatgctaaagtttgagataaacggacttgatttccggctgttttgacactatccagaatgccttgcagatgggtggggcatgctaaatactgcacgtcgatacgcgtggggatcctctagagtcgagctcgcgaggatcatcaccggtgctagccggagccagaagcaccataagggacatgataagggagccagcagacctctgatctcttcctgaatgctaatcttaaacatcctgaggaagaatgggacttccatttggggtgggcctatgatagggtaataagacagtagtgaatatcaagctacaaaaagccccctttcaaattcttctcagtcctaacttttcatactaagcccagtccttccaaagcagactgtgaaagagtgatagttccgggagactagcaccggctagccgagcttggaacactttcccttcattaagaaccatccttgctactcagctgcaatcaatccagcccccaggtcttcactgaaccttttcccatctcttccaaaacatctgtttctgagaagtcctgtcctatagaggtctttcttcccaccggatttctcctacaccatttactcccacttgcagaactcccgtgtacaagtgtctttactgcttttatttgctcaacaaaatgcacatctcatataaaaataaatgaggagcatgcacacaccacaaacacaaacaggcatgcagaaatacacatacacacttccctcaatataaaccctttgtggctcatatatttaaaaagatgtaaaaaaaagagctgaagaaaatcatgtgtgatctctcagcagaatagatttattatttgtattgcttgcagaataaagcctatccttgaaagctctgaatcatgggcaagaggctcagtggtatctggaggacagggcactggccactgcagtcaccatcttctgccaggaagcctgcacctcaggggtgaattctttgccaaagtgaatggccagcacggtgaccagcacgttgcccaggagctgtgggaggaagataagaggtatgaacatgattagcaaaagggcctagcttggactcagaataatccagccttatcccaaccataaaataaaagcagaatggtagctggattgtagctgctattagcaatatgaaacctcttacatcagttacaatttatatgcagaaatatttatatgcagaaatattgctattgccttaacccagaaattatcactgttattctttagaatggtgcaaagaggcatgatacattgtatcattattgccctgaaagaaagagattagggaaagtattagaaataagataaacaaaaaagtatattaaaagaagaaagcattttttaaaattacaaatgcaaaattaccctgatttggtcaatatgtgtaccctgttacttctccccttcctatgacatgaacttaaccatagaaaagaaggggaaagaaaacatcaagggtcccatagactcaccttgaagttctcaggatccacatgcagcttgtcacagtgcagttcactcagctgggcaaaggtgcccttgagatcatccaggtgctttatggcatctcccaaggaagtcagcaccttcttgccatgtgccttgactttggggttgcccatgatggcagaggcagaggacaggttgccaaagctgtcaaagaacctctgggtccatgggtagacaaccaggagcctgtgagattgacaagaacagtttgacagtcagaaggtgccacaaatcctgagaagcaacctggacttttgccaggcacagggtccttccttccctcccttgtcctggtcaccagagcctaccttcccagggtttctcctccagcatcttccacattcaccttgtcccacaggcttgtgatagtagccttgtcctcctctgtgaaatgacccatggtgtctgtttgaggttgctagtgaacacagttgtgtcagaagcaaatgtaagcaatagatggctctgccctgacttttatgcccagccctggctcctgccctccctgctcctgggagtagattggccaaccctagggtgtggctccacagggtgaggtctaagtgatgacagccgtacctgtccttggctcttctggcactggcttaggagttggacttcaaaccctcagccctccctctaagatatatctcttggccccataccatcagtacaaattgctactaaaaacatcctcctttgcaagtgtatttacgacggtatcgatgtatgtgagcatgtgtcctctaacagcacaggccttttgccacctagctgtccaggggtgccttaaaatggcaaacaaggtttgttttcttttcctgttttcatgccttcctcttccatatccttgtttcatattaatacatgtgtatagatcctaaaaatctatacacatgtattaataaagcctgattctgccgcttctaggtatagaggccacctgcaagataaatatttgattcacaataactaatcattctatggcaattgataacaacaaatatatatatatatatatatatacgtatatgtgtatatatatatatatattcaggaaataatatattctagaatatgtcacattctgtctcaggcatccattttctttatgatgccgtttgaggtggagttttagtcaggtggtcagcttctccttttttttgccatctgccctgtaagcatcctgctggggacccagataggagtcatcactctaggctgagaacatctgggcacacaccctaagcctcagcatgactcatcatgactcagcattgctgtgcttgagccagaaggtttgcttagaaggttacacagaaccagaaggcgggggtggggcactgaccccgacaggggcctggccagaactgctcatgcttggactatgggaggtcactaatggagacacacagaaatgtaacaggaactaagggaattccggtgccctgcttaggagcttaatctttaatgaaagctaagctttcattaaaaaaagtctaaccagctgcattcgactttgactgcagcagctggttagaaggttctactggaggagggtcccagcccattgctaaattaacatcaggctctgagactggcagtatatctctaacagtggttgatgctatcttctggaacttgcctgctacattgagaccactgacccatacataggaagcccatagctctgtcctgaactgttaggccactggtccagagagtgtgcatctcctttgatcctcataataaccctatgagatagacacaattattactcttactttatagatgatgatcctgaaaacataggagtcaaggcacttgcccctagctgggggtataggggagcagtcccatgtagtagtagaatgaaaaatgctgctatgctgtgcctcccccacctttcccatgtctgccctctactcatggtctatctctcctggctcctgggagtcatggactccacccagcaccaccaacctgacctaaccacctatctgagcctgccagcctataacccatctgggccctgatagctggtggccagccctgaccccaccccaccctccctggaacctctgatagacacatctggcacaccagctcgcaaagtcaccgtgagggtcttgtgtttgctgagtcaaaattccttgaaatccaagtccttagagactcctgctcccaaatttacagtcatagacttcttcatggctgtctcctttatccacagaatgattcctttgcttcattgccccatccatctgatcctcctcatcagtgcagcacagggcccatgagcagtagctgcagagtctcacataggtctggcactgcctctgacatgtccgaccttaggcaaatgcttgactcttctgagctcggatcccttgagctcaggaggtcaaggctgcagtgagacatgatcttgccactgcactccagcctggacagcagagtgaaaccttgcctcacgaaacagaatacaaaaacaaacaaacaaaaaactgctccgcaatgcgcttccttgatgctctaccacataggtctgggtactttgtacacattatctcattgctgttcataattgttagattaattttgtaatattgatattattcctagaaagctgaggcctcaagatgataacttttattttctggacttgtaatagctttctcttgtattcaccatgttgtaactttcttagagtagtaacaatataaagttattgtgagtttttgcaaacacagcaaacacaacgacccatatagacattgatgtgaaattgtctattgtcaatttatgggaaaacaagtatgtactttttctactaagccattgaaacaggaataacagaacaagattgaaagaatacattttccgaaattacttgagtattatacaaagacaagcacgtggacctgggaggagggttattgtccatgactggtgtgtggagacaaatgcaggtttataatagatgggatggcatctagcgcaatgactttgccatcacttttagagagctcttgggggccccagtacacaagaggggacgcagggtatatgtagacatctcattctttttcttagtgtgagaataagaatagccatgacctgagtttatagacaatgagcccttttctctctcccactcagcagctatgagatggcttgccctgcctctctactaggctgactcactccaaggcccagcaatgggcagggctctgtcagggctttgatagcactatctgcagagccagggccgagaaggggtggactccagagactctccctcccattcccgagcagggtttgcttatttatgcatttaaatgatatatttattttaaaagaaataacaggagactgcccagccctggctgtgacatggaaactatgtagaatattttgggttccatttttttttccttctttcagttagaggaaaaggggctcactgcacatacactagacagaaagtcaggagctttgaatccaagcctgatcatttccatgtcatactgagaaagtccccacccttctctgagcctcagtttctctttttataagtaggagtctggagtaaatgatttccaatggctctcatttcaatacaaaatttccgtttattaaatgcatgagcttccgttactccaagactgagaaggaaattgaacctgagactcattgactggcaagatgtccccagaggctctcattcagcaataaaattctcaccttcacccaggcccactagtgtcagatttgcatgcgttaacgcggccgcatcgatgccgtagtacctttaagaccaatgacttacaaggcagctgtagatcttagccactttttaaaagaaaaggggggactggaagggctaattcactcccaaagaagacaagatccctgcaggcattcaaggccaggctggatgtggctctgggcagcctgggctgctggttgatgaccctgcacatagcagggggttggatctggatgagcactgtgctcctttgcaacccaggccgttctatgattctgtcattctaaatctctctttcagcctaaagctttttccccgtatccccccaggtgtctgcaggctcaaagagcagcgagaagcgttcagaggaaagcgatcccgtgccaccttccccgtgcccgggctgtccccgcacgctgccggctcggggatgcggggggagcgccggaccggagcggagccccgggcggctcgctgctgccccctagcgggggagggacgtaattacatccctgggggctttgggggggggctgtccccgtgagctccccagatctgctttttgcctgtactgggtctctctggttagaccagatctgagcctgggagctctctggctaactagggaacccactgcttaagcctcaataaagcttcagctgctcgagctagcagatctttttccctctgccaaaaattatggggacatcatgaagccccttgagcatctgacttctggctaataaaggaaatttattttcattgcaatagtgtgttggaattttttgtgtctctcactcggaaggacatatgggagggcaaatcatttaaaacatcagaatgagtatttggtttagagtttggcaacatatgcccatatgctggctgccatgaacaaaggttggctataaagaggtcatcagtatatgaaacagccccctgctgtccattccttattccatagaaaagccttgacttgaggttagattttttttatattttgttttgtgttatttttttctttaacatccctaaaattttccttacatgttttactagccagatttttcctcctctcctgactactcccagtcatagctgtccctcttctcttatggagatccctcgacctgcagcccaagcttggcgtaatcatggtcatagctgtttcctgtgtgaaattgttatccgctcacaattccacacaacatacgagccggaagcataaagtgtaaagcctggggtgcctaatgagtgagctaactcacattaattgcgttgcgctcactgcccgctttccagtcgggaaacctgtcgtgccagcggatccgcatctcaattagtcagcaaccatagtcccgcccctaactccgcccatcccgcccctaactccgcccagttccgcccattctccgccccatggctgactaattttttttatttatgcagaggccgaggccgcctcggcctctgagctattccagaagtagtgaggaggcttttttggaggcctaggcttttgcaaaaagctgtcgactgcagaggcctgcatgcaagcttggcgtaatcatggtcatagctgtttcctgtgtgaaattgttatccgctcacaattccacacaacatacgagccggaagcataaagtgtaaagcctggggtgcctaatgagtgagctaactcacattaattgcgttgcgctcactgcccgctttccagtcgggaaacctgtcgtgccagctgcattaatgaatcggccaacgcgcggggagaggcggtttgcgtattgggcgctcttccgcttcctcgctcactgactcgctgcgctcggtcgttcggctgcggcgagcggtatcagctcactcaaaggcggtaatacggttatccacagaatcaggggataacgcaggaaagaacatgtgagcaaaaggccagcaaaaggccaggaaccgtaaaaaggccgcgttgctggcgtttttccataggctccgcccccctgacgagcatcacaaaaatcgacgctcaagtcagaggtggcgaaacccgacaggactataaagataccaggcgtttccccctggaagctccctcgtgcgctctcctgttccgaccctgccgcttaccggatacctgtccgcctttctcccttcgggaagcgtggcgctttctcatagctcacgctgtaggtatctcagttcggtgtaggtcgttcgctccaagctgggctgtgtgcacgaaccccccgttcagcccgaccgctgcgccttatccggtaactatcgtcttgagtccaacccggtaagacacgacttatcgccactggcagcagccactggtaacaggattagcagagcgaggtatgtaggcggtgctacagagttcttgaagtggtggcctaactacggctacactagaagaacagtatttggtatctgcgctctgctgaagccagttaccttcggaaaaagagttggtagctcttgatccggcaaacaaaccaccgctggtagcggtggtttttttgtttgcaagcagcagattacgcgcagaaaaaaaggatctcaagaagatcctttgatcttttctacggggtctgacgctcagtggaacgaaaactcacgttaagggattttggtcatgagattatcaaaaaggatcttcacctagatccttttaaattaaaaatgaagttttaaatcaatctaaagtatatatgagtaaacttggtctgacagttaccaatgcttaatcagtgaggcacctatctcagcgatctgtctatttcgttcatccatagttgcctgactccccgtcgtgtagataactacgatacgggagggcttaccatctggccccagtgctgcaatgataccgcgagacccacgctcaccggctccagatttatcagcaataaaccagccagccggaagggccgagcgcagaagtggtcctgcaactttatccgcctccatccagtctattaattgttgccgggaagctagagtaagtagttcgccagttaatagtttgcgcaacgttgttgccattgctacaggcatcgtggtgtcacgctcgtcgtttggtatggcttcattcagctccggttcccaacgatcaaggcgagttacatgatcccccatgttgtgcaaaaaagcggttagctccttcggtcctccgatcgttgtcagaagtaagttggccgcagtgttatcactcatggttatggcagcactgcataattctcttactgtcatgccatccgtaagatgcttttctgtgactggtgagtactcaaccaagtcattctgagaatagtgtatgcggcgaccgagttgctcttgcccggcgtcaatacgggataataccgcgccacatagcagaactttaaaagtgctcatcattggaaaacgttcttcggggcgaaaactctcaaggatcttaccgctgttgagatccagttcgatgtaacccactcgtgcacccaactgatcttcagcatcttttactttcaccagcgtttctgggtgagcaaaaacaggaaggcaaaatgccgcaaaaaagggaataagggcgacacggaaatgttgaatactcatactcttcctttttcaatattattgaagcatttatcagggttattgtctcatgagcggatacatatttgaatgtatttagaaaaataaacaaataggggttccgcgcacatttccccgaaaagtgccacctgacgtctaagaaaccattattatcatgacattaacctataaaaataggcgtatcacgaggccctttcgtctcgcgcgtttcggtgatgacggtgaaaacctctgacacatgcagctcccggagacggtcacagcttgtctgtaagcggatgccgggagcagacaagcccgtcagggcgcgtcagcgggtgttggcgggtgtcggggctggcttaactatgcggcatcagagcagattgtactgagagtgcaccatatgcggtgtgaaataccgcacagatgcgtaaggagaaaataccgcatcaggcgccattcgccattcaggctgcgcaactgttgggaagggcgatcggtgcgggcctcttcgctattacgccagctggcgaaagggggatgtgctgcaaggcgattaagttgggtaacgccagggttttcccagtcacgacgttgtaaaacgacggccagtgaattc

SEQ ID NO: 9 - DNA, 12081 bp, Artificial Sequence
  Synthetic: TL20c-rGbGM-7SKM1/sh734
ggccgcctcggccaaacagcccttgagtttaccactccctatcagtgatagagaaaagtgaaagtcgagtttaccactccctatcagtgatagagaaaagtgaaagtcgagtttaccactccctatcagtgatagagaaaagtgaaagtcgagtttaccactccctatcagtgatagagaaaagtgaaagtcgagtttaccagtccctatcagtgatagagaaaagtgaaagtcgagtttaccactccctatcagtgatagagaaaagtgaaagtcgagtttaccactccctatcagtgatagagaaaagtgaaagtcgagctcgccatgggaggcgtggcctgggcgggactggggagtggcgagccctcagatcctgcatataagcagctgctttttgcctgtactgggtctctctggttagaccagatctgagcctgggagctctctggctaactagggaacccactgcttaagcctcaataaagcttgccttgagtgcttcaagtagtgtgtgcccgtctgttgtgtgactctggtaactagagatccctcagacccttttagtcagtgtggaaaatctctagcagtggcgcccgaacagggacttgaaagcgaaagggaaaccagaggagctctctcgacgcaggactcggcttgctgaagcgcgcacggcaagaggcgaggggcggcgactggtgagtacgccaaaaattttgactagcggaggctagaaggagagagatgggtgcgagagcgtcagtattaagcgggggagaattagatcgcgatgggaaaaaattcggttaaggccagggggaaagaaaaaatataaattaaaacatatagtatgggcaagcagggagctagaacgattcgcagttaatactggcctgttagaaacatcagaaggctgtagacaaatactgggacagctacaaccatcccttcagacaggatcagaagaacttagatcattatataatacagtagcaaccctctattgtgtgcatcaaaggatagagataaaagacaccaaggaagctttagacaagatagaggaagagcaaaacaaaagtaagaaaaaagcacagcaagcagcaggatcttcagacctggaaattccctacaatccccaaagtcaaggagtagtagaatctatgaataaagaattaaagaaaattataggacaggtaagagatcaggctgaacatcttaagacagcagtacaaatggcagtattcatccacaattttaaaagaaaaggggggattggggggtacagtgcaggggaaagaatagtagacataatagcaacagacatacaaactaaagaattacaaaaacaaattacaaaaattcaaaattttcgggtttattacagggacagcagaaatccactttggaaaggaccagcaaagctcctctggaaaggtgaaggggcagtagtaatacaagataatagtgacataaaagtagtgccaagaagaaaagcaaagatcattagggattatggaaaacagatggcaggtgatgattgtgtggcaagtagacaggatgaggattagaacatggaaaagtttagtaaaacaccataaggaggagatatgagggacaattggagaagtgaattatataaatataaagtagtaaaaattgaaccattaggagtagcacccaccaaggcaaagagaagagtggtgcagagagaaaaaagagcagtgggaataggagctttgttccttgggttcttgggagcagcaggaagcactatgggcgcagcgtcaatgacgctgacggtacaggccagacaattattgtctggtatagtgcagcagcagaacaatttgctgagggctattgaggcgcaacagcatctgttgcaactcacagtctggggcatcaagcagctccaggcaagaatcctggctgtggaaagatacctaaaggatcaacagctcctggggatttggggttgctctggaaaactcatttgcaccactgctgtgccttggaatgctagttggagtaataaatctctggaacagatttggaatcacacgacctggatggagtgggacagagaaattaacaattacacaagcttaatacactccttaattgaagaatcgcaaaaccagcaagaaaagaatgaacaagaattattggaattagataaatgggcaagtttgtggaattggtttaacataacaaattggctgtggtatataaaattattcataatgatagtaggaggcttggtaggtttaagaatagtttttgctgtactttctatagtgaatagagttaggcagggatattcaccattatcgtttcagacccacctcccaaccccgaggggaccgagctcaagcttcgaacgcgtggggatcctctagagtcgagctcgcgaggatcatcaccggtgctagccggagccagaagcaccataagggacatgataagggagccagcagacctctgatctcttcctgaatgctaatcttaaacatcctgaggaagaatgggacttccatttggggtgggcctatgatagggtaataagacagtagtgaatatcaagctacaaaaagccccctttcaaattcttctcagtcctaacttttcatactaagcccagtccttccaaagcagactgtgaaagagtgatagttccgggagactagcaccggctagccgagcttggaacactttcccttcattaagaaccatccttgctactcagctgcaatcaatccagcccccaggtcttcactgaaccttttcccatctcttccaaaacatctgtttctgagaagtcctgtcctatagaggtctttcttcccaccggatttctcctacaccatttactcccacttgcagaactcccgtgtacaagtgtctttactgcttttatttgctcaacaaaatgcacatctcatataaaaataaatgaggagcatgcacacaccacaaacacaaacaggcatgcagaaatacacatacacacttccctcaatataaaccctttgtggctcatatatttaaaaagatgtaaaaaaaagagctgaagaaaatcatgtgtgatctctcagcagaatagatttattatttgtattgcttgcagaataaagcctatccttgaaagctctgaatcatgggcaagaggctcagtggtatctggaggacagggcactggccactgcagtcaccatcttctgccaggaagcctgcacctcaggggtgaattctttgccaaagtgaatggccagcacggtgaccagcacgttgcccaggagctgtgggaggaagataagaggtatgaacatgattagcaaaagggcctagcttggactcagaataatccagccttatcccaaccataaaataaaagcagaatggtagctggattgtagctgctattagcaatatgaaacctcttacatcagttacaatttatatgcagaaatatttatatgcagaaatattgctattgccttaacccagaaattatcactgttattctttagaatggtgcaaagaggcatgatacattgtatcattattgccctgaaagaaagagattagggaaagtattagaaataagataaacaaaaaagtatattaaaagaagaaagcattttttaaaattacaaatgcaaaattaccctgatttggtcaatatgtgtaccctgttacttctccccttcctatgacatgaacttaaccatagaaaagaaggggaaagaaaacatcaagggtcccatagactcaccttgaagttctcaggatccacatgcagcttgtcacagtgcagttcactcagctgggcaaaggtgcccttgagatcatccaggtgctttatggcatctcccaaggaagtcagcaccttcttgccatgtgccttgactttggggttgcccatgatggcagaggcagaggacaggttgccaaagctgtcaaagaacctctgggtccatgggtagacaaccaggagcctgtgagattgacaagaacagtttgacagtcagaaggtgccacaaatcctgagaagcaacctggacttttgccaggcacagggtccttccttccctcccttgtcctggtcaccagagcctaccttcccagggtttctcctccagcatcttccacattcaccttgtcccacaggcttgtgatagtagccttgtcctcctctgtgaaatgacccatggtgtctgtttgaggttgctagtgaacacagttgtgtcagaagcaaatgtaagcaatagatggctctgccctgacttttatgcccagccctggctcctgccctccctgctcctgggagtagattggccaaccctagggtgtggctccacagggtgaggtctaagtgatgacagccgtacctgtccttggctcttctggcactggcttaggagttggacttcaaaccctcagccctccctctaagatatatctcttggccccataccatcagtacaaattgctactaaaaacatcctcctttgcaagtgtatttacgacggtatcgatgtatgtgagcatgtgtcctctaacagcacaggccttttgccacctagctgtccaggggtgccttaaaatggcaaacaaggtttgttttcttttcctgttttcatgccttcctcttccatatccttgtttcatattaatacatgtgtatagatcctaaaaatctatacacatgtattaataaagcctgattctgccgcttctaggtatagaggccacctgcaagataaatatttgattcacaataactaatcattctatggcaattgataacaacaaatatatatatatatatatatatacgtatatgtgtatatatatatatatattcaggaaataatatattctagaatatgtcacattctgtctcaggcatccattttctttatgatgccgtttgaggtggagttttagtcaggtggtcagcttctccttttttttgccatctgccctgtaagcatcctgctggggacccagataggagtcatcactctaggctgagaacatctgggcacacaccctaagcctcagcatgactcatcatgactcagcattgctgtgcttgagccagaaggtttgcttagaaggttacacagaaccagaaggcgggggtggggcactgaccccgacaggggcctggccagaactgctcatgcttggactatgggaggtcactaatggagacacacagaaatgtaacaggaactaagggaattccggtgccctgcttaggagcttaatctttaatgaaagctaagctttcattaaaaaaagtctaaccagctgcattcgactttgactgcagcagctggttagaaggttctactggaggagggtcccagcccattgctaaattaacatcaggctctgagactggcagtatatctctaacagtggttgatgctatcttctggaacttgcctgctacattgagaccactgacccatacataggaagcccatagctctgtcctgaactgttaggccactggtccagagagtgtgcatctcctttgatcctcataataaccctatgagatagacacaattattactcttactttatagatgatgatcctgaaaacataggagtcaaggcacttgcccctagctgggggtataggggagcagtcccatgtagtagtagaatgaaaaatgctgctatgctgtgcctcccccacctttcccatgtctgccctctactcatggtctatctctcctggctcctgggagtcatggactccacccagcaccaccaacctgacctaaccacctatctgagcctgccagcctataacccatctgggccctgatagctggtggccagccctgaccccaccccaccctccctggaacctctgatagacacatctggcacaccagctcgcaaagtcaccgtgagggtcttgtgtttgctgagtcaaaattccttgaaatccaagtccttagagactcctgctcccaaatttacagtcatagacttcttcatggctgtctcctttatccacagaatgattcctttgcttcattgccccatccatctgatcctcctcatcagtgcagcacagggcccatgagcagtagctgcagagtctcacataggtctggcactgcctctgacatgtccgaccttaggcaaatgcttgactcttctgagctcggatcccttgagctcaggaggtcaaggctgcagtgagacatgatcttgccactgcactccagcctggacagcagagtgaaaccttgcctcacgaaacagaatacaaaaacaaacaaacaaaaaactgctccgcaatgcgcttccttgatgctctaccacataggtctgggtactttgtacacattatctcattgctgttcataattgttagattaattttgtaatattgatattattcctagaaagctgaggcctcaagatgataacttttattttctggacttgtaatagctttctcttgtattcaccatgttgtaactttcttagagtagtaacaatataaagttattgtgagtttttgcaaacacagcaaacacaacgacccatatagacattgatgtgaaattgtctattgtcaatttatgggaaaacaagtatgtactttttctactaagccattgaaacaggaataacagaacaagattgaaagaatacattttccgaaattacttgagtattatacaaagacaagcacgtggacctgggaggagggttattgtccatgactggtgtgtggagacaaatgcaggtttataatagatgggatggcatctagcgcaatgactttgccatcacttttagagagctcttgggggccccagtacacaagaggggacgcagggtatatgtagacatctcattctttttcttagtgtgagaataagaatagccatgacctgagtttatagacaatgagcccttttctctctcccactcagcagctatgagatggcttgccctgcctctctactaggctgactcactccaaggcccagcaatgggcagggctctgtcagggctttgatagcactatctgcagagccagggccgagaaggggtggactccagagactctccctcccattcccgagcagggtttgcttatttatgcatttaaatgatatatttattttaaaagaaataacaggagactgcccagccctggctgtgacatggaaactatgtagaatattttgggttccatttttttttccttctttcagttagaggaaaaggggctcactgcacatacactagacagaaagtcaggagctttgaatccaagcctgatcatttccatgtcatactgagaaagtccccacccttctctgagcctcagtttctctttttataagtaggagtctggagtaaatgatttccaatggctctcatttcaatacaaaatttccgtttattaaatgcatgagcttccgttactccaagactgagaaggaaattgaacctgagactcattgactggcaagatgtccccagaggctctcattcagcaataaaattctcaccttcacccaggcccactagtgtcagatttgcatgcgttcgcgttcgacgtgcagtcgggctactgccccacccatagtaccggcattctggatagtgtcaaaacagccggaaatcaagtccgtttatctcaaactttagcattttgggaataaatgatatttgctatgctggttaaattagattttagttaaatttcctgctgaagctctagtacgataagtaacttgacctaagtgtaaagttgagatttccttcaggtttatatagcttgtgcgccgcctgggtacctcaggatatgcccttgactatttgtccgacatagtcaagggcatatccttttttgcggccgcatcgatgccgtagtacctttaagaccaatgacttacaaggcagctgtagatcttagccactttttaaaagaaaaggggggactggaagggctaattcactcccaaagaagacaagatccctgcaggcattcaaggccaggctggatgtggctctgggcagcctgggctgctggttgatgaccctgcacatagcagggggttggatctggatgagcactgtgctcctttgcaacccaggccgttctatgattctgtcattctaaatctctctttcagcctaaagctttttccccgtatccccccaggtgtctgcaggctcaaagagcagcgagaagcgttcagaggaaagcgatcccgtgccaccttccccgtgcccgggctgtccccgcacgctgccggctcggggatgcggggggagcgccggaccggagcggagccccgggcggctcgctgctgccccctagcgggggagggacgtaattacatccctgggggctttgggggggggctgtccccgtgagctccccagatctgctttttgcctgtactgggtctctctggttagaccagatctgagcctgggagctctctggctaactagggaacccactgcttaagcctcaataaagcttcagctgctcgagctagcagatctttttccctctgccaaaaattatggggacatcatgaagccccttgagcatctgacttctggctaataaaggaaatttattttcattgcaatagtgtgttggaattttttgtgtctctcactcggaaggacatatgggagggcaaatcatttaaaacatcagaatgagtatttggtttagagtttggcaacatatgcccatatgctggctgccatgaacaaaggttggctataaagaggtcatcagtatatgaaacagccccctgctgtccattccttattccatagaaaagccttgacttgaggttagattttttttatattttgttttgtgttatttttttctttaacatccctaaaattttccttacatgttttactagccagatttttcctcctctcctgactactcccagtcatagctgtccctcttctcttatggagatccctcgacctgcagcccaagcttggcgtaatcatggtcatagctgtttcctgtgtgaaattgttatccgctcacaattccacacaacatacgagccggaagcataaagtgtaaagcctggggtgcctaatgagtgagctaactcacattaattgcgttgcgctcactgcccgctttccagtcgggaaacctgtcgtgccagcggatccgcatctcaattagtcagcaaccatagtcccgcccctaactccgcccatcccgcccctaactccgcccagttccgcccattctccgccccatggctgactaattttttttatttatgcagaggccgaggccgcctcggcctctgagctattccagaagtagtgaggaggcttttttggaggcctaggcttttgcaaaaagctgtcgactgcagaggcctgcatgcaagcttggcgtaatcatggtcatagctgtttcctgtgtgaaattgttatccgctcacaattccacacaacatacgagccggaagcataaagtgtaaagcctggggtgcctaatgagtgagctaactcacattaattgcgttgcgctcactgcccgctttccagtcgggaaacctgtcgtgccagctgcattaatgaatcggccaacgcgcggggagaggcggtttgcgtattgggcgctcttccgcttcctcgctcactgactcgctgcgctcggtcgttcggctgcggcgagcggtatcagctcactcaaaggcggtaatacggttatccacagaatcaggggataacgcaggaaagaacatgtgagcaaaaggccagcaaaaggccaggaaccgtaaaaaggccgcgttgctggcgtttttccataggctccgcccccctgacgagcatcacaaaaatcgacgctcaagtcagaggtggcgaaacccgacaggactataaagataccaggcgtttccccctggaagctccctcgtgcgctctcctgttccgaccctgccgcttaccggatacctgtccgcctttctcccttcgggaagcgtggcgctttctcatagctcacgctgtaggtatctcagttcggtgtaggtcgttcgctccaagctgggctgtgtgcacgaaccccccgttcagcccgaccgctgcgccttatccggtaactatcgtcttgagtccaacccggtaagacacgacttatcgccactggcagcagccactggtaacaggattagcagagcgaggtatgtaggcggtgctacagagttcttgaagtggtggcctaactacggctacactagaagaacagtatttggtatctgcgctctgctgaagccagttaccttcggaaaaagagttggtagctcttgatccggcaaacaaaccaccgctggtagcggtggtttttttgtttgcaagcagcagattacgcgcagaaaaaaaggatctcaagaagatcctttgatcttttctacggggtctgacgctcagtggaacgaaaactcacgttaagggattttggtcatgagattatcaaaaaggatcttcacctagatccttttaaattaaaaatgaagttttaaatcaatctaaagtatatatgagtaaacttggtctgacagttaccaatgcttaatcagtgaggcacctatctcagcgatctgtctatttcgttcatccatagttgcctgactccccgtcgtgtagataactacgatacgggagggcttaccatctggccccagtgctgcaatgataccgcgagacccacgctcaccggctccagatttatcagcaataaaccagccagccggaagggccgagcgcagaagtggtcctgcaactttatccgcctccatccagtctattaattgttgccgggaagctagagtaagtagttcgccagttaatagtttgcgcaacgttgttgccattgctacaggcatcgtggtgtcacgctcgtcgtttggtatggcttcattcagctccggttcccaacgatcaaggcgagttacatgatcccccatgttgtgcaaaaaagcggttagctccttcggtcctccgatcgttgtcagaagtaagttggccgcagtgttatcactcatggttatggcagcactgcataattctcttactgtcatgccatccgtaagatgcttttctgtgactggtgagtactcaaccaagtcattctgagaatagtgtatgcggcgaccgagttgctcttgcccggcgtcaatacgggataataccgcgccacatagcagaactttaaaagtgctcatcattggaaaacgttcttcggggcgaaaactctcaaggatcttaccgctgttgagatccagttcgatgtaacccactcgtgcacccaactgatcttcagcatcttttactttcaccagcgtttctgggtgagcaaaaacaggaaggcaaaatgccgcaaaaaagggaataagggcgacacggaaatgttgaatactcatactcttcctttttcaatattattgaagcatttatcagggttattgtctcatgagcggatacatatttgaatgtatttagaaaaataaacaaataggggttccgcgcacatttccccgaaaagtgccacctgacgtctaagaaaccattattatcatgacattaacctataaaaataggcgtatcacgaggccctttcgtctcgcgcgtttcggtgatgacggtgaaaacctctgacacatgcagctcccggagacggtcacagcttgtctgtaagcggatgccgggagcagacaagcccgtcagggcgcgtcagcgggtgttggcgggtgtcggggctggcttaactatgcggcatcagagcagattgtactgagagtgcaccatatgcggtgtgaaataccgcacagatgcgtaaggagaaaataccgcatcaggcgccattcgccattcaggctgcgcaactgttgggaagggcgatcggtgcgggcctcttcgctattacgccagctggcgaaagggggatgtgctgcaaggcgattaagttgggtaacgccagggttttcccagtcacgacgttgtaaaacgacggccagtgaattc

SEQ ID NO: 10 - DNA, 12084 bp, Artificial Sequence
  Synthetic: TL20c-rGbGM-7SK/sh734
ggccgcctcggccaaacagcccttgagtttaccactccctatcagtgatagagaaaagtgaaagtcgagtttaccactccctatcagtgatagagaaaagtgaaagtcgagtttaccactccctatcagtgatagagaaaagtgaaagtcgagtttaccactccctatcagtgatagagaaaagtgaaagtcgagtttaccagtccctatcagtgatagagaaaagtgaaagtcgagtttaccactccctatcagtgatagagaaaagtgaaagtcgagtttaccactccctatcagtgatagagaaaagtgaaagtcgagctcgccatgggaggcgtggcctgggcgggactggggagtggcgagccctcagatcctgcatataagcagctgctttttgcctgtactgggtctctctggttagaccagatctgagcctgggagctctctggctaactagggaacccactgcttaagcctcaataaagcttgccttgagtgcttcaagtagtgtgtgcccgtctgttgtgtgactctggtaactagagatccctcagacccttttagtcagtgtggaaaatctctagcagtggcgcccgaacagggacttgaaagcgaaagggaaaccagaggagctctctcgacgcaggactcggcttgctgaagcgcgcacggcaagaggcgaggggcggcgactggtgagtacgccaaaaattttgactagcggaggctagaaggagagagatgggtgcgagagcgtcagtattaagcgggggagaattagatcgcgatgggaaaaaattcggttaaggccagggggaaagaaaaaatataaattaaaacatatagtatgggcaagcagggagctagaacgattcgcagttaatactggcctgttagaaacatcagaaggctgtagacaaatactgggacagctacaaccatcccttcagacaggatcagaagaacttagatcattatataatacagtagcaaccctctattgtgtgcatcaaaggatagagataaaagacaccaaggaagctttagacaagatagaggaagagcaaaacaaaagtaagaaaaaagcacagcaagcagcaggatcttcagacctggaaattccctacaatccccaaagtcaaggagtagtagaatctatgaataaagaattaaagaaaattataggacaggtaagagatcaggctgaacatcttaagacagcagtacaaatggcagtattcatccacaattttaaaagaaaaggggggattggggggtacagtgcaggggaaagaatagtagacataatagcaacagacatacaaactaaagaattacaaaaacaaattacaaaaattcaaaattttcgggtttattacagggacagcagaaatccactttggaaaggaccagcaaagctcctctggaaaggtgaaggggcagtagtaatacaagataatagtgacataaaagtagtgccaagaagaaaagcaaagatcattagggattatggaaaacagatggcaggtgatgattgtgtggcaagtagacaggatgaggattagaacatggaaaagtttagtaaaacaccataaggaggagatatgagggacaattggagaagtgaattatataaatataaagtagtaaaaattgaaccattaggagtagcacccaccaaggcaaagagaagagtggtgcagagagaaaaaagagcagtgggaataggagctttgttccttgggttcttgggagcagcaggaagcactatgggcgcagcgtcaatgacgctgacggtacaggccagacaattattgtctggtatagtgcagcagcagaacaatttgctgagggctattgaggcgcaacagcatctgttgcaactcacagtctggggcatcaagcagctccaggcaagaatcctggctgtggaaagatacctaaaggatcaacagctcctggggatttggggttgctctggaaaactcatttgcaccactgctgtgccttggaatgctagttggagtaataaatctctggaacagatttggaatcacacgacctggatggagtgggacagagaaattaacaattacacaagcttaatacactccttaattgaagaatcgcaaaaccagcaagaaaagaatgaacaagaattattggaattagataaatgggcaagtttgtggaattggtttaacataacaaattggctgtggtatataaaattattcataatgatagtaggaggcttggtaggtttaagaatagtttttgctgtactttctatagtgaatagagttaggcagggatattcaccattatcgtttcagacccacctcccaaccccgaggggaccgagctcaagcttcgaacgcgtggggatcctctagagtcgagctcgcgaggatcatcaccggtgctagccggagccagaagcaccataagggacatgataagggagccagcagacctctgatctcttcctgaatgctaatcttaaacatcctgaggaagaatgggacttccatttggggtgggcctatgatagggtaataagacagtagtgaatatcaagctacaaaaagccccctttcaaattcttctcagtcctaacttttcatactaagcccagtccttccaaagcagactgtgaaagagtgatagttccgggagactagcaccggctagccgagcttggaacactttcccttcattaagaaccatccttgctactcagctgcaatcaatccagcccccaggtcttcactgaaccttttcccatctcttccaaaacatctgtttctgagaagtcctgtcctatagaggtctttcttcccaccggatttctcctacaccatttactcccacttgcagaactcccgtgtacaagtgtctttactgcttttatttgctcaacaaaatgcacatctcatataaaaataaatgaggagcatgcacacaccacaaacacaaacaggcatgcagaaatacacatacacacttccctcaatataaaccctttgtggctcatatatttaaaaagatgtaaaaaaaagagctgaagaaaatcatgtgtgatctctcagcagaatagatttattatttgtattgcttgcagaataaagcctatccttgaaagctctgaatcatgggcaagaggctcagtggtatctggaggacagggcactggccactgcagtcaccatcttctgccaggaagcctgcacctcaggggtgaattctttgccaaagtgaatggccagcacggtgaccagcacgttgcccaggagctgtgggaggaagataagaggtatgaacatgattagcaaaagggcctagcttggactcagaataatccagccttatcccaaccataaaataaaagcagaatggtagctggattgtagctgctattagcaatatgaaacctcttacatcagttacaatttatatgcagaaatatttatatgcagaaatattgctattgccttaacccagaaattatcactgttattctttagaatggtgcaaagaggcatgatacattgtatcattattgccctgaaagaaagagattagggaaagtattagaaataagataaacaaaaaagtatattaaaagaagaaagcattttttaaaattacaaatgcaaaattaccctgatttggtcaatatgtgtaccctgttacttctccccttcctatgacatgaacttaaccatagaaaagaaggggaaagaaaacatcaagggtcccatagactcaccttgaagttctcaggatccacatgcagcttgtcacagtgcagttcactcagctgggcaaaggtgcccttgagatcatccaggtgctttatggcatctcccaaggaagtcagcaccttcttgccatgtgccttgactttggggttgcccatgatggcagaggcagaggacaggttgccaaagctgtcaaagaacctctgggtccatgggtagacaaccaggagcctgtgagattgacaagaacagtttgacagtcagaaggtgccacaaatcctgagaagcaacctggacttttgccaggcacagggtccttccttccctcccttgtcctggtcaccagagcctaccttcccagggtttctcctccagcatcttccacattcaccttgtcccacaggcttgtgatagtagccttgtcctcctctgtgaaatgacccatggtgtctgtttgaggttgctagtgaacacagttgtgtcagaagcaaatgtaagcaatagatggctctgccctgacttttatgcccagccctggctcctgccctccctgctcctgggagtagattggccaaccctagggtgtggctccacagggtgaggtctaagtgatgacagccgtacctgtccttggctcttctggcactggcttaggagttggacttcaaaccctcagccctccctctaagatatatctcttggccccataccatcagtacaaattgctactaaaaacatcctcctttgcaagtgtatttacgacggtatcgatgtatgtgagcatgtgtcctctaacagcacaggccttttgccacctagctgtccaggggtgccttaaaatggcaaacaaggtttgttttcttttcctgttttcatgccttcctcttccatatccttgtttcatattaatacatgtgtatagatcctaaaaatctatacacatgtattaataaagcctgattctgccgcttctaggtatagaggccacctgcaagataaatatttgattcacaataactaatcattctatggcaattgataacaacaaatatatatatatatatatatatacgtatatgtgtatatatatatatatattcaggaaataatatattctagaatatgtcacattctgtctcaggcatccattttctttatgatgccgtttgaggtggagttttagtcaggtggtcagcttctccttttttttgccatctgccctgtaagcatcctgctggggacccagataggagtcatcactctaggctgagaacatctgggcacacaccctaagcctcagcatgactcatcatgactcagcattgctgtgcttgagccagaaggtttgcttagaaggttacacagaaccagaaggcgggggtggggcactgaccccgacaggggcctggccagaactgctcatgcttggactatgggaggtcactaatggagacacacagaaatgtaacaggaactaagggaattccggtgccctgcttaggagcttaatctttaatgaaagctaagctttcattaaaaaaagtctaaccagctgcattcgactttgactgcagcagctggttagaaggttctactggaggagggtcccagcccattgctaaattaacatcaggctctgagactggcagtatatctctaacagtggttgatgctatcttctggaacttgcctgctacattgagaccactgacccatacataggaagcccatagctctgtcctgaactgttaggccactggtccagagagtgtgcatctcctttgatcctcataataaccctatgagatagacacaattattactcttactttatagatgatgatcctgaaaacataggagtcaaggcacttgcccctagctgggggtataggggagcagtcccatgtagtagtagaatgaaaaatgctgctatgctgtgcctcccccacctttcccatgtctgccctctactcatggtctatctctcctggctcctgggagtcatggactccacccagcaccaccaacctgacctaaccacctatctgagcctgccagcctataacccatctgggccctgatagctggtggccagccctgaccccaccccaccctccctggaacctctgatagacacatctggcacaccagctcgcaaagtcaccgtgagggtcttgtgtttgctgagtcaaaattccttgaaatccaagtccttagagactcctgctcccaaatttacagtcatagacttcttcatggctgtctcctttatccacagaatgattcctttgcttcattgccccatccatctgatcctcctcatcagtgcagcacagggcccatgagcagtagctgcagagtctcacataggtctggcactgcctctgacatgtccgaccttaggcaaatgcttgactcttctgagctcggatcccttgagctcaggaggtcaaggctgcagtgagacatgatcttgccactgcactccagcctggacagcagagtgaaaccttgcctcacgaaacagaatacaaaaacaaacaaacaaaaaactgctccgcaatgcgcttccttgatgctctaccacataggtctgggtactttgtacacattatctcattgctgttcataattgttagattaattttgtaatattgatattattcctagaaagctgaggcctcaagatgataacttttattttctggacttgtaatagctttctcttgtattcaccatgttgtaactttcttagagtagtaacaatataaagttattgtgagtttttgcaaacacagcaaacacaacgacccatatagacattgatgtgaaattgtctattgtcaatttatgggaaaacaagtatgtactttttctactaagccattgaaacaggaataacagaacaagattgaaagaatacattttccgaaattacttgagtattatacaaagacaagcacgtggacctgggaggagggttattgtccatgactggtgtgtggagacaaatgcaggtttataatagatgggatggcatctagcgcaatgactttgccatcacttttagagagctcttgggggccccagtacacaagaggggacgcagggtatatgtagacatctcattctttttcttagtgtgagaataagaatagccatgacctgagtttatagacaatgagcccttttctctctcccactcagcagctatgagatggcttgccctgcctctctactaggctgactcactccaaggcccagcaatgggcagggctctgtcagggctttgatagcactatctgcagagccagggccgagaaggggtggactccagagactctccctcccattcccgagcagggtttgcttatttatgcatttaaatgatatatttattttaaaagaaataacaggagactgcccagccctggctgtgacatggaaactatgtagaatattttgggttccatttttttttccttctttcagttagaggaaaaggggctcactgcacatacactagacagaaagtcaggagctttgaatccaagcctgatcatttccatgtcatactgagaaagtccccacccttctctgagcctcagtttctctttttataagtaggagtctggagtaaatgatttccaatggctctcatttcaatacaaaatttccgtttattaaatgcatgagcttccgttactccaagactgagaaggaaattgaacctgagactcattgactggcaagatgtccccagaggctctcattcagcaataaaattctcaccttcacccaggcccactagtgtcagatttgcatgcgttcgcgtatcgacgtgcagtatttagcatgccccacccatctgcaaggcattctggatagtgtcaaaacagccggaaatcaagtccgtttatctcaaactttagcattttgggaataaatgatatttgctatgctggttaaattagattttagttaaatttcctgctgaagctctagtacgataagtaacttgacctaagtgtaaagttgagatttccttcaggtttatatagcttgtgcgccgcctgggtacctcaggatatgcccttgactatttgtccgacatagtcaagggcatatccttttttgtgcggccgcatcgatgccgtagtacctttaagaccaatgacttacaaggcagctgtagatcttagccactttttaaaagaaaaggggggactggaagggctaattcactcccaaagaagacaagatccctgcaggcattcaaggccaggctggatgtggctctgggcagcctgggctgctggttgatgaccctgcacatagcagggggttggatctggatgagcactgtgctcctttgcaacccaggccgttctatgattctgtcattctaaatctctctttcagcctaaagctttttccccgtatccccccaggtgtctgcaggctcaaagagcagcgagaagcgttcagaggaaagcgatcccgtgccaccttccccgtgcccgggctgtccccgcacgctgccggctcggggatgcggggggagcgccggaccggagcggagccccgggcggctcgctgctgccccctagcgggggagggacgtaattacatccctgggggctttgggggggggctgtccccgtgagctccccagatctgctttttgcctgtactgggtctctctggttagaccagatctgagcctgggagctctctggctaactagggaacccactgcttaagcctcaataaagcttcagctgctcgagctagcagatctttttccctctgccaaaaattatggggacatcatgaagccccttgagcatctgacttctggctaataaaggaaatttattttcattgcaatagtgtgttggaattttttgtgtctctcactcggaaggacatatgggagggcaaatcatttaaaacatcagaatgagtatttggtttagagtttggcaacatatgcccatatgctggctgccatgaacaaaggttggctataaagaggtcatcagtatatgaaacagccccctgctgtccattccttattccatagaaaagccttgacttgaggttagattttttttatattttgttttgtgttatttttttctttaacatccctaaaattttccttacatgttttactagccagatttttcctcctctcctgactactcccagtcatagctgtccctcttctcttatggagatccctcgacctgcagcccaagcttggcgtaatcatggtcatagctgtttcctgtgtgaaattgttatccgctcacaattccacacaacatacgagccggaagcataaagtgtaaagcctggggtgcctaatgagtgagctaactcacattaattgcgttgcgctcactgcccgctttccagtcgggaaacctgtcgtgccagcggatccgcatctcaattagtcagcaaccatagtcccgcccctaactccgcccatcccgcccctaactccgcccagttccgcccattctccgccccatggctgactaattttttttatttatgcagaggccgaggccgcctcggcctctgagctattccagaagtagtgaggaggcttttttggaggcctaggcttttgcaaaaagctgtcgactgcagaggcctgcatgcaagcttggcgtaatcatggtcatagctgtttcctgtgtgaaattgttatccgctcacaattccacacaacatacgagccggaagcataaagtgtaaagcctggggtgcctaatgagtgagctaactcacattaattgcgttgcgctcactgcccgctttccagtcgggaaacctgtcgtgccagctgcattaatgaatcggccaacgcgcggggagaggcggtttgcgtattgggcgctcttccgcttcctcgctcactgactcgctgcgctcggtcgttcggctgcggcgagcggtatcagctcactcaaaggcggtaatacggttatccacagaatcaggggataacgcaggaaagaacatgtgagcaaaaggccagcaaaaggccaggaaccgtaaaaaggccgcgttgctggcgtttttccataggctccgcccccctgacgagcatcacaaaaatcgacgctcaagtcagaggtggcgaaacccgacaggactataaagataccaggcgtttccccctggaagctccctcgtgcgctctcctgttccgaccctgccgcttaccggatacctgtccgcctttctcccttcgggaagcgtggcgctttctcatagctcacgctgtaggtatctcagttcggtgtaggtcgttcgctccaagctgggctgtgtgcacgaaccccccgttcagcccgaccgctgcgccttatccggtaactatcgtcttgagtccaacccggtaagacacgacttatcgccactggcagcagccactggtaacaggattagcagagcgaggtatgtaggcggtgctacagagttcttgaagtggtggcctaactacggctacactagaagaacagtatttggtatctgcgctctgctgaagccagttaccttcggaaaaagagttggtagctcttgatccggcaaacaaaccaccgctggtagcggtggtttttttgtttgcaagcagcagattacgcgcagaaaaaaaggatctcaagaagatcctttgatcttttctacggggtctgacgctcagtggaacgaaaactcacgttaagggattttggtcatgagattatcaaaaaggatcttcacctagatccttttaaattaaaaatgaagttttaaatcaatctaaagtatatatgagtaaacttggtctgacagttaccaatgcttaatcagtgaggcacctatctcagcgatctgtctatttcgttcatccatagttgcctgactccccgtcgtgtagataactacgatacgggagggcttaccatctggccccagtgctgcaatgataccgcgagacccacgctcaccggctccagatttatcagcaataaaccagccagccggaagggccgagcgcagaagtggtcctgcaactttatccgcctccatccagtctattaattgttgccgggaagctagagtaagtagttcgccagttaatagtttgcgcaacgttgttgccattgctacaggcatcgtggtgtcacgctcgtcgtttggtatggcttcattcagctccggttcccaacgatcaaggcgagttacatgatcccccatgttgtgcaaaaaagcggttagctccttcggtcctccgatcgttgtcagaagtaagttggccgcagtgttatcactcatggttatggcagcactgcataattctcttactgtcatgccatccgtaagatgcttttctgtgactggtgagtactcaaccaagtcattctgagaatagtgtatgcggcgaccgagttgctcttgcccggcgtcaatacgggataataccgcgccacatagcagaactttaaaagtgctcatcattggaaaacgttcttcggggcgaaaactctcaaggatcttaccgctgttgagatccagttcgatgtaacccactcgtgcacccaactgatcttcagcatcttttactttcaccagcgtttctgggtgagcaaaaacaggaaggcaaaatgccgcaaaaaagggaataagggcgacacggaaatgttgaatactcatactcttcctttttcaatattattgaagcatttatcagggttattgtctcatgagcggatacatatttgaatgtatttagaaaaataaacaaataggggttccgcgcacatttccccgaaaagtgccacctgacgtctaagaaaccattattatcatgacattaacctataaaaataggcgtatcacgaggccctttcgtctcgcgcgtttcggtgatgacggtgaaaacctctgacacatgcagctcccggagacggtcacagcttgtctgtaagcggatgccgggagcagacaagcccgtcagggcgcgtcagcgggtgttggcgggtgtcggggctggcttaactatgcggcatcagagcagattgtactgagagtgcaccatatgcggtgtgaaataccgcacagatgcgtaaggagaaaataccgcatcaggcgccattcgccattcaggctgcgcaactgttgggaagggcgatcggtgcgggcctcttcgctattacgccagctggcgaaagggggatgtgctgcaaggcgattaagttgggtaacgccagggttttcccagtcacgacgttgtaaaacgacggccagtgaattc

SEQ ID NO: 11 - DNA, 12081 bp, Artificial Sequence
  Synthetic: TL20c-rGbGM-r7SKM1/sh734
ggccgcctcggccaaacagcccttgagtttaccactccctatcagtgatagagaaaagtgaaagtcgagtttaccactccctatcagtgatagagaaaagtgaaagtcgagtttaccactccctatcagtgatagagaaaagtgaaagtcgagtttaccactccctatcagtgatagagaaaagtgaaagtcgagtttaccagtccctatcagtgatagagaaaagtgaaagtcgagtttaccactccctatcagtgatagagaaaagtgaaagtcgagtttaccactccctatcagtgatagagaaaagtgaaagtcgagctcgccatgggaggcgtggcctgggcgggactggggagtggcgagccctcagatcctgcatataagcagctgctttttgcctgtactgggtctctctggttagaccagatctgagcctgggagctctctggctaactagggaacccactgcttaagcctcaataaagcttgccttgagtgcttcaagtagtgtgtgcccgtctgttgtgtgactctggtaactagagatccctcagacccttttagtcagtgtggaaaatctctagcagtggcgcccgaacagggacttgaaagcgaaagggaaaccagaggagctctctcgacgcaggactcggcttgctgaagcgcgcacggcaagaggcgaggggcggcgactggtgagtacgccaaaaattttgactagcggaggctagaaggagagagatgggtgcgagagcgtcagtattaagcgggggagaattagatcgcgatgggaaaaaattcggttaaggccagggggaaagaaaaaatataaattaaaacatatagtatgggcaagcagggagctagaacgattcgcagttaatactggcctgttagaaacatcagaaggctgtagacaaatactgggacagctacaaccatcccttcagacaggatcagaagaacttagatcattatataatacagtagcaaccctctattgtgtgcatcaaaggatagagataaaagacaccaaggaagctttagacaagatagaggaagagcaaaacaaaagtaagaaaaaagcacagcaagcagcaggatcttcagacctggaaattccctacaatccccaaagtcaaggagtagtagaatctatgaataaagaattaaagaaaattataggacaggtaagagatcaggctgaacatcttaagacagcagtacaaatggcagtattcatccacaattttaaaagaaaaggggggattggggggtacagtgcaggggaaagaatagtagacataatagcaacagacatacaaactaaagaattacaaaaacaaattacaaaaattcaaaattttcgggtttattacagggacagcagaaatccactttggaaaggaccagcaaagctcctctggaaaggtgaaggggcagtagtaatacaagataatagtgacataaaagtagtgccaagaagaaaagcaaagatcattagggattatggaaaacagatggcaggtgatgattgtgtggcaagtagacaggatgaggattagaacatggaaaagtttagtaaaacaccataaggaggagatatgagggacaattggagaagtgaattatataaatataaagtagtaaaaattgaaccattaggagtagcacccaccaaggcaaagagaagagtggtgcagagagaaaaaagagcagtgggaataggagctttgttccttgggttcttgggagcagcaggaagcactatgggcgcagcgtcaatgacgctgacggtacaggccagacaattattgtctggtatagtgcagcagcagaacaatttgctgagggctattgaggcgcaacagcatctgttgcaactcacagtctggggcatcaagcagctccaggcaagaatcctggctgtggaaagatacctaaaggatcaacagctcctggggatttggggttgctctggaaaactcatttgcaccactgctgtgccttggaatgctagttggagtaataaatctctggaacagatttggaatcacacgacctggatggagtgggacagagaaattaacaattacacaagcttaatacactccttaattgaagaatcgcaaaaccagcaagaaaagaatgaacaagaattattggaattagataaatgggcaagtttgtggaattggtttaacataacaaattggctgtggtatataaaattattcataatgatagtaggaggcttggtaggtttaagaatagtttttgctgtactttctatagtgaatagagttaggcagggatattcaccattatcgtttcagacccacctcccaaccccgaggggaccgagctcaagcttcgaacgcgtggggatcctctagagtcgagctcgcgaggatcatcaccggtgctagccggagccagaagcaccataagggacatgataagggagccagcagacctctgatctcttcctgaatgctaatcttaaacatcctgaggaagaatgggacttccatttggggtgggcctatgatagggtaataagacagtagtgaatatcaagctacaaaaagccccctttcaaattcttctcagtcctaacttttcatactaagcccagtccttccaaagcagactgtgaaagagtgatagttccgggagactagcaccggctagccgagcttggaacactttcccttcattaagaaccatccttgctactcagctgcaatcaatccagcccccaggtcttcactgaaccttttcccatctcttccaaaacatctgtttctgagaagtcctgtcctatagaggtctttcttcccaccggatttctcctacaccatttactcccacttgcagaactcccgtgtacaagtgtctttactgcttttatttgctcaacaaaatgcacatctcatataaaaataaatgaggagcatgcacacaccacaaacacaaacaggcatgcagaaatacacatacacacttccctcaatataaaccctttgtggctcatatatttaaaaagatgtaaaaaaaagagctgaagaaaatcatgtgtgatctctcagcagaatagatttattatttgtattgcttgcagaataaagcctatccttgaaagctctgaatcatgggcaagaggctcagtggtatctggaggacagggcactggccactgcagtcaccatcttctgccaggaagcctgcacctcaggggtgaattctttgccaaagtgaatggccagcacggtgaccagcacgttgcccaggagctgtgggaggaagataagaggtatgaacatgattagcaaaagggcctagcttggactcagaataatccagccttatcccaaccataaaataaaagcagaatggtagctggattgtagctgctattagcaatatgaaacctcttacatcagttacaatttatatgcagaaatatttatatgcagaaatattgctattgccttaacccagaaattatcactgttattctttagaatggtgcaaagaggcatgatacattgtatcattattgccctgaaagaaagagattagggaaagtattagaaataagataaacaaaaaagtatattaaaagaagaaagcattttttaaaattacaaatgcaaaattaccctgatttggtcaatatgtgtaccctgttacttctccccttcctatgacatgaacttaaccatagaaaagaaggggaaagaaaacatcaagggtcccatagactcaccttgaagttctcaggatccacatgcagcttgtcacagtgcagttcactcagctgggcaaaggtgcccttgagatcatccaggtgctttatggcatctcccaaggaagtcagcaccttcttgccatgtgccttgactttggggttgcccatgatggcagaggcagaggacaggttgccaaagctgtcaaagaacctctgggtccatgggtagacaaccaggagcctgtgagattgacaagaacagtttgacagtcagaaggtgccacaaatcctgagaagcaacctggacttttgccaggcacagggtccttccttccctcccttgtcctggtcaccagagcctaccttcccagggtttctcctccagcatcttccacattcaccttgtcccacaggcttgtgatagtagccttgtcctcctctgtgaaatgacccatggtgtctgtttgaggttgctagtgaacacagttgtgtcagaagcaaatgtaagcaatagatggctctgccctgacttttatgcccagccctggctcctgccctccctgctcctgggagtagattggccaaccctagggtgtggctccacagggtgaggtctaagtgatgacagccgtacctgtccttggctcttctggcactggcttaggagttggacttcaaaccctcagccctccctctaagatatatctcttggccccataccatcagtacaaattgctactaaaaacatcctcctttgcaagtgtatttacgacggtatcgatgtatgtgagcatgtgtcctctaacagcacaggccttttgccacctagctgtccaggggtgccttaaaatggcaaacaaggtttgttttcttttcctgttttcatgccttcctcttccatatccttgtttcatattaatacatgtgtatagatcctaaaaatctatacacatgtattaataaagcctgattctgccgcttctaggtatagaggccacctgcaagataaatatttgattcacaataactaatcattctatggcaattgataacaacaaatatatatatatatatatatatacgtatatgtgtatatatatatatatattcaggaaataatatattctagaatatgtcacattctgtctcaggcatccattttctttatgatgccgtttgaggtggagttttagtcaggtggtcagcttctccttttttttgccatctgccctgtaagcatcctgctggggacccagataggagtcatcactctaggctgagaacatctgggcacacaccctaagcctcagcatgactcatcatgactcagcattgctgtgcttgagccagaaggtttgcttagaaggttacacagaaccagaaggcgggggtggggcactgaccccgacaggggcctggccagaactgctcatgcttggactatgggaggtcactaatggagacacacagaaatgtaacaggaactaagggaattccggtgccctgcttaggagcttaatctttaatgaaagctaagctttcattaaaaaaagtctaaccagctgcattcgactttgactgcagcagctggttagaaggttctactggaggagggtcccagcccattgctaaattaacatcaggctctgagactggcagtatatctctaacagtggttgatgctatcttctggaacttgcctgctacattgagaccactgacccatacataggaagcccatagctctgtcctgaactgttaggccactggtccagagagtgtgcatctcctttgatcctcataataaccctatgagatagacacaattattactcttactttatagatgatgatcctgaaaacataggagtcaaggcacttgcccctagctgggggtataggggagcagtcccatgtagtagtagaatgaaaaatgctgctatgctgtgcctcccccacctttcccatgtctgccctctactcatggtctatctctcctggctcctgggagtcatggactccacccagcaccaccaacctgacctaaccacctatctgagcctgccagcctataacccatctgggccctgatagctggtggccagccctgaccccaccccaccctccctggaacctctgatagacacatctggcacaccagctcgcaaagtcaccgtgagggtcttgtgtttgctgagtcaaaattccttgaaatccaagtccttagagactcctgctcccaaatttacagtcatagacttcttcatggctgtctcctttatccacagaatgattcctttgcttcattgccccatccatctgatcctcctcatcagtgcagcacagggcccatgagcagtagctgcagagtctcacataggtctggcactgcctctgacatgtccgaccttaggcaaatgcttgactcttctgagctcggatcccttgagctcaggaggtcaaggctgcagtgagacatgatcttgccactgcactccagcctggacagcagagtgaaaccttgcctcacgaaacagaatacaaaaacaaacaaacaaaaaactgctccgcaatgcgcttccttgatgctctaccacataggtctgggtactttgtacacattatctcattgctgttcataattgttagattaattttgtaatattgatattattcctagaaagctgaggcctcaagatgataacttttattttctggacttgtaatagctttctcttgtattcaccatgttgtaactttcttagagtagtaacaatataaagttattgtgagtttttgcaaacacagcaaacacaacgacccatatagacattgatgtgaaattgtctattgtcaatttatgggaaaacaagtatgtactttttctactaagccattgaaacaggaataacagaacaagattgaaagaatacattttccgaaattacttgagtattatacaaagacaagcacgtggacctgggaggagggttattgtccatgactggtgtgtggagacaaatgcaggtttataatagatgggatggcatctagcgcaatgactttgccatcacttttagagagctcttgggggccccagtacacaagaggggacgcagggtatatgtagacatctcattctttttcttagtgtgagaataagaatagccatgacctgagtttatagacaatgagcccttttctctctcccactcagcagctatgagatggcttgccctgcctctctactaggctgactcactccaaggcccagcaatgggcagggctctgtcagggctttgatagcactatctgcagagccagggccgagaaggggtggactccagagactctccctcccattcccgagcagggtttgcttatttatgcatttaaatgatatatttattttaaaagaaataacaggagactgcccagccctggctgtgacatggaaactatgtagaatattttgggttccatttttttttccttctttcagttagaggaaaaggggctcactgcacatacactagacagaaagtcaggagctttgaatccaagcctgatcatttccatgtcatactgagaaagtccccacccttctctgagcctcagtttctctttttataagtaggagtctggagtaaatgatttccaatggctctcatttcaatacaaaatttccgtttattaaatgcatgagcttccgttactccaagactgagaaggaaattgaacctgagactcattgactggcaagatgtccccagaggctctcattcagcaataaaattctcaccttcacccaggcccactagtgtcagatttgcatgcgttcgcgtaaaaaaggatatgcccttgactatgtcggacaaatagtcaagggcatatcctgaggtacccaggcggcgcacaagctatataaacctgaaggaaatctcaactttacacttaggtcaagttacttatcgtactagagcttcagcaggaaatttaactaaaatctaatttaaccagcatagcaaatatcatttattcccaaaatgctaaagtttgagataaacggacttgatttccggctgttttgacactatccagaatgccggtactatgggtggggcagtagcccgactgcacgtcgagcggccgcatcgatgccgtagtacctttaagaccaatgacttacaaggcagctgtagatcttagccactttttaaaagaaaaggggggactggaagggctaattcactcccaaagaagacaagatccctgcaggcattcaaggccaggctggatgtggctctgggcagcctgggctgctggttgatgaccctgcacatagcagggggttggatctggatgagcactgtgctcctttgcaacccaggccgttctatgattctgtcattctaaatctctctttcagcctaaagctttttccccgtatccccccaggtgtctgcaggctcaaagagcagcgagaagcgttcagaggaaagcgatcccgtgccaccttccccgtgcccgggctgtccccgcacgctgccggctcggggatgcggggggagcgccggaccggagcggagccccgggcggctcgctgctgccccctagcgggggagggacgtaattacatccctgggggctttgggggggggctgtccccgtgagctccccagatctgctttttgcctgtactgggtctctctggttagaccagatctgagcctgggagctctctggctaactagggaacccactgcttaagcctcaataaagcttcagctgctcgagctagcagatctttttccctctgccaaaaattatggggacatcatgaagccccttgagcatctgacttctggctaataaaggaaatttattttcattgcaatagtgtgttggaattttttgtgtctctcactcggaaggacatatgggagggcaaatcatttaaaacatcagaatgagtatttggtttagagtttggcaacatatgcccatatgctggctgccatgaacaaaggttggctataaagaggtcatcagtatatgaaacagccccctgctgtccattccttattccatagaaaagccttgacttgaggttagattttttttatattttgttttgtgttatttttttctttaacatccctaaaattttccttacatgttttactagccagatttttcctcctctcctgactactcccagtcatagctgtccctcttctcttatggagatccctcgacctgcagcccaagcttggcgtaatcatggtcatagctgtttcctgtgtgaaattgttatccgctcacaattccacacaacatacgagccggaagcataaagtgtaaagcctggggtgcctaatgagtgagctaactcacattaattgcgttgcgctcactgcccgctttccagtcgggaaacctgtcgtgccagcggatccgcatctcaattagtcagcaaccatagtcccgcccctaactccgcccatcccgcccctaactccgcccagttccgcccattctccgccccatggctgactaattttttttatttatgcagaggccgaggccgcctcggcctctgagctattccagaagtagtgaggaggcttttttggaggcctaggcttttgcaaaaagctgtcgactgcagaggcctgcatgcaagcttggcgtaatcatggtcatagctgtttcctgtgtgaaattgttatccgctcacaattccacacaacatacgagccggaagcataaagtgtaaagcctggggtgcctaatgagtgagctaactcacattaattgcgttgcgctcactgcccgctttccagtcgggaaacctgtcgtgccagctgcattaatgaatcggccaacgcgcggggagaggcggtttgcgtattgggcgctcttccgcttcctcgctcactgactcgctgcgctcggtcgttcggctgcggcgagcggtatcagctcactcaaaggcggtaatacggttatccacagaatcaggggataacgcaggaaagaacatgtgagcaaaaggccagcaaaaggccaggaaccgtaaaaaggccgcgttgctggcgtttttccataggctccgcccccctgacgagcatcacaaaaatcgacgctcaagtcagaggtggcgaaacccgacaggactataaagataccaggcgtttccccctggaagctccctcgtgcgctctcctgttccgaccctgccgcttaccggatacctgtccgcctttctcccttcgggaagcgtggcgctttctcatagctcacgctgtaggtatctcagttcggtgtaggtcgttcgctccaagctgggctgtgtgcacgaaccccccgttcagcccgaccgctgcgccttatccggtaactatcgtcttgagtccaacccggtaagacacgacttatcgccactggcagcagccactggtaacaggattagcagagcgaggtatgtaggcggtgctacagagttcttgaagtggtggcctaactacggctacactagaagaacagtatttggtatctgcgctctgctgaagccagttaccttcggaaaaagagttggtagctcttgatccggcaaacaaaccaccgctggtagcggtggtttttttgtttgcaagcagcagattacgcgcagaaaaaaaggatctcaagaagatcctttgatcttttctacggggtctgacgctcagtggaacgaaaactcacgttaagggattttggtcatgagattatcaaaaaggatcttcacctagatccttttaaattaaaaatgaagttttaaatcaatctaaagtatatatgagtaaacttggtctgacagttaccaatgcttaatcagtgaggcacctatctcagcgatctgtctatttcgttcatccatagttgcctgactccccgtcgtgtagataactacgatacgggagggcttaccatctggccccagtgctgcaatgataccgcgagacccacgctcaccggctccagatttatcagcaataaaccagccagccggaagggccgagcgcagaagtggtcctgcaactttatccgcctccatccagtctattaattgttgccgggaagctagagtaagtagttcgccagttaatagtttgcgcaacgttgttgccattgctacaggcatcgtggtgtcacgctcgtcgtttggtatggcttcattcagctccggttcccaacgatcaaggcgagttacatgatcccccatgttgtgcaaaaaagcggttagctccttcggtcctccgatcgttgtcagaagtaagttggccgcagtgttatcactcatggttatggcagcactgcataattctcttactgtcatgccatccgtaagatgcttttctgtgactggtgagtactcaaccaagtcattctgagaatagtgtatgcggcgaccgagttgctcttgcccggcgtcaatacgggataataccgcgccacatagcagaactttaaaagtgctcatcattggaaaacgttcttcggggcgaaaactctcaaggatcttaccgctgttgagatccagttcgatgtaacccactcgtgcacccaactgatcttcagcatcttttactttcaccagcgtttctgggtgagcaaaaacaggaaggcaaaatgccgcaaaaaagggaataagggcgacacggaaatgttgaatactcatactcttcctttttcaatattattgaagcatttatcagggttattgtctcatgagcggatacatatttgaatgtatttagaaaaataaacaaataggggttccgcgcacatttccccgaaaagtgccacctgacgtctaagaaaccattattatcatgacattaacctataaaaataggcgtatcacgaggccctttcgtctcgcgcgtttcggtgatgacggtgaaaacctctgacacatgcagctcccggagacggtcacagcttgtctgtaagcggatgccgggagcagacaagcccgtcagggcgcgtcagcgggtgttggcgggtgtcggggctggcttaactatgcggcatcagagcagattgtactgagagtgcaccatatgcggtgtgaaataccgcacagatgcgtaaggagaaaataccgcatcaggcgccattcgccattcaggctgcgcaactgttgggaagggcgatcggtgcgggcctcttcgctattacgccagctggcgaaagggggatgtgctgcaaggcgattaagttgggtaacgccagggttttcccagtcacgacgttgtaaaacgacggccagtgaattc

SEQ ID NO: 12 - DNA, 12084 bp, Artificial Sequence
  Synthetic: TL20c-rGbGM-r7SK/sh734
ggccgcctcggccaaacagcccttgagtttaccactccctatcagtgatagagaaaagtgaaagtcgagtttaccactccctatcagtgatagagaaaagtgaaagtcgagtttaccactccctatcagtgatagagaaaagtgaaagtcgagtttaccactccctatcagtgatagagaaaagtgaaagtcgagtttaccagtccctatcagtgatagagaaaagtgaaagtcgagtttaccactccctatcagtgatagagaaaagtgaaagtcgagtttaccactccctatcagtgatagagaaaagtgaaagtcgagctcgccatgggaggcgtggcctgggcgggactggggagtggcgagccctcagatcctgcatataagcagctgctttttgcctgtactgggtctctctggttagaccagatctgagcctgggagctctctggctaactagggaacccactgcttaagcctcaataaagcttgccttgagtgcttcaagtagtgtgtgcccgtctgttgtgtgactctggtaactagagatccctcagacccttttagtcagtgtggaaaatctctagcagtggcgcccgaacagggacttgaaagcgaaagggaaaccagaggagctctctcgacgcaggactcggcttgctgaagcgcgcacggcaagaggcgaggggcggcgactggtgagtacgccaaaaattttgactagcggaggctagaaggagagagatgggtgcgagagcgtcagtattaagcgggggagaattagatcgcgatgggaaaaaattcggttaaggccagggggaaagaaaaaatataaattaaaacatatagtatgggcaagcagggagctagaacgattcgcagttaatactggcctgttagaaacatcagaaggctgtagacaaatactgggacagctacaaccatcccttcagacaggatcagaagaacttagatcattatataatacagtagcaaccctctattgtgtgcatcaaaggatagagataaaagacaccaaggaagctttagacaagatagaggaagagcaaaacaaaagtaagaaaaaagcacagcaagcagcaggatcttcagacctggaaattccctacaatccccaaagtcaaggagtagtagaatctatgaataaagaattaaagaaaattataggacaggtaagagatcaggctgaacatcttaagacagcagtacaaatggcagtattcatccacaattttaaaagaaaaggggggattggggggtacagtgcaggggaaagaatagtagacataatagcaacagacatacaaactaaagaattacaaaaacaaattacaaaaattcaaaattttcgggtttattacagggacagcagaaatccactttggaaaggaccagcaaagctcctctggaaaggtgaaggggcagtagtaatacaagataatagtgacataaaagtagtgccaagaagaaaagcaaagatcattagggattatggaaaacagatggcaggtgatgattgtgtggcaagtagacaggatgaggattagaacatggaaaagtttagtaaaacaccataaggaggagatatgagggacaattggagaagtgaattatataaatataaagtagtaaaaattgaaccattaggagtagcacccaccaaggcaaagagaagagtggtgcagagagaaaaaagagcagtgggaataggagctttgttccttgggttcttgggagcagcaggaagcactatgggcgcagcgtcaatgacgctgacggtacaggccagacaattattgtctggtatagtgcagcagcagaacaatttgctgagggctattgaggcgcaacagcatctgttgcaactcacagtctggggcatcaagcagctccaggcaagaatcctggctgtggaaagatacctaaaggatcaacagctcctggggatttggggttgctctggaaaactcatttgcaccactgctgtgccttggaatgctagttggagtaataaatctctggaacagatttggaatcacacgacctggatggagtgggacagagaaattaacaattacacaagcttaatacactccttaattgaagaatcgcaaaaccagcaagaaaagaatgaacaagaattattggaattagataaatgggcaagtttgtggaattggtttaacataacaaattggctgtggtatataaaattattcataatgatagtaggaggcttggtaggtttaagaatagtttttgctgtactttctatagtgaatagagttaggcagggatattcaccattatcgtttcagacccacctcccaaccccgaggggaccgagctcaagcttcgaacgcgtggggatcctctagagtcgagctcgcgaggatcatcaccggtgctagccggagccagaagcaccataagggacatgataagggagccagcagacctctgatctcttcctgaatgctaatcttaaacatcctgaggaagaatgggacttccatttggggtgggcctatgatagggtaataagacagtagtgaatatcaagctacaaaaagccccctttcaaattcttctcagtcctaacttttcatactaagcccagtccttccaaagcagactgtgaaagagtgatagttccgggagactagcaccggctagccgagcttggaacactttcccttcattaagaaccatccttgctactcagctgcaatcaatccagcccccaggtcttcactgaaccttttcccatctcttccaaaacatctgtttctgagaagtcctgtcctatagaggtctttcttcccaccggatttctcctacaccatttactcccacttgcagaactcccgtgtacaagtgtctttactgcttttatttgctcaacaaaatgcacatctcatataaaaataaatgaggagcatgcacacaccacaaacacaaacaggcatgcagaaatacacatacacacttccctcaatataaaccctttgtggctcatatatttaaaaagatgtaaaaaaaagagctgaagaaaatcatgtgtgatctctcagcagaatagatttattatttgtattgcttgcagaataaagcctatccttgaaagctctgaatcatgggcaagaggctcagtggtatctggaggacagggcactggccactgcagtcaccatcttctgccaggaagcctgcacctcaggggtgaattctttgccaaagtgaatggccagcacggtgaccagcacgttgcccaggagctgtgggaggaagataagaggtatgaacatgattagcaaaagggcctagcttggactcagaataatccagccttatcccaaccataaaataaaagcagaatggtagctggattgtagctgctattagcaatatgaaacctcttacatcagttacaatttatatgcagaaatatttatatgcagaaatattgctattgccttaacccagaaattatcactgttattctttagaatggtgcaaagaggcatgatacattgtatcattattgccctgaaagaaagagattagggaaagtattagaaataagataaacaaaaaagtatattaaaagaagaaagcattttttaaaattacaaatgcaaaattaccctgatttggtcaatatgtgtaccctgttacttctccccttcctatgacatgaacttaaccatagaaaagaaggggaaagaaaacatcaagggtcccatagactcaccttgaagttctcaggatccacatgcagcttgtcacagtgcagttcactcagctgggcaaaggtgcccttgagatcatccaggtgctttatggcatctcccaaggaagtcagcaccttcttgccatgtgccttgactttggggttgcccatgatggcagaggcagaggacaggttgccaaagctgtcaaagaacctctgggtccatgggtagacaaccaggagcctgtgagattgacaagaacagtttgacagtcagaaggtgccacaaatcctgagaagcaacctggacttttgccaggcacagggtccttccttccctcccttgtcctggtcaccagagcctaccttcccagggtttctcctccagcatcttccacattcaccttgtcccacaggcttgtgatagtagccttgtcctcctctgtgaaatgacccatggtgtctgtttgaggttgctagtgaacacagttgtgtcagaagcaaatgtaagcaatagatggctctgccctgacttttatgcccagccctggctcctgccctccctgctcctgggagtagattggccaaccctagggtgtggctccacagggtgaggtctaagtgatgacagccgtacctgtccttggctcttctggcactggcttaggagttggacttcaaaccctcagccctccctctaagatatatctcttggccccataccatcagtacaaattgctactaaaaacatcctcctttgcaagtgtatttacgacggtatcgatgtatgtgagcatgtgtcctctaacagcacaggccttttgccacctagctgtccaggggtgccttaaaatggcaaacaaggtttgttttcttttcctgttttcatgccttcctcttccatatccttgtttcatattaatacatgtgtatagatcctaaaaatctatacacatgtattaataaagcctgattctgccgcttctaggtatagaggccacctgcaagataaatatttgattcacaataactaatcattctatggcaattgataacaacaaatatatatatatatatatatatacgtatatgtgtatatatatatatatattcaggaaataatatattctagaatatgtcacattctgtctcaggcatccattttctttatgatgccgtttgaggtggagttttagtcaggtggtcagcttctccttttttttgccatctgccctgtaagcatcctgctggggacccagataggagtcatcactctaggctgagaacatctgggcacacaccctaagcctcagcatgactcatcatgactcagcattgctgtgcttgagccagaaggtttgcttagaaggttacacagaaccagaaggcgggggtggggcactgaccccgacaggggcctggccagaactgctcatgcttggactatgggaggtcactaatggagacacacagaaatgtaacaggaactaagggaattccggtgccctgcttaggagcttaatctttaatgaaagctaagctttcattaaaaaaagtctaaccagctgcattcgactttgactgcagcagctggttagaaggttctactggaggagggtcccagcccattgctaaattaacatcaggctctgagactggcagtatatctctaacagtggttgatgctatcttctggaacttgcctgctacattgagaccactgacccatacataggaagcccatagctctgtcctgaactgttaggccactggtccagagagtgtgcatctcctttgatcctcataataaccctatgagatagacacaattattactcttactttatagatgatgatcctgaaaacataggagtcaaggcacttgcccctagctgggggtataggggagcagtcccatgtagtagtagaatgaaaaatgctgctatgctgtgcctcccccacctttcccatgtctgccctctactcatggtctatctctcctggctcctgggagtcatggactccacccagcaccaccaacctgacctaaccacctatctgagcctgccagcctataacccatctgggccctgatagctggtggccagccctgaccccaccccaccctccctggaacctctgatagacacatctggcacaccagctcgcaaagtcaccgtgagggtcttgtgtttgctgagtcaaaattccttgaaatccaagtccttagagactcctgctcccaaatttacagtcatagacttcttcatggctgtctcctttatccacagaatgattcctttgcttcattgccccatccatctgatcctcctcatcagtgcagcacagggcccatgagcagtagctgcagagtctcacataggtctggcactgcctctgacatgtccgaccttaggcaaatgcttgactcttctgagctcggatcccttgagctcaggaggtcaaggctgcagtgagacatgatcttgccactgcactccagcctggacagcagagtgaaaccttgcctcacgaaacagaatacaaaaacaaacaaacaaaaaactgctccgcaatgcgcttccttgatgctctaccacataggtctgggtactttgtacacattatctcattgctgttcataattgttagattaattttgtaatattgatattattcctagaaagctgaggcctcaagatgataacttttattttctggacttgtaatagctttctcttgtattcaccatgttgtaactttcttagagtagtaacaatataaagttattgtgagtttttgcaaacacagcaaacacaacgacccatatagacattgatgtgaaattgtctattgtcaatttatgggaaaacaagtatgtactttttctactaagccattgaaacaggaataacagaacaagattgaaagaatacattttccgaaattacttgagtattatacaaagacaagcacgtggacctgggaggagggttattgtccatgactggtgtgtggagacaaatgcaggtttataatagatgggatggcatctagcgcaatgactttgccatcacttttagagagctcttgggggccccagtacacaagaggggacgcagggtatatgtagacatctcattctttttcttagtgtgagaataagaatagccatgacctgagtttatagacaatgagcccttttctctctcccactcagcagctatgagatggcttgccctgcctctctactaggctgactcactccaaggcccagcaatgggcagggctctgtcagggctttgatagcactatctgcagagccagggccgagaaggggtggactccagagactctccctcccattcccgagcagggtttgcttatttatgcatttaaatgatatatttattttaaaagaaataacaggagactgcccagccctggctgtgacatggaaactatgtagaatattttgggttccatttttttttccttctttcagttagaggaaaaggggctcactgcacatacactagacagaaagtcaggagctttgaatccaagcctgatcatttccatgtcatactgagaaagtccccacccttctctgagcctcagtttctctttttataagtaggagtctggagtaaatgatttccaatggctctcatttcaatacaaaatttccgtttattaaatgcatgagcttccgttactccaagactgagaaggaaattgaacctgagactcattgactggcaagatgtccccagaggctctcattcagcaataaaattctcaccttcacccaggcccactagtgtcagatttgcatgcgttcgcgtacaaaaaaggatatgcccttgactatgtcggacaaatagtcaagggcatatcctgaggtacccaggcggcgcacaagctatataaacctgaaggaaatctcaactttacacttaggtcaagttacttatcgtactagagcttcagcaggaaatttaactaaaatctaatttaaccagcatagcaaatatcatttattcccaaaatgctaaagtttgagataaacggacttgatttccggctgttttgacactatccagaatgccttgcagatgggtggggcatgctaaatactgcacgtcgatgcggccgcatcgatgccgtagtacctttaagaccaatgacttacaaggcagctgtagatcttagccactttttaaaagaaaaggggggactggaagggctaattcactcccaaagaagacaagatccctgcaggcattcaaggccaggctggatgtggctctgggcagcctgggctgctggttgatgaccctgcacatagcagggggttggatctggatgagcactgtgctcctttgcaacccaggccgttctatgattctgtcattctaaatctctctttcagcctaaagctttttccccgtatccccccaggtgtctgcaggctcaaagagcagcgagaagcgttcagaggaaagcgatcccgtgccaccttccccgtgcccgggctgtccccgcacgctgccggctcggggatgcggggggagcgccggaccggagcggagccccgggcggctcgctgctgccccctagcgggggagggacgtaattacatccctgggggctttgggggggggctgtccccgtgagctccccagatctgctttttgcctgtactgggtctctctggttagaccagatctgagcctgggagctctctggctaactagggaacccactgcttaagcctcaataaagcttcagctgctcgagctagcagatctttttccctctgccaaaaattatggggacatcatgaagccccttgagcatctgacttctggctaataaaggaaatttattttcattgcaatagtgtgttggaattttttgtgtctctcactcggaaggacatatgggagggcaaatcatttaaaacatcagaatgagtatttggtttagagtttggcaacatatgcccatatgctggctgccatgaacaaaggttggctataaagaggtcatcagtatatgaaacagccccctgctgtccattccttattccatagaaaagccttgacttgaggttagattttttttatattttgttttgtgttatttttttctttaacatccctaaaattttccttacatgttttactagccagatttttcctcctctcctgactactcccagtcatagctgtccctcttctcttatggagatccctcgacctgcagcccaagcttggcgtaatcatggtcatagctgtttcctgtgtgaaattgttatccgctcacaattccacacaacatacgagccggaagcataaagtgtaaagcctggggtgcctaatgagtgagctaactcacattaattgcgttgcgctcactgcccgctttccagtcgggaaacctgtcgtgccagcggatccgcatctcaattagtcagcaaccatagtcccgcccctaactccgcccatcccgcccctaactccgcccagttccgcccattctccgccccatggctgactaattttttttatttatgcagaggccgaggccgcctcggcctctgagctattccagaagtagtgaggaggcttttttggaggcctaggcttttgcaaaaagctgtcgactgcagaggcctgcatgcaagcttggcgtaatcatggtcatagctgtttcctgtgtgaaattgttatccgctcacaattccacacaacatacgagccggaagcataaagtgtaaagcctggggtgcctaatgagtgagctaactcacattaattgcgttgcgctcactgcccgctttccagtcgggaaacctgtcgtgccagctgcattaatgaatcggccaacgcgcggggagaggcggtttgcgtattgggcgctcttccgcttcctcgctcactgactcgctgcgctcggtcgttcggctgcggcgagcggtatcagctcactcaaaggcggtaatacggttatccacagaatcaggggataacgcaggaaagaacatgtgagcaaaaggccagcaaaaggccaggaaccgtaaaaaggccgcgttgctggcgtttttccataggctccgcccccctgacgagcatcacaaaaatcgacgctcaagtcagaggtggcgaaacccgacaggactataaagataccaggcgtttccccctggaagctccctcgtgcgctctcctgttccgaccctgccgcttaccggatacctgtccgcctttctcccttcgggaagcgtggcgctttctcatagctcacgctgtaggtatctcagttcggtgtaggtcgttcgctccaagctgggctgtgtgcacgaaccccccgttcagcccgaccgctgcgccttatccggtaactatcgtcttgagtccaacccggtaagacacgacttatcgccactggcagcagccactggtaacaggattagcagagcgaggtatgtaggcggtgctacagagttcttgaagtggtggcctaactacggctacactagaagaacagtatttggtatctgcgctctgctgaagccagttaccttcggaaaaagagttggtagctcttgatccggcaaacaaaccaccgctggtagcggtggtttttttgtttgcaagcagcagattacgcgcagaaaaaaaggatctcaagaagatcctttgatcttttctacggggtctgacgctcagtggaacgaaaactcacgttaagggattttggtcatgagattatcaaaaaggatcttcacctagatccttttaaattaaaaatgaagttttaaatcaatctaaagtatatatgagtaaacttggtctgacagttaccaatgcttaatcagtgaggcacctatctcagcgatctgtctatttcgttcatccatagttgcctgactccccgtcgtgtagataactacgatacgggagggcttaccatctggccccagtgctgcaatgataccgcgagacccacgctcaccggctccagatttatcagcaataaaccagccagccggaagggccgagcgcagaagtggtcctgcaactttatccgcctccatccagtctattaattgttgccgggaagctagagtaagtagttcgccagttaatagtttgcgcaacgttgttgccattgctacaggcatcgtggtgtcacgctcgtcgtttggtatggcttcattcagctccggttcccaacgatcaaggcgagttacatgatcccccatgttgtgcaaaaaagcggttagctccttcggtcctccgatcgttgtcagaagtaagttggccgcagtgttatcactcatggttatggcagcactgcataattctcttactgtcatgccatccgtaagatgcttttctgtgactggtgagtactcaaccaagtcattctgagaatagtgtatgcggcgaccgagttgctcttgcccggcgtcaatacgggataataccgcgccacatagcagaactttaaaagtgctcatcattggaaaacgttcttcggggcgaaaactctcaaggatcttaccgctgttgagatccagttcgatgtaacccactcgtgcacccaactgatcttcagcatcttttactttcaccagcgtttctgggtgagcaaaaacaggaaggcaaaatgccgcaaaaaagggaataagggcgacacggaaatgttgaatactcatactcttcctttttcaatattattgaagcatttatcagggttattgtctcatgagcggatacatatttgaatgtatttagaaaaataaacaaataggggttccgcgcacatttccccgaaaagtgccacctgacgtctaagaaaccattattatcatgacattaacctataaaaataggcgtatcacgaggccctttcgtctcgcgcgtttcggtgatgacggtgaaaacctctgacacatgcagctcccggagacggtcacagcttgtctgtaagcggatgccgggagcagacaagcccgtcagggcgcgtcagcgggtgttggcgggtgtcggggctggcttaactatgcggcatcagagcagattgtactgagagtgcaccatatgcggtgtgaaataccgcacagatgcgtaaggagaaaataccgcatcaggcgccattcgccattcaggctgcgcaactgttgggaagggcgatcggtgcgggcctcttcgctattacgccagctggcgaaagggggatgtgctgcaaggcgattaagttgggtaacgccagggttttcccagtcacgacgttgtaaaacgacggccagtgaattc

SEQ ID NO: 13 - DNA, 11779 bp, Artificial Sequence
  Synthetic: TL20c-rGbGM
ggccgcctcggccaaacagcccttgagtttaccactccctatcagtgatagagaaaagtgaaagtcgagtttaccactccctatcagtgatagagaaaagtgaaagtcgagtttaccactccctatcagtgatagagaaaagtgaaagtcgagtttaccactccctatcagtgatagagaaaagtgaaagtcgagtttaccagtccctatcagtgatagagaaaagtgaaagtcgagtttaccactccctatcagtgatagagaaaagtgaaagtcgagtttaccactccctatcagtgatagagaaaagtgaaagtcgagctcgccatgggaggcgtggcctgggcgggactggggagtggcgagccctcagatcctgcatataagcagctgctttttgcctgtactgggtctctctggttagaccagatctgagcctgggagctctctggctaactagggaacccactgcttaagcctcaataaagcttgccttgagtgcttcaagtagtgtgtgcccgtctgttgtgtgactctggtaactagagatccctcagacccttttagtcagtgtggaaaatctctagcagtggcgcccgaacagggacttgaaagcgaaagggaaaccagaggagctctctcgacgcaggactcggcttgctgaagcgcgcacggcaagaggcgaggggcggcgactggtgagtacgccaaaaattttgactagcggaggctagaaggagagagatgggtgcgagagcgtcagtattaagcgggggagaattagatcgcgatgggaaaaaattcggttaaggccagggggaaagaaaaaatataaattaaaacatatagtatgggcaagcagggagctagaacgattcgcagttaatactggcctgttagaaacatcagaaggctgtagacaaatactgggacagctacaaccatcccttcagacaggatcagaagaacttagatcattatataatacagtagcaaccctctattgtgtgcatcaaaggatagagataaaagacaccaaggaagctttagacaagatagaggaagagcaaaacaaaagtaagaaaaaagcacagcaagcagcaggatcttcagacctggaaattccctacaatccccaaagtcaaggagtagtagaatctatgaataaagaattaaagaaaattataggacaggtaagagatcaggctgaacatcttaagacagcagtacaaatggcagtattcatccacaattttaaaagaaaaggggggattggggggtacagtgcaggggaaagaatagtagacataatagcaacagacatacaaactaaagaattacaaaaacaaattacaaaaattcaaaattttcgggtttattacagggacagcagaaatccactttggaaaggaccagcaaagctcctctggaaaggtgaaggggcagtagtaatacaagataatagtgacataaaagtagtgccaagaagaaaagcaaagatcattagggattatggaaaacagatggcaggtgatgattgtgtggcaagtagacaggatgaggattagaacatggaaaagtttagtaaaacaccataaggaggagatatgagggacaattggagaagtgaattatataaatataaagtagtaaaaattgaaccattaggagtagcacccaccaaggcaaagagaagagtggtgcagagagaaaaaagagcagtgggaataggagctttgttccttgggttcttgggagcagcaggaagcactatgggcgcagcgtcaatgacgctgacggtacaggccagacaattattgtctggtatagtgcagcagcagaacaatttgctgagggctattgaggcgcaacagcatctgttgcaactcacagtctggggcatcaagcagctccaggcaagaatcctggctgtggaaagatacctaaaggatcaacagctcctggggatttggggttgctctggaaaactcatttgcaccactgctgtgccttggaatgctagttggagtaataaatctctggaacagatttggaatcacacgacctggatggagtgggacagagaaattaacaattacacaagcttaatacactccttaattgaagaatcgcaaaaccagcaagaaaagaatgaacaagaattattggaattagataaatgggcaagtttgtggaattggtttaacataacaaattggctgtggtatataaaattattcataatgatagtaggaggcttggtaggtttaagaatagtttttgctgtactttctatagtgaatagagttaggcagggatattcaccattatcgtttcagacccacctcccaaccccgaggggaccgagctcaagcttcgaacgcgtggggatcctctagagtcgagctcgcgaggatcatcaccggtgctagccggagccagaagcaccataagggacatgataagggagccagcagacctctgatctcttcctgaatgctaatcttaaacatcctgaggaagaatgggacttccatttggggtgggcctatgatagggtaataagacagtagtgaatatcaagctacaaaaagccccctttcaaattcttctcagtcctaacttttcatactaagcccagtccttccaaagcagactgtgaaagagtgatagttccgggagactagcaccggctagccgagcttggaacactttcccttcattaagaaccatccttgctactcagctgcaatcaatccagcccccaggtcttcactgaaccttttcccatctcttccaaaacatctgtttctgagaagtcctgtcctatagaggtctttcttcccaccggatttctcctacaccatttactcccacttgcagaactcccgtgtacaagtgtctttactgcttttatttgctcaacaaaatgcacatctcatataaaaataaatgaggagcatgcacacaccacaaacacaaacaggcatgcagaaatacacatacacacttccctcaatataaaccctttgtggctcatatatttaaaaagatgtaaaaaaaagagctgaagaaaatcatgtgtgatctctcagcagaatagatttattatttgtattgcttgcagaataaagcctatccttgaaagctctgaatcatgggcaagaggctcagtggtatctggaggacagggcactggccactgcagtcaccatcttctgccaggaagcctgcacctcaggggtgaattctttgccaaagtgaatggccagcacggtgaccagcacgttgcccaggagctgtgggaggaagataagaggtatgaacatgattagcaaaagggcctagcttggactcagaataatccagccttatcccaaccataaaataaaagcagaatggtagctggattgtagctgctattagcaatatgaaacctcttacatcagttacaatttatatgcagaaatatttatatgcagaaatattgctattgccttaacccagaaattatcactgttattctttagaatggtgcaaagaggcatgatacattgtatcattattgccctgaaagaaagagattagggaaagtattagaaataagataaacaaaaaagtatattaaaagaagaaagcattttttaaaattacaaatgcaaaattaccctgatttggtcaatatgtgtaccctgttacttctccccttcctatgacatgaacttaaccatagaaaagaaggggaaagaaaacatcaagggtcccatagactcaccttgaagttctcaggatccacatgcagcttgtcacagtgcagttcactcagctgggcaaaggtgcccttgagatcatccaggtgctttatggcatctcccaaggaagtcagcaccttcttgccatgtgccttgactttggggttgcccatgatggcagaggcagaggacaggttgccaaagctgtcaaagaacctctgggtccatgggtagacaaccaggagcctgtgagattgacaagaacagtttgacagtcagaaggtgccacaaatcctgagaagcaacctggacttttgccaggcacagggtccttccttccctcccttgtcctggtcaccagagcctaccttcccagggtttctcctccagcatcttccacattcaccttgtcccacaggcttgtgatagtagccttgtcctcctctgtgaaatgacccatggtgtctgtttgaggttgctagtgaacacagttgtgtcagaagcaaatgtaagcaatagatggctctgccctgacttttatgcccagccctggctcctgccctccctgctcctgggagtagattggccaaccctagggtgtggctccacagggtgaggtctaagtgatgacagccgtacctgtccttggctcttctggcactggcttaggagttggacttcaaaccctcagccctccctctaagatatatctcttggccccataccatcagtacaaattgctactaaaaacatcctcctttgcaagtgtatttacgacggtatcgatgtatgtgagcatgtgtcctctaacagcacaggccttttgccacctagctgtccaggggtgccttaaaatggcaaacaaggtttgttttcttttcctgttttcatgccttcctcttccatatccttgtttcatattaatacatgtgtatagatcctaaaaatctatacacatgtattaataaagcctgattctgccgcttctaggtatagaggccacctgcaagataaatatttgattcacaataactaatcattctatggcaattgataacaacaaatatatatatatatatatatatacgtatatgtgtatatatatatatatattcaggaaataatatattctagaatatgtcacattctgtctcaggcatccattttctttatgatgccgtttgaggtggagttttagtcaggtggtcagcttctccttttttttgccatctgccctgtaagcatcctgctggggacccagataggagtcatcactctaggctgagaacatctgggcacacaccctaagcctcagcatgactcatcatgactcagcattgctgtgcttgagccagaaggtttgcttagaaggttacacagaaccagaaggcgggggtggggcactgaccccgacaggggcctggccagaactgctcatgcttggactatgggaggtcactaatggagacacacagaaatgtaacaggaactaagggaattccggtgccctgcttaggagcttaatctttaatgaaagctaagctttcattaaaaaaagtctaaccagctgcattcgactttgactgcagcagctggttagaaggttctactggaggagggtcccagcccattgctaaattaacatcaggctctgagactggcagtatatctctaacagtggttgatgctatcttctggaacttgcctgctacattgagaccactgacccatacataggaagcccatagctctgtcctgaactgttaggccactggtccagagagtgtgcatctcctttgatcctcataataaccctatgagatagacacaattattactcttactttatagatgatgatcctgaaaacataggagtcaaggcacttgcccctagctgggggtataggggagcagtcccatgtagtagtagaatgaaaaatgctgctatgctgtgcctcccccacctttcccatgtctgccctctactcatggtctatctctcctggctcctgggagtcatggactccacccagcaccaccaacctgacctaaccacctatctgagcctgccagcctataacccatctgggccctgatagctggtggccagccctgaccccaccccaccctccctggaacctctgatagacacatctggcacaccagctcgcaaagtcaccgtgagggtcttgtgtttgctgagtcaaaattccttgaaatccaagtccttagagactcctgctcccaaatttacagtcatagacttcttcatggctgtctcctttatccacagaatgattcctttgcttcattgccccatccatctgatcctcctcatcagtgcagcacagggcccatgagcagtagctgcagagtctcacataggtctggcactgcctctgacatgtccgaccttaggcaaatgcttgactcttctgagctcggatcccttgagctcaggaggtcaaggctgcagtgagacatgatcttgccactgcactccagcctggacagcagagtgaaaccttgcctcacgaaacagaatacaaaaacaaacaaacaaaaaactgctccgcaatgcgcttccttgatgctctaccacataggtctgggtactttgtacacattatctcattgctgttcataattgttagattaattttgtaatattgatattattcctagaaagctgaggcctcaagatgataacttttattttctggacttgtaatagctttctcttgtattcaccatgttgtaactttcttagagtagtaacaatataaagttattgtgagtttttgcaaacacagcaaacacaacgacccatatagacattgatgtgaaattgtctattgtcaatttatgggaaaacaagtatgtactttttctactaagccattgaaacaggaataacagaacaagattgaaagaatacattttccgaaattacttgagtattatacaaagacaagcacgtggacctgggaggagggttattgtccatgactggtgtgtggagacaaatgcaggtttataatagatgggatggcatctagcgcaatgactttgccatcacttttagagagctcttgggggccccagtacacaagaggggacgcagggtatatgtagacatctcattctttttcttagtgtgagaataagaatagccatgacctgagtttatagacaatgagcccttttctctctcccactcagcagctatgagatggcttgccctgcctctctactaggctgactcactccaaggcccagcaatgggcagggctctgtcagggctttgatagcactatctgcagagccagggccgagaaggggtggactccagagactctccctcccattcccgagcagggtttgcttatttatgcatttaaatgatatatttattttaaaagaaataacaggagactgcccagccctggctgtgacatggaaactatgtagaatattttgggttccatttttttttccttctttcagttagaggaaaaggggctcactgcacatacactagacagaaagtcaggagctttgaatccaagcctgatcatttccatgtcatactgagaaagtccccacccttctctgagcctcagtttctctttttataagtaggagtctggagtaaatgatttccaatggctctcatttcaatacaaaatttccgtttattaaatgcatgagcttccgttactccaagactgagaaggaaattgaacctgagactcattgactggcaagatgtccccagaggctctcattcagcaataaaattctcaccttcacccaggcccactagtgtcagatttgcatgcgttaacgcggccgcatcgatgccgtagtacctttaagaccaatgacttacaaggcagctgtagatcttagccactttttaaaagaaaaggggggactggaagggctaattcactcccaaagaagacaagatccctgcaggcattcaaggccaggctggatgtggctctgggcagcctgggctgctggttgatgaccctgcacatagcagggggttggatctggatgagcactgtgctcctttgcaacccaggccgttctatgattctgtcattctaaatctctctttcagcctaaagctttttccccgtatccccccaggtgtctgcaggctcaaagagcagcgagaagcgttcagaggaaagcgatcccgtgccaccttccccgtgcccgggctgtccccgcacgctgccggctcggggatgcggggggagcgccggaccggagcggagccccgggcggctcgctgctgccccctagcgggggagggacgtaattacatccctgggggctttgggggggggctgtccccgtgagctccccagatctgctttttgcctgtactgggtctctctggttagaccagatctgagcctgggagctctctggctaactagggaacccactgcttaagcctcaataaagcttcagctgctcgagctagcagatctttttccctctgccaaaaattatggggacatcatgaagccccttgagcatctgacttctggctaataaaggaaatttattttcattgcaatagtgtgttggaattttttgtgtctctcactcggaaggacatatgggagggcaaatcatttaaaacatcagaatgagtatttggtttagagtttggcaacatatgcccatatgctggctgccatgaacaaaggttggctataaagaggtcatcagtatatgaaacagccccctgctgtccattccttattccatagaaaagccttgacttgaggttagattttttttatattttgttttgtgttatttttttctttaacatccctaaaattttccttacatgttttactagccagatttttcctcctctcctgactactcccagtcatagctgtccctcttctcttatggagatccctcgacctgcagcccaagcttggcgtaatcatggtcatagctgtttcctgtgtgaaattgttatccgctcacaattccacacaacatacgagccggaagcataaagtgtaaagcctggggtgcctaatgagtgagctaactcacattaattgcgttgcgctcactgcccgctttccagtcgggaaacctgtcgtgccagcggatccgcatctcaattagtcagcaaccatagtcccgcccctaactccgcccatcccgcccctaactccgcccagttccgcccattctccgccccatggctgactaattttttttatttatgcagaggccgaggccgcctcggcctctgagctattccagaagtagtgaggaggcttttttggaggcctaggcttttgcaaaaagctgtcgactgcagaggcctgcatgcaagcttggcgtaatcatggtcatagctgtttcctgtgtgaaattgttatccgctcacaattccacacaacatacgagccggaagcataaagtgtaaagcctggggtgcctaatgagtgagctaactcacattaattgcgttgcgctcactgcccgctttccagtcgggaaacctgtcgtgccagctgcattaatgaatcggccaacgcgcggggagaggcggtttgcgtattgggcgctcttccgcttcctcgctcactgactcgctgcgctcggtcgttcggctgcggcgagcggtatcagctcactcaaaggcggtaatacggttatccacagaatcaggggataacgcaggaaagaacatgtgagcaaaaggccagcaaaaggccaggaaccgtaaaaaggccgcgttgctggcgtttttccataggctccgcccccctgacgagcatcacaaaaatcgacgctcaagtcagaggtggcgaaacccgacaggactataaagataccaggcgtttccccctggaagctccctcgtgcgctctcctgttccgaccctgccgcttaccggatacctgtccgcctttctcccttcgggaagcgtggcgctttctcatagctcacgctgtaggtatctcagttcggtgtaggtcgttcgctccaagctgggctgtgtgcacgaaccccccgttcagcccgaccgctgcgccttatccggtaactatcgtcttgagtccaacccggtaagacacgacttatcgccactggcagcagccactggtaacaggattagcagagcgaggtatgtaggcggtgctacagagttcttgaagtggtggcctaactacggctacactagaagaacagtatttggtatctgcgctctgctgaagccagttaccttcggaaaaagagttggtagctcttgatccggcaaacaaaccaccgctggtagcggtggtttttttgtttgcaagcagcagattacgcgcagaaaaaaaggatctcaagaagatcctttgatcttttctacggggtctgacgctcagtggaacgaaaactcacgttaagggattttggtcatgagattatcaaaaaggatcttcacctagatccttttaaattaaaaatgaagttttaaatcaatctaaagtatatatgagtaaacttggtctgacagttaccaatgcttaatcagtgaggcacctatctcagcgatctgtctatttcgttcatccatagttgcctgactccccgtcgtgtagataactacgatacgggagggcttaccatctggccccagtgctgcaatgataccgcgagacccacgctcaccggctccagatttatcagcaataaaccagccagccggaagggccgagcgcagaagtggtcctgcaactttatccgcctccatccagtctattaattgttgccgggaagctagagtaagtagttcgccagttaatagtttgcgcaacgttgttgccattgctacaggcatcgtggtgtcacgctcgtcgtttggtatggcttcattcagctccggttcccaacgatcaaggcgagttacatgatcccccatgttgtgcaaaaaagcggttagctccttcggtcctccgatcgttgtcagaagtaagttggccgcagtgttatcactcatggttatggcagcactgcataattctcttactgtcatgccatccgtaagatgcttttctgtgactggtgagtactcaaccaagtcattctgagaatagtgtatgcggcgaccgagttgctcttgcccggcgtcaatacgggataataccgcgccacatagcagaactttaaaagtgctcatcattggaaaacgttcttcggggcgaaaactctcaaggatcttaccgctgttgagatccagttcgatgtaacccactcgtgcacccaactgatcttcagcatcttttactttcaccagcgtttctgggtgagcaaaaacaggaaggcaaaatgccgcaaaaaagggaataagggcgacacggaaatgttgaatactcatactcttcctttttcaatattattgaagcatttatcagggttattgtctcatgagcggatacatatttgaatgtatttagaaaaataaacaaataggggttccgcgcacatttccccgaaaagtgccacctgacgtctaagaaaccattattatcatgacattaacctataaaaataggcgtatcacgaggccctttcgtctcgcgcgtttcggtgatgacggtgaaaacctctgacacatgcagctcccggagacggtcacagcttgtctgtaagcggatgccgggagcagacaagcccgtcagggcgcgtcagcgggtgttggcgggtgtcggggctggcttaactatgcggcatcagagcagattgtactgagagtgcaccatatgcggtgtgaaataccgcacagatgcgtaaggagaaaataccgcatcaggcgccattcgccattcaggctgcgcaactgttgggaagggcgatcggtgcgggcctcttcgctattacgccagctggcgaaagggggatgtgctgcaaggcgattaagttgggtaacgccagggttttcccagtcacgacgttgtaaaacgacggccagtgaattc

SEQ ID NO: 14 - DNA, 11678 bp, Artificial Sequence
  Synthetic: TL20d-7SKM1/sh734-rGbGM
ggccgcctcggccaaacagcccttgagtttaccactccctatcagtgatagagaaaagtgaaagtcgagtttaccactccctatcagtgatagagaaaagtgaaagtcgagtttaccactccctatcagtgatagagaaaagtgaaagtcgagtttaccactccctatcagtgatagagaaaagtgaaagtcgagtttaccagtccctatcagtgatagagaaaagtgaaagtcgagtttaccactccctatcagtgatagagaaaagtgaaagtcgagtttaccactccctatcagtgatagagaaaagtgaaagtcgagctcgccatgggaggcgtggcctgggcgggactggggagtggcgagccctcagatcctgcatataagcagctgctttttgcctgtactgggtctctctggttagaccagatctgagcctgggagctctctggctaactagggaacccactgcttaagcctcaataaagcttgccttgagtgcttcaagtagtgtgtgcccgtctgttgtgtgactctggtaactagagatccctcagacccttttagtcagtgtggaaaatctctagcagtggcgcccgaacagggacttgaaagcgaaagggaaaccagaggagctctctcgacgcaggactcggcttgctgaagcgcgcacggcaagaggcgaggggcggcgactggtgagtacgccaaaaattttgactagcggaggctagaaggagagagatgggtgcgagagcgtcagtattaagcgggggagaattagatcgcgatgggaaaaaattcggttaaggccagggggaaagaaaaaatataaattaaaacatatagtatgggcaagcagggagctagaacgattcgcagttaatactggcctgttagaaacatcagaaggctgtagacaaatactgggacagctacaaccatcccttcagacaggatcagaagaacttagatcattatataatacagtagcaaccctctattgtgtgcatcaaaggatagagataaaagacaccaaggaagctttagacaagatagaggaagagcaaaacaaaagtaagaaaaaagcacagcaagcagcaggatcttcagacctggaaattccctacaatccccaaagtcaaggagtagtagaatctatgaataaagaattaaagaaaattataggacaggtaagagatcaggctgaacatcttaagacagcagtacaaatggcagtattcatccacaattttaaaagaaaaggggggattggggggtacagtgcaggggaaagaatagtagacataatagcaacagacatacaaactaaagaattacaaaaacaaattacaaaaattcaaaattttcgggtttattacagggacagcagaaatccactttggaaaggaccagcaaagctcctctggaaaggtgaaggggcagtagtaatacaagataatagtgacataaaagtagtgccaagaagaaaagcaaagatcattagggattatggaaaacagatggcaggtgatgattgtgtggcaagtagacaggatgaggattagaacatggaaaagtttagtaaaacaccataaggaggagatatgagggacaattggagaagtgaattatataaatataaagtagtaaaaattgaaccattaggagtagcacccaccaaggcaaagagaagagtggtgcagagagaaaaaagagcagtgggaataggagctttgttccttgggttcttgggagcagcaggaagcactatgggcgcagcgtcaatgacgctgacggtacaggccagacaattattgtctggtatagtgcagcagcagaacaatttgctgagggctattgaggcgcaacagcatctgttgcaactcacagtctggggcatcaagcagctccaggcaagaatcctggctgtggaaagatacctaaaggatcaacagctcctggggatttggggttgctctggaaaactcatttgcaccactgctgtgccttggaatgctagttggagtaataaatctctggaacagatttggaatcacacgacctggatggagtgggacagagaaattaacaattacacaagcttaatacactccttaattgaagaatcgcaaaaccagcaagaaaagaatgaacaagaattattggaattagataaatgggcaagtttgtggaattggtttaacataacaaattggctgtggtatataaaattattcataatgatagtaggaggcttggtaggtttaagaatagtttttgctgtactttctatagtgaatagagttaggcagggatattcaccattatcgtttcagacccacctcccaaccccgaggggaccgagctcaagcttcgaagcggccgctcgacgtgcagtcgggctactgccccacccatagtaccggcattctggatagtgtcaaaacagccggaaatcaagtccgtttatctcaaactttagcattttgggaataaatgatatttgctatgctggttaaattagattttagttaaatttcctgctgaagctctagtacgataagtaacttgacctaagtgtaaagttgagatttccttcaggtttatatagcttgtgcgccgcctgggtacctcaggatatgcccttgactatttgtccgacatagtcaagggcatatccttttttacgcgtggggatcctctagagtcgagctcgcgaggatcatcaccggtgctagccggagccagaagcaccataagggacatgataagggagccagcagacctctgatctcttcctgaatgctaatcttaaacatcctgaggaagaatgggacttccatttggggtgggcctatgatagggtaataagacagtagtgaatatcaagctacaaaaagccccctttcaaattcttctcagtcctaacttttcatactaagcccagtccttccaaagcagactgtgaaagagtgatagttccgggagactagcaccggctagccgagcttggaacactttcccttcattaagaaccatccttgctactcagctgcaatcaatccagcccccaggtcttcactgaaccttttcccatctcttccaaaacatctgtttctgagaagtcctgtcctatagaggtctttcttcccaccggatttctcctacaccatttactcccacttgcagaactcccgtgtacaagtgtctttactgcttttatttgctcaacaaaatgcacatctcatataaaaataaatgaggagcatgcacacaccacaaacacaaacaggcatgcagaaatacacatacacacttccctcaatataaaccctttgtggctcatatatttaaaaagatgtaaaaaaaagagctgaagaaaatcatgtgtgatctctcagcagaatagatttattatttgtattgcttgcagaataaagcctatccttgaaagctctgaatcatgggcaagaggctcagtggtatctggaggacagggcactggccactgcagtcaccatcttctgccaggaagcctgcacctcaggggtgaattctttgccaaagtgaatggccagcacggtgaccagcacgttgcccaggagctgtgggaggaagataagaggtatgaacatgattagcaaaagggcctagcttggactcagaataatccagccttatcccaaccataaaataaaagcagaatggtagctggattgtagctgctattagcaatatgaaacctcttacatcagttacaatttatatgcagaaatatttatatgcagaaatattgctattgccttaacccagaaattatcactgttattctttagaatggtgcaaagaggcatgatacattgtatcattattgccctgaaagaaagagattagggaaagtattagaaataagataaacaaaaaagtatattaaaagaagaaagcattttttaaaattacaaatgcaaaattaccctgatttggtcaatatgtgtaccctgttacttctccccttcctatgacatgaacttaaccatagaaaagaaggggaaagaaaacatcaagggtcccatagactcaccttgaagttctcaggatccacatgcagcttgtcacagtgcagttcactcagctgggcaaaggtgcccttgagatcatccaggtgctttatggcatctcccaaggaagtcagcaccttcttgccatgtgccttgactttggggttgcccatgatggcagaggcagaggacaggttgccaaagctgtcaaagaacctctgggtccatgggtagacaaccaggagcctgtgagattgacaagaacagtttgacagtcagaaggtgccacaaatcctgagaagcaacctggacttttgccaggcacagggtccttccttccctcccttgtcctggtcaccagagcctaccttcccagggtttctcctccagcatcttccacattcaccttgtcccacaggcttgtgatagtagccttgtcctcctctgtgaaatgacccatggtgtctgtttgaggttgctagtgaacacagttgtgtcagaagcaaatgtaagcaatagatggctctgccctgacttttatgcccagccctggctcctgccctccctgctcctgggagtagattggccaaccctagggtgtggctccacagggtgaggtctaagtgatgacagccgtacctgtccttggctcttctggcactggcttaggagttggacttcaaaccctcagccctccctctaagatatatctcttggccccataccatcagtacaaattgctactaaaaacatcctcctttgcaagtgtatttacgacggtatcgatgtatgtgagcatgtgtcctctaacagcacaggccttttgccacctagctgtccaggggtgccttaaaatggcaaacaaggtttgttttcttttcctgttttcatgccttcctcttccatatccttgtttcatattaatacatgtgtatagatcctaaaaatctatacacatgtattaataaagcctgattctgccgcttctaggtatagaggccacctgcaagataaatatttgattcacaataactaatcattctatggcaattgataacaacaaatatatatatatatatatatatacgtatatgtgtatatatatatatatattcaggaaataatatattctagaatatgtcacattctgtctcaggcatccattttctttatgatgccgtttgaggtggagttttagtcaggtggtcagcttctccttttttttgccatctgccctgtaagcatcctgctggggacccagataggagtcatcactctaggctgagaacatctgggcacacaccctaagcctcagcatgactcatcatgactcagcattgctgtgcttgagccagaaggtttgcttagaaggttacacagaaccagaaggcgggggtggggcactgaccccgacaggggcctggccagaactgctcatgcttggactatgggaggtcactaatggagacacacagaaatgtaacaggaactaagggaattccggtgccctgcttaggagcttaatctttaatgaaagctaagctttcattaaaaaaagtctaaccagctgcattcgactttgactgcagcagctggttagaaggttctactggaggagggtcccagcccattgctaaattaacatcaggctctgagactggcagtatatctctaacagtggttgatgctatcttctggaacttgcctgctacattgagaccactgacccatacataggaagcccatagctctgtcctgaactgttaggccactggtccagagagtgtgcatctcctttgatcctcataataaccctatgagatagacacaattattactcttactttatagatgatgatcctgaaaacataggagtcaaggcacttgcccctagctgggggtataggggagcagtcccatgtagtagtagaatgaaaaatgctgctatgctgtgcctcccccacctttcccatgtctgccctctactcatggtctatctctcctggctcctgggagtcatggactccacccagcaccaccaacctgacctaaccacctatctgagcctgccagcctataacccatctgggccctgatagctggtggccagccctgaccccaccccaccctccctggaacctctgatagacacatctggcacaccagctcgcaaagtcaccgtgagggtcttgtgtttgctgagtcaaaattccttgaaatccaagtccttagagactcctgctcccaaatttacagtcatagacttcttcatggctgtctcctttatccacagaatgattcctttgcttcattgccccatccatctgatcctcctcatcagtgcagcacagggcccatgagcagtagctgcagagtctcacataggtctggcactgcctctgacatgtccgaccttaggcaaatgcttgactcttctgagctcggatcccttgagctcaggaggtcaaggctgcagtgagacatgatcttgccactgcactccagcctggacagcagagtgaaaccttgcctcacgaaacagaatacaaaaacaaacaaacaaaaaactgctccgcaatgcgcttccttgatgctctaccacataggtctgggtactttgtacacattatctcattgctgttcataattgttagattaattttgtaatattgatattattcctagaaagctgaggcctcaagatgataacttttattttctggacttgtaatagctttctcttgtattcaccatgttgtaactttcttagagtagtaacaatataaagttattgtgagtttttgcaaacacagcaaacacaacgacccatatagacattgatgtgaaattgtctattgtcaatttatgggaaaacaagtatgtactttttctactaagccattgaaacaggaataacagaacaagattgaaagaatacattttccgaaattacttgagtattatacaaagacaagcacgtggacctgggaggagggttattgtccatgactggtgtgtggagacaaatgcaggtttataatagatgggatggcatctagcgcaatgactttgccatcacttttagagagctcttgggggccccagtacacaagaggggacgcagggtatatgtagacatctcattctttttcttagtgtgagaataagaatagccatgacctgagtttatagacaatgagcccttttctctctcccactcagcagctatgagatggcttgccctgcctctctactaggctgactcactccaaggcccagcaatgggcagggctctgtcagggctttgatagcactatctgcagagccagggccgagaaggggtggactccagagactctccctcccattcccgagcagggtttgcttatttatgcatttaaatgatatatttattttaaaagaaataacaggagactgcccagccctggctgtgacatggaaactatgtagaatattttgggttccatttttttttccttctttcagttagaggaaaaggggctcactgcacatacactagacagaaagtcaggagctttgaatccaagcctgatcatttccatgtcatactgagaaagtccccacccttctctgagcctcagtttctctttttataagtaggagtctggagtaaatgatttccaatggctctcatttcaatacaaaatttccgtttattaaatgcatgagcttccgttactccaagactgagaaggaaattgaacctgagactcattgactggcaagatgtccccagaggctctcattcagcaataaaattctcaccttcacccaggcccactagtgtcagatttgcatgcgttaacgcggccgcatcgatgccgtagtacctttaagaccaatgacttacaaggcagctgtagatcttagccactttttaaaagaaaaggggggactggaagggctaattcactcccaaagaagacaagatagatctgctttttgcctgtactgggtctctctggttagaccagatctgagcctgggagctctctggctaactagggaacccactgcttaagcctcaataaagcttcagctgctcgagctagcagatctttttccctctgccaaaaattatggggacatcatgaagccccttgagcatctgacttctggctaataaaggaaatttattttcattgcaatagtgtgttggaattttttgtgtctctcactcggaaggacatatgggagggcaaatcatttaaaacatcagaatgagtatttggtttagagtttggcaacatatgcccatatgctggctgccatgaacaaaggttggctataaagaggtcatcagtatatgaaacagccccctgctgtccattccttattccatagaaaagccttgacttgaggttagattttttttatattttgttttgtgttatttttttctttaacatccctaaaattttccttacatgttttactagccagatttttcctcctctcctgactactcccagtcatagctgtccctcttctcttatggagatccctcgacctgcagcccaagcttggcgtaatcatggtcatagctgtttcctgtgtgaaattgttatccgctcacaattccacacaacatacgagccggaagcataaagtgtaaagcctggggtgcctaatgagtgagctaactcacattaattgcgttgcgctcactgcccgctttccagtcgggaaacctgtcgtgccagcggatccgcatctcaattagtcagcaaccatagtcccgcccctaactccgcccatcccgcccctaactccgcccagttccgcccattctccgccccatggctgactaattttttttatttatgcagaggccgaggccgcctcggcctctgagctattccagaagtagtgaggaggcttttttggaggcctaggcttttgcaaaaagctgtcgactgcagaggcctgcatgcaagcttggcgtaatcatggtcatagctgtttcctgtgtgaaattgttatccgctcacaattccacacaacatacgagccggaagcataaagtgtaaagcctggggtgcctaatgagtgagctaactcacattaattgcgttgcgctcactgcccgctttccagtcgggaaacctgtcgtgccagctgcattaatgaatcggccaacgcgcggggagaggcggtttgcgtattgggcgctcttccgcttcctcgctcactgactcgctgcgctcggtcgttcggctgcggcgagcggtatcagctcactcaaaggcggtaatacggttatccacagaatcaggggataacgcaggaaagaacatgtgagcaaaaggccagcaaaaggccaggaaccgtaaaaaggccgcgttgctggcgtttttccataggctccgcccccctgacgagcatcacaaaaatcgacgctcaagtcagaggtggcgaaacccgacaggactataaagataccaggcgtttccccctggaagctccctcgtgcgctctcctgttccgaccctgccgcttaccggatacctgtccgcctttctcccttcgggaagcgtggcgctttctcatagctcacgctgtaggtatctcagttcggtgtaggtcgttcgctccaagctgggctgtgtgcacgaaccccccgttcagcccgaccgctgcgccttatccggtaactatcgtcttgagtccaacccggtaagacacgacttatcgccactggcagcagccactggtaacaggattagcagagcgaggtatgtaggcggtgctacagagttcttgaagtggtggcctaactacggctacactagaagaacagtatttggtatctgcgctctgctgaagccagttaccttcggaaaaagagttggtagctcttgatccggcaaacaaaccaccgctggtagcggtggtttttttgtttgcaagcagcagattacgcgcagaaaaaaaggatctcaagaagatcctttgatcttttctacggggtctgacgctcagtggaacgaaaactcacgttaagggattttggtcatgagattatcaaaaaggatcttcacctagatccttttaaattaaaaatgaagttttaaatcaatctaaagtatatatgagtaaacttggtctgacagttaccaatgcttaatcagtgaggcacctatctcagcgatctgtctatttcgttcatccatagttgcctgactccccgtcgtgtagataactacgatacgggagggcttaccatctggccccagtgctgcaatgataccgcgagacccacgctcaccggctccagatttatcagcaataaaccagccagccggaagggccgagcgcagaagtggtcctgcaactttatccgcctccatccagtctattaattgttgccgggaagctagagtaagtagttcgccagttaatagtttgcgcaacgttgttgccattgctacaggcatcgtggtgtcacgctcgtcgtttggtatggcttcattcagctccggttcccaacgatcaaggcgagttacatgatcccccatgttgtgcaaaaaagcggttagctccttcggtcctccgatcgttgtcagaagtaagttggccgcagtgttatcactcatggttatggcagcactgcataattctcttactgtcatgccatccgtaagatgcttttctgtgactggtgagtactcaaccaagtcattctgagaatagtgtatgcggcgaccgagttgctcttgcccggcgtcaatacgggataataccgcgccacatagcagaactttaaaagtgctcatcattggaaaacgttcttcggggcgaaaactctcaaggatcttaccgctgttgagatccagttcgatgtaacccactcgtgcacccaactgatcttcagcatcttttactttcaccagcgtttctgggtgagcaaaaacaggaaggcaaaatgccgcaaaaaagggaataagggcgacacggaaatgttgaatactcatactcttcctttttcaatattattgaagcatttatcagggttattgtctcatgagcggatacatatttgaatgtatttagaaaaataaacaaataggggttccgcgcacatttccccgaaaagtgccacctgacgtctaagaaaccattattatcatgacattaacctataaaaataggcgtatcacgaggccctttcgtctcgcgcgtttcggtgatgacggtgaaaacctctgacacatgcagctcccggagacggtcacagcttgtctgtaagcggatgccgggagcagacaagcccgtcagggcgcgtcagcgggtgttggcgggtgtcggggctggcttaactatgcggcatcagagcagattgtactgagagtgcaccatatgcggtgtgaaataccgcacagatgcgtaaggagaaaataccgcatcaggcgccattcgccattcaggctgcgcaactgttgggaagggcgatcggtgcgggcctcttcgctattacgccagctggcgaaagggggatgtgctgcaaggcgattaagttgggtaacgccagggttttcccagtcacgacgttgtaaaacgacggccagtgaattc

SEQ ID NO: 15 - DNA, 11681 bp, Artificial Sequence
  Synthetic: TL20d-7SK/sh734-rGbGM
ggccgcctcggccaaacagcccttgagtttaccactccctatcagtgatagagaaaagtgaaagtcgagtttaccactccctatcagtgatagagaaaagtgaaagtcgagtttaccactccctatcagtgatagagaaaagtgaaagtcgagtttaccactccctatcagtgatagagaaaagtgaaagtcgagtttaccagtccctatcagtgatagagaaaagtgaaagtcgagtttaccactccctatcagtgatagagaaaagtgaaagtcgagtttaccactccctatcagtgatagagaaaagtgaaagtcgagctcgccatgggaggcgtggcctgggcgggactggggagtggcgagccctcagatcctgcatataagcagctgctttttgcctgtactgggtctctctggttagaccagatctgagcctgggagctctctggctaactagggaacccactgcttaagcctcaataaagcttgccttgagtgcttcaagtagtgtgtgcccgtctgttgtgtgactctggtaactagagatccctcagacccttttagtcagtgtggaaaatctctagcagtggcgcccgaacagggacttgaaagcgaaagggaaaccagaggagctctctcgacgcaggactcggcttgctgaagcgcgcacggcaagaggcgaggggcggcgactggtgagtacgccaaaaattttgactagcggaggctagaaggagagagatgggtgcgagagcgtcagtattaagcgggggagaattagatcgcgatgggaaaaaattcggttaaggccagggggaaagaaaaaatataaattaaaacatatagtatgggcaagcagggagctagaacgattcgcagttaatactggcctgttagaaacatcagaaggctgtagacaaatactgggacagctacaaccatcccttcagacaggatcagaagaacttagatcattatataatacagtagcaaccctctattgtgtgcatcaaaggatagagataaaagacaccaaggaagctttagacaagatagaggaagagcaaaacaaaagtaagaaaaaagcacagcaagcagcaggatcttcagacctggaaattccctacaatccccaaagtcaaggagtagtagaatctatgaataaagaattaaagaaaattataggacaggtaagagatcaggctgaacatcttaagacagcagtacaaatggcagtattcatccacaattttaaaagaaaaggggggattggggggtacagtgcaggggaaagaatagtagacataatagcaacagacatacaaactaaagaattacaaaaacaaattacaaaaattcaaaattttcgggtttattacagggacagcagaaatccactttggaaaggaccagcaaagctcctctggaaaggtgaaggggcagtagtaatacaagataatagtgacataaaagtagtgccaagaagaaaagcaaagatcattagggattatggaaaacagatggcaggtgatgattgtgtggcaagtagacaggatgaggattagaacatggaaaagtttagtaaaacaccataaggaggagatatgagggacaattggagaagtgaattatataaatataaagtagtaaaaattgaaccattaggagtagcacccaccaaggcaaagagaagagtggtgcagagagaaaaaagagcagtgggaataggagctttgttccttgggttcttgggagcagcaggaagcactatgggcgcagcgtcaatgacgctgacggtacaggccagacaattattgtctggtatagtgcagcagcagaacaatttgctgagggctattgaggcgcaacagcatctgttgcaactcacagtctggggcatcaagcagctccaggcaagaatcctggctgtggaaagatacctaaaggatcaacagctcctggggatttggggttgctctggaaaactcatttgcaccactgctgtgccttggaatgctagttggagtaataaatctctggaacagatttggaatcacacgacctggatggagtgggacagagaaattaacaattacacaagcttaatacactccttaattgaagaatcgcaaaaccagcaagaaaagaatgaacaagaattattggaattagataaatgggcaagtttgtggaattggtttaacataacaaattggctgtggtatataaaattattcataatgatagtaggaggcttggtaggtttaagaatagtttttgctgtactttctatagtgaatagagttaggcagggatattcaccattatcgtttcagacccacctcccaaccccgaggggaccgagctcaagcttcgaagcggccgcatcgacgtgcagtatttagcatgccccacccatctgcaaggcattctggatagtgtcaaaacagccggaaatcaagtccgtttatctcaaactttagcattttgggaataaatgatatttgctatgctggttaaattagattttagttaaatttcctgctgaagctctagtacgataagtaacttgacctaagtgtaaagttgagatttccttcaggtttatatagcttgtgcgccgcctgggtacctcaggatatgcccttgactatttgtccgacatagtcaagggcatatccttttttgtacgcgtggggatcctctagagtcgagctcgcgaggatcatcaccggtgctagccggagccagaagcaccataagggacatgataagggagccagcagacctctgatctcttcctgaatgctaatcttaaacatcctgaggaagaatgggacttccatttggggtgggcctatgatagggtaataagacagtagtgaatatcaagctacaaaaagccccctttcaaattcttctcagtcctaacttttcatactaagcccagtccttccaaagcagactgtgaaagagtgatagttccgggagactagcaccggctagccgagcttggaacactttcccttcattaagaaccatccttgctactcagctgcaatcaatccagcccccaggtcttcactgaaccttttcccatctcttccaaaacatctgtttctgagaagtcctgtcctatagaggtctttcttcccaccggatttctcctacaccatttactcccacttgcagaactcccgtgtacaagtgtctttactgcttttatttgctcaacaaaatgcacatctcatataaaaataaatgaggagcatgcacacaccacaaacacaaacaggcatgcagaaatacacatacacacttccctcaatataaaccctttgtggctcatatatttaaaaagatgtaaaaaaaagagctgaagaaaatcatgtgtgatctctcagcagaatagatttattatttgtattgcttgcagaataaagcctatccttgaaagctctgaatcatgggcaagaggctcagtggtatctggaggacagggcactggccactgcagtcaccatcttctgccaggaagcctgcacctcaggggtgaattctttgccaaagtgaatggccagcacggtgaccagcacgttgcccaggagctgtgggaggaagataagaggtatgaacatgattagcaaaagggcctagcttggactcagaataatccagccttatcccaaccataaaataaaagcagaatggtagctggattgtagctgctattagcaatatgaaacctcttacatcagttacaatttatatgcagaaatatttatatgcagaaatattgctattgccttaacccagaaattatcactgttattctttagaatggtgcaaagaggcatgatacattgtatcattattgccctgaaagaaagagattagggaaagtattagaaataagataaacaaaaaagtatattaaaagaagaaagcattttttaaaattacaaatgcaaaattaccctgatttggtcaatatgtgtaccctgttacttctccccttcctatgacatgaacttaaccatagaaaagaaggggaaagaaaacatcaagggtcccatagactcaccttgaagttctcaggatccacatgcagcttgtcacagtgcagttcactcagctgggcaaaggtgcccttgagatcatccaggtgctttatggcatctcccaaggaagtcagcaccttcttgccatgtgccttgactttggggttgcccatgatggcagaggcagaggacaggttgccaaagctgtcaaagaacctctgggtccatgggtagacaaccaggagcctgtgagattgacaagaacagtttgacagtcagaaggtgccacaaatcctgagaagcaacctggacttttgccaggcacagggtccttccttccctcccttgtcctggtcaccagagcctaccttcccagggtttctcctccagcatcttccacattcaccttgtcccacaggcttgtgatagtagccttgtcctcctctgtgaaatgacccatggtgtctgtttgaggttgctagtgaacacagttgtgtcagaagcaaatgtaagcaatagatggctctgccctgacttttatgcccagccctggctcctgccctccctgctcctgggagtagattggccaaccctagggtgtggctccacagggtgaggtctaagtgatgacagccgtacctgtccttggctcttctggcactggcttaggagttggacttcaaaccctcagccctccctctaagatatatctcttggccccataccatcagtacaaattgctactaaaaacatcctcctttgcaagtgtatttacgacggtatcgatgtatgtgagcatgtgtcctctaacagcacaggccttttgccacctagctgtccaggggtgccttaaaatggcaaacaaggtttgttttcttttcctgttttcatgccttcctcttccatatccttgtttcatattaatacatgtgtatagatcctaaaaatctatacacatgtattaataaagcctgattctgccgcttctaggtatagaggccacctgcaagataaatatttgattcacaataactaatcattctatggcaattgataacaacaaatatatatatatatatatatatacgtatatgtgtatatatatatatatattcaggaaataatatattctagaatatgtcacattctgtctcaggcatccattttctttatgatgccgtttgaggtggagttttagtcaggtggtcagcttctccttttttttgccatctgccctgtaagcatcctgctggggacccagataggagtcatcactctaggctgagaacatctgggcacacaccctaagcctcagcatgactcatcatgactcagcattgctgtgcttgagccagaaggtttgcttagaaggttacacagaaccagaaggcgggggtggggcactgaccccgacaggggcctggccagaactgctcatgcttggactatgggaggtcactaatggagacacacagaaatgtaacaggaactaagggaattccggtgccctgcttaggagcttaatctttaatgaaagctaagctttcattaaaaaaagtctaaccagctgcattcgactttgactgcagcagctggttagaaggttctactggaggagggtcccagcccattgctaaattaacatcaggctctgagactggcagtatatctctaacagtggttgatgctatcttctggaacttgcctgctacattgagaccactgacccatacataggaagcccatagctctgtcctgaactgttaggccactggtccagagagtgtgcatctcctttgatcctcataataaccctatgagatagacacaattattactcttactttatagatgatgatcctgaaaacataggagtcaaggcacttgcccctagctgggggtataggggagcagtcccatgtagtagtagaatgaaaaatgctgctatgctgtgcctcccccacctttcccatgtctgccctctactcatggtctatctctcctggctcctgggagtcatggactccacccagcaccaccaacctgacctaaccacctatctgagcctgccagcctataacccatctgggccctgatagctggtggccagccctgaccccaccccaccctccctggaacctctgatagacacatctggcacaccagctcgcaaagtcaccgtgagggtcttgtgtttgctgagtcaaaattccttgaaatccaagtccttagagactcctgctcccaaatttacagtcatagacttcttcatggctgtctcctttatccacagaatgattcctttgcttcattgccccatccatctgatcctcctcatcagtgcagcacagggcccatgagcagtagctgcagagtctcacataggtctggcactgcctctgacatgtccgaccttaggcaaatgcttgactcttctgagctcggatcccttgagctcaggaggtcaaggctgcagtgagacatgatcttgccactgcactccagcctggacagcagagtgaaaccttgcctcacgaaacagaatacaaaaacaaacaaacaaaaaactgctccgcaatgcgcttccttgatgctctaccacataggtctgggtactttgtacacattatctcattgctgttcataattgttagattaattttgtaatattgatattattcctagaaagctgaggcctcaagatgataacttttattttctggacttgtaatagctttctcttgtattcaccatgttgtaactttcttagagtagtaacaatataaagttattgtgagtttttgcaaacacagcaaacacaacgacccatatagacattgatgtgaaattgtctattgtcaatttatgggaaaacaagtatgtactttttctactaagccattgaaacaggaataacagaacaagattgaaagaatacattttccgaaattacttgagtattatacaaagacaagcacgtggacctgggaggagggttattgtccatgactggtgtgtggagacaaatgcaggtttataatagatgggatggcatctagcgcaatgactttgccatcacttttagagagctcttgggggccccagtacacaagaggggacgcagggtatatgtagacatctcattctttttcttagtgtgagaataagaatagccatgacctgagtttatagacaatgagcccttttctctctcccactcagcagctatgagatggcttgccctgcctctctactaggctgactcactccaaggcccagcaatgggcagggctctgtcagggctttgatagcactatctgcagagccagggccgagaaggggtggactccagagactctccctcccattcccgagcagggtttgcttatttatgcatttaaatgatatatttattttaaaagaaataacaggagactgcccagccctggctgtgacatggaaactatgtagaatattttgggttccatttttttttccttctttcagttagaggaaaaggggctcactgcacatacactagacagaaagtcaggagctttgaatccaagcctgatcatttccatgtcatactgagaaagtccccacccttctctgagcctcagtttctctttttataagtaggagtctggagtaaatgatttccaatggctctcatttcaatacaaaatttccgtttattaaatgcatgagcttccgttactccaagactgagaaggaaattgaacctgagactcattgactggcaagatgtccccagaggctctcattcagcaataaaattctcaccttcacccaggcccactagtgtcagatttgcatgcgttaacgcggccgcatcgatgccgtagtacctttaagaccaatgacttacaaggcagctgtagatcttagccactttttaaaagaaaaggggggactggaagggctaattcactcccaaagaagacaagatagatctgctttttgcctgtactgggtctctctggttagaccagatctgagcctgggagctctctggctaactagggaacccactgcttaagcctcaataaagcttcagctgctcgagctagcagatctttttccctctgccaaaaattatggggacatcatgaagccccttgagcatctgacttctggctaataaaggaaatttattttcattgcaatagtgtgttggaattttttgtgtctctcactcggaaggacatatgggagggcaaatcatttaaaacatcagaatgagtatttggtttagagtttggcaacatatgcccatatgctggctgccatgaacaaaggttggctataaagaggtcatcagtatatgaaacagccccctgctgtccattccttattccatagaaaagccttgacttgaggttagattttttttatattttgttttgtgttatttttttctttaacatccctaaaattttccttacatgttttactagccagatttttcctcctctcctgactactcccagtcatagctgtccctcttctcttatggagatccctcgacctgcagcccaagcttggcgtaatcatggtcatagctgtttcctgtgtgaaattgttatccgctcacaattccacacaacatacgagccggaagcataaagtgtaaagcctggggtgcctaatgagtgagctaactcacattaattgcgttgcgctcactgcccgctttccagtcgggaaacctgtcgtgccagcggatccgcatctcaattagtcagcaaccatagtcccgcccctaactccgcccatcccgcccctaactccgcccagttccgcccattctccgccccatggctgactaattttttttatttatgcagaggccgaggccgcctcggcctctgagctattccagaagtagtgaggaggcttttttggaggcctaggcttttgcaaaaagctgtcgactgcagaggcctgcatgcaagcttggcgtaatcatggtcatagctgtttcctgtgtgaaattgttatccgctcacaattccacacaacatacgagccggaagcataaagtgtaaagcctggggtgcctaatgagtgagctaactcacattaattgcgttgcgctcactgcccgctttccagtcgggaaacctgtcgtgccagctgcattaatgaatcggccaacgcgcggggagaggcggtttgcgtattgggcgctcttccgcttcctcgctcactgactcgctgcgctcggtcgttcggctgcggcgagcggtatcagctcactcaaaggcggtaatacggttatccacagaatcaggggataacgcaggaaagaacatgtgagcaaaaggccagcaaaaggccaggaaccgtaaaaaggccgcgttgctggcgtttttccataggctccgcccccctgacgagcatcacaaaaatcgacgctcaagtcagaggtggcgaaacccgacaggactataaagataccaggcgtttccccctggaagctccctcgtgcgctctcctgttccgaccctgccgcttaccggatacctgtccgcctttctcccttcgggaagcgtggcgctttctcatagctcacgctgtaggtatctcagttcggtgtaggtcgttcgctccaagctgggctgtgtgcacgaaccccccgttcagcccgaccgctgcgccttatccggtaactatcgtcttgagtccaacccggtaagacacgacttatcgccactggcagcagccactggtaacaggattagcagagcgaggtatgtaggcggtgctacagagttcttgaagtggtggcctaactacggctacactagaagaacagtatttggtatctgcgctctgctgaagccagttaccttcggaaaaagagttggtagctcttgatccggcaaacaaaccaccgctggtagcggtggtttttttgtttgcaagcagcagattacgcgcagaaaaaaaggatctcaagaagatcctttgatcttttctacggggtctgacgctcagtggaacgaaaactcacgttaagggattttggtcatgagattatcaaaaaggatcttcacctagatccttttaaattaaaaatgaagttttaaatcaatctaaagtatatatgagtaaacttggtctgacagttaccaatgcttaatcagtgaggcacctatctcagcgatctgtctatttcgttcatccatagttgcctgactccccgtcgtgtagataactacgatacgggagggcttaccatctggccccagtgctgcaatgataccgcgagacccacgctcaccggctccagatttatcagcaataaaccagccagccggaagggccgagcgcagaagtggtcctgcaactttatccgcctccatccagtctattaattgttgccgggaagctagagtaagtagttcgccagttaatagtttgcgcaacgttgttgccattgctacaggcatcgtggtgtcacgctcgtcgtttggtatggcttcattcagctccggttcccaacgatcaaggcgagttacatgatcccccatgttgtgcaaaaaagcggttagctccttcggtcctccgatcgttgtcagaagtaagttggccgcagtgttatcactcatggttatggcagcactgcataattctcttactgtcatgccatccgtaagatgcttttctgtgactggtgagtactcaaccaagtcattctgagaatagtgtatgcggcgaccgagttgctcttgcccggcgtcaatacgggataataccgcgccacatagcagaactttaaaagtgctcatcattggaaaacgttcttcggggcgaaaactctcaaggatcttaccgctgttgagatccagttcgatgtaacccactcgtgcacccaactgatcttcagcatcttttactttcaccagcgtttctgggtgagcaaaaacaggaaggcaaaatgccgcaaaaaagggaataagggcgacacggaaatgttgaatactcatactcttcctttttcaatattattgaagcatttatcagggttattgtctcatgagcggatacatatttgaatgtatttagaaaaataaacaaataggggttccgcgcacatttccccgaaaagtgccacctgacgtctaagaaaccattattatcatgacattaacctataaaaataggcgtatcacgaggccctttcgtctcgcgcgtttcggtgatgacggtgaaaacctctgacacatgcagctcccggagacggtcacagcttgtctgtaagcggatgccgggagcagacaagcccgtcagggcgcgtcagcgggtgttggcgggtgtcggggctggcttaactatgcggcatcagagcagattgtactgagagtgcaccatatgcggtgtgaaataccgcacagatgcgtaaggagaaaataccgcatcaggcgccattcgccattcaggctgcgcaactgttgggaagggcgatcggtgcgggcctcttcgctattacgccagctggcgaaagggggatgtgctgcaaggcgattaagttgggtaacgccagggttttcccagtcacgacgttgtaaaacgacggccagtgaattc

SEQ ID NO: 16 - DNA, 11678 bp, Artificial Sequence
  Synthetic: TL20d-r7SKM1/sh734-rGbGM
ggccgcctcggccaaacagcccttgagtttaccactccctatcagtgatagagaaaagtgaaagtcgagtttaccactccctatcagtgatagagaaaagtgaaagtcgagtttaccactccctatcagtgatagagaaaagtgaaagtcgagtttaccactccctatcagtgatagagaaaagtgaaagtcgagtttaccagtccctatcagtgatagagaaaagtgaaagtcgagtttaccactccctatcagtgatagagaaaagtgaaagtcgagtttaccactccctatcagtgatagagaaaagtgaaagtcgagctcgccatgggaggcgtggcctgggcgggactggggagtggcgagccctcagatcctgcatataagcagctgctttttgcctgtactgggtctctctggttagaccagatctgagcctgggagctctctggctaactagggaacccactgcttaagcctcaataaagcttgccttgagtgcttcaagtagtgtgtgcccgtctgttgtgtgactctggtaactagagatccctcagacccttttagtcagtgtggaaaatctctagcagtggcgcccgaacagggacttgaaagcgaaagggaaaccagaggagctctctcgacgcaggactcggcttgctgaagcgcgcacggcaagaggcgaggggcggcgactggtgagtacgccaaaaattttgactagcggaggctagaaggagagagatgggtgcgagagcgtcagtattaagcgggggagaattagatcgcgatgggaaaaaattcggttaaggccagggggaaagaaaaaatataaattaaaacatatagtatgggcaagcagggagctagaacgattcgcagttaatactggcctgttagaaacatcagaaggctgtagacaaatactgggacagctacaaccatcccttcagacaggatcagaagaacttagatcattatataatacagtagcaaccctctattgtgtgcatcaaaggatagagataaaagacaccaaggaagctttagacaagatagaggaagagcaaaacaaaagtaagaaaaaagcacagcaagcagcaggatcttcagacctggaaattccctacaatccccaaagtcaaggagtagtagaatctatgaataaagaattaaagaaaattataggacaggtaagagatcaggctgaacatcttaagacagcagtacaaatggcagtattcatccacaattttaaaagaaaaggggggattggggggtacagtgcaggggaaagaatagtagacataatagcaacagacatacaaactaaagaattacaaaaacaaattacaaaaattcaaaattttcgggtttattacagggacagcagaaatccactttggaaaggaccagcaaagctcctctggaaaggtgaaggggcagtagtaatacaagataatagtgacataaaagtagtgccaagaagaaaagcaaagatcattagggattatggaaaacagatggcaggtgatgattgtgtggcaagtagacaggatgaggattagaacatggaaaagtttagtaaaacaccataaggaggagatatgagggacaattggagaagtgaattatataaatataaagtagtaaaaattgaaccattaggagtagcacccaccaaggcaaagagaagagtggtgcagagagaaaaaagagcagtgggaataggagctttgttccttgggttcttgggagcagcaggaagcactatgggcgcagcgtcaatgacgctgacggtacaggccagacaattattgtctggtatagtgcagcagcagaacaatttgctgagggctattgaggcgcaacagcatctgttgcaactcacagtctggggcatcaagcagctccaggcaagaatcctggctgtggaaagatacctaaaggatcaacagctcctggggatttggggttgctctggaaaactcatttgcaccactgctgtgccttggaatgctagttggagtaataaatctctggaacagatttggaatcacacgacctggatggagtgggacagagaaattaacaattacacaagcttaatacactccttaattgaagaatcgcaaaaccagcaagaaaagaatgaacaagaattattggaattagataaatgggcaagtttgtggaattggtttaacataacaaattggctgtggtatataaaattattcataatgatagtaggaggcttggtaggtttaagaatagtttttgctgtactttctatagtgaatagagttaggcagggatattcaccattatcgtttcagacccacctcccaaccccgaggggaccgagctcaagcttcgaagcggccgcaaaaaaggatatgcccttgactatgtcggacaaatagtcaagggcatatcctgaggtacccaggcggcgcacaagctatataaacctgaaggaaatctcaactttacacttaggtcaagttacttatcgtactagagcttcagcaggaaatttaactaaaatctaatttaaccagcatagcaaatatcatttattcccaaaatgctaaagtttgagataaacggacttgatttccggctgttttgacactatccagaatgccggtactatgggtggggcagtagcccgactgcacgtcgaacgcgtggggatcctctagagtcgagctcgcgaggatcatcaccggtgctagccggagccagaagcaccataagggacatgataagggagccagcagacctctgatctcttcctgaatgctaatcttaaacatcctgaggaagaatgggacttccatttggggtgggcctatgatagggtaataagacagtagtgaatatcaagctacaaaaagccccctttcaaattcttctcagtcctaacttttcatactaagcccagtccttccaaagcagactgtgaaagagtgatagttccgggagactagcaccggctagccgagcttggaacactttcccttcattaagaaccatccttgctactcagctgcaatcaatccagcccccaggtcttcactgaaccttttcccatctcttccaaaacatctgtttctgagaagtcctgtcctatagaggtctttcttcccaccggatttctcctacaccatttactcccacttgcagaactcccgtgtacaagtgtctttactgcttttatttgctcaacaaaatgcacatctcatataaaaataaatgaggagcatgcacacaccacaaacacaaacaggcatgcagaaatacacatacacacttccctcaatataaaccctttgtggctcatatatttaaaaagatgtaaaaaaaagagctgaagaaaatcatgtgtgatctctcagcagaatagatttattatttgtattgcttgcagaataaagcctatccttgaaagctctgaatcatgggcaagaggctcagtggtatctggaggacagggcactggccactgcagtcaccatcttctgccaggaagcctgcacctcaggggtgaattctttgccaaagtgaatggccagcacggtgaccagcacgttgcccaggagctgtgggaggaagataagaggtatgaacatgattagcaaaagggcctagcttggactcagaataatccagccttatcccaaccataaaataaaagcagaatggtagctggattgtagctgctattagcaatatgaaacctcttacatcagttacaatttatatgcagaaatatttatatgcagaaatattgctattgccttaacccagaaattatcactgttattctttagaatggtgcaaagaggcatgatacattgtatcattattgccctgaaagaaagagattagggaaagtattagaaataagataaacaaaaaagtatattaaaagaagaaagcattttttaaaattacaaatgcaaaattaccctgatttggtcaatatgtgtaccctgttacttctccccttcctatgacatgaacttaaccatagaaaagaaggggaaagaaaacatcaagggtcccatagactcaccttgaagttctcaggatccacatgcagcttgtcacagtgcagttcactcagctgggcaaaggtgcccttgagatcatccaggtgctttatggcatctcccaaggaagtcagcaccttcttgccatgtgccttgactttggggttgcccatgatggcagaggcagaggacaggttgccaaagctgtcaaagaacctctgggtccatgggtagacaaccaggagcctgtgagattgacaagaacagtttgacagtcagaaggtgccacaaatcctgagaagcaacctggacttttgccaggcacagggtccttccttccctcccttgtcctggtcaccagagcctaccttcccagggtttctcctccagcatcttccacattcaccttgtcccacaggcttgtgatagtagccttgtcctcctctgtgaaatgacccatggtgtctgtttgaggttgctagtgaacacagttgtgtcagaagcaaatgtaagcaatagatggctctgccctgacttttatgcccagccctggctcctgccctccctgctcctgggagtagattggccaaccctagggtgtggctccacagggtgaggtctaagtgatgacagccgtacctgtccttggctcttctggcactggcttaggagttggacttcaaaccctcagccctccctctaagatatatctcttggccccataccatcagtacaaattgctactaaaaacatcctcctttgcaagtgtatttacgacggtatcgatgtatgtgagcatgtgtcctctaacagcacaggccttttgccacctagctgtccaggggtgccttaaaatggcaaacaaggtttgttttcttttcctgttttcatgccttcctcttccatatccttgtttcatattaatacatgtgtatagatcctaaaaatctatacacatgtattaataaagcctgattctgccgcttctaggtatagaggccacctgcaagataaatatttgattcacaataactaatcattctatggcaattgataacaacaaatatatatatatatatatatatacgtatatgtgtatatatatatatatattcaggaaataatatattctagaatatgtcacattctgtctcaggcatccattttctttatgatgccgtttgaggtggagttttagtcaggtggtcagcttctccttttttttgccatctgccctgtaagcatcctgctggggacccagataggagtcatcactctaggctgagaacatctgggcacacaccctaagcctcagcatgactcatcatgactcagcattgctgtgcttgagccagaaggtttgcttagaaggttacacagaaccagaaggcgggggtggggcactgaccccgacaggggcctggccagaactgctcatgcttggactatgggaggtcactaatggagacacacagaaatgtaacaggaactaagggaattccggtgccctgcttaggagcttaatctttaatgaaagctaagctttcattaaaaaaagtctaaccagctgcattcgactttgactgcagcagctggttagaaggttctactggaggagggtcccagcccattgctaaattaacatcaggctctgagactggcagtatatctctaacagtggttgatgctatcttctggaacttgcctgctacattgagaccactgacccatacataggaagcccatagctctgtcctgaactgttaggccactggtccagagagtgtgcatctcctttgatcctcataataaccctatgagatagacacaattattactcttactttatagatgatgatcctgaaaacataggagtcaaggcacttgcccctagctgggggtataggggagcagtcccatgtagtagtagaatgaaaaatgctgctatgctgtgcctcccccacctttcccatgtctgccctctactcatggtctatctctcctggctcctgggagtcatggactccacccagcaccaccaacctgacctaaccacctatctgagcctgccagcctataacccatctgggccctgatagctggtggccagccctgaccccaccccaccctccctggaacctctgatagacacatctggcacaccagctcgcaaagtcaccgtgagggtcttgtgtttgctgagtcaaaattccttgaaatccaagtccttagagactcctgctcccaaatttacagtcatagacttcttcatggctgtctcctttatccacagaatgattcctttgcttcattgccccatccatctgatcctcctcatcagtgcagcacagggcccatgagcagtagctgcagagtctcacataggtctggcactgcctctgacatgtccgaccttaggcaaatgcttgactcttctgagctcggatcccttgagctcaggaggtcaaggctgcagtgagacatgatcttgccactgcactccagcctggacagcagagtgaaaccttgcctcacgaaacagaatacaaaaacaaacaaacaaaaaactgctccgcaatgcgcttccttgatgctctaccacataggtctgggtactttgtacacattatctcattgctgttcataattgttagattaattttgtaatattgatattattcctagaaagctgaggcctcaagatgataacttttattttctggacttgtaatagctttctcttgtattcaccatgttgtaactttcttagagtagtaacaatataaagttattgtgagtttttgcaaacacagcaaacacaacgacccatatagacattgatgtgaaattgtctattgtcaatttatgggaaaacaagtatgtactttttctactaagccattgaaacaggaataacagaacaagattgaaagaatacattttccgaaattacttgagtattatacaaagacaagcacgtggacctgggaggagggttattgtccatgactggtgtgtggagacaaatgcaggtttataatagatgggatggcatctagcgcaatgactttgccatcacttttagagagctcttgggggccccagtacacaagaggggacgcagggtatatgtagacatctcattctttttcttagtgtgagaataagaatagccatgacctgagtttatagacaatgagcccttttctctctcccactcagcagctatgagatggcttgccctgcctctctactaggctgactcactccaaggcccagcaatgggcagggctctgtcagggctttgatagcactatctgcagagccagggccgagaaggggtggactccagagactctccctcccattcccgagcagggtttgcttatttatgcatttaaatgatatatttattttaaaagaaataacaggagactgcccagccctggctgtgacatggaaactatgtagaatattttgggttccatttttttttccttctttcagttagaggaaaaggggctcactgcacatacactagacagaaagtcaggagctttgaatccaagcctgatcatttccatgtcatactgagaaagtccccacccttctctgagcctcagtttctctttttataagtaggagtctggagtaaatgatttccaatggctctcatttcaatacaaaatttccgtttattaaatgcatgagcttccgttactccaagactgagaaggaaattgaacctgagactcattgactggcaagatgtccccagaggctctcattcagcaataaaattctcaccttcacccaggcccactagtgtcagatttgcatgcgttaacgcggccgcatcgatgccgtagtacctttaagaccaatgacttacaaggcagctgtagatcttagccactttttaaaagaaaaggggggactggaagggctaattcactcccaaagaagacaagatagatctgctttttgcctgtactgggtctctctggttagaccagatctgagcctgggagctctctggctaactagggaacccactgcttaagcctcaataaagcttcagctgctcgagctagcagatctttttccctctgccaaaaattatggggacatcatgaagccccttgagcatctgacttctggctaataaaggaaatttattttcattgcaatagtgtgttggaattttttgtgtctctcactcggaaggacatatgggagggcaaatcatttaaaacatcagaatgagtatttggtttagagtttggcaacatatgcccatatgctggctgccatgaacaaaggttggctataaagaggtcatcagtatatgaaacagccccctgctgtccattccttattccatagaaaagccttgacttgaggttagattttttttatattttgttttgtgttatttttttctttaacatccctaaaattttccttacatgttttactagccagatttttcctcctctcctgactactcccagtcatagctgtccctcttctcttatggagatccctcgacctgcagcccaagcttggcgtaatcatggtcatagctgtttcctgtgtgaaattgttatccgctcacaattccacacaacatacgagccggaagcataaagtgtaaagcctggggtgcctaatgagtgagctaactcacattaattgcgttgcgctcactgcccgctttccagtcgggaaacctgtcgtgccagcggatccgcatctcaattagtcagcaaccatagtcccgcccctaactccgcccatcccgcccctaactccgcccagttccgcccattctccgccccatggctgactaattttttttatttatgcagaggccgaggccgcctcggcctctgagctattccagaagtagtgaggaggcttttttggaggcctaggcttttgcaaaaagctgtcgactgcagaggcctgcatgcaagcttggcgtaatcatggtcatagctgtttcctgtgtgaaattgttatccgctcacaattccacacaacatacgagccggaagcataaagtgtaaagcctggggtgcctaatgagtgagctaactcacattaattgcgttgcgctcactgcccgctttccagtcgggaaacctgtcgtgccagctgcattaatgaatcggccaacgcgcggggagaggcggtttgcgtattgggcgctcttccgcttcctcgctcactgactcgctgcgctcggtcgttcggctgcggcgagcggtatcagctcactcaaaggcggtaatacggttatccacagaatcaggggataacgcaggaaagaacatgtgagcaaaaggccagcaaaaggccaggaaccgtaaaaaggccgcgttgctggcgtttttccataggctccgcccccctgacgagcatcacaaaaatcgacgctcaagtcagaggtggcgaaacccgacaggactataaagataccaggcgtttccccctggaagctccctcgtgcgctctcctgttccgaccctgccgcttaccggatacctgtccgcctttctcccttcgggaagcgtggcgctttctcatagctcacgctgtaggtatctcagttcggtgtaggtcgttcgctccaagctgggctgtgtgcacgaaccccccgttcagcccgaccgctgcgccttatccggtaactatcgtcttgagtccaacccggtaagacacgacttatcgccactggcagcagccactggtaacaggattagcagagcgaggtatgtaggcggtgctacagagttcttgaagtggtggcctaactacggctacactagaagaacagtatttggtatctgcgctctgctgaagccagttaccttcggaaaaagagttggtagctcttgatccggcaaacaaaccaccgctggtagcggtggtttttttgtttgcaagcagcagattacgcgcagaaaaaaaggatctcaagaagatcctttgatcttttctacggggtctgacgctcagtggaacgaaaactcacgttaagggattttggtcatgagattatcaaaaaggatcttcacctagatccttttaaattaaaaatgaagttttaaatcaatctaaagtatatatgagtaaacttggtctgacagttaccaatgcttaatcagtgaggcacctatctcagcgatctgtctatttcgttcatccatagttgcctgactccccgtcgtgtagataactacgatacgggagggcttaccatctggccccagtgctgcaatgataccgcgagacccacgctcaccggctccagatttatcagcaataaaccagccagccggaagggccgagcgcagaagtggtcctgcaactttatccgcctccatccagtctattaattgttgccgggaagctagagtaagtagttcgccagttaatagtttgcgcaacgttgttgccattgctacaggcatcgtggtgtcacgctcgtcgtttggtatggcttcattcagctccggttcccaacgatcaaggcgagttacatgatcccccatgttgtgcaaaaaagcggttagctccttcggtcctccgatcgttgtcagaagtaagttggccgcagtgttatcactcatggttatggcagcactgcataattctcttactgtcatgccatccgtaagatgcttttctgtgactggtgagtactcaaccaagtcattctgagaatagtgtatgcggcgaccgagttgctcttgcccggcgtcaatacgggataataccgcgccacatagcagaactttaaaagtgctcatcattggaaaacgttcttcggggcgaaaactctcaaggatcttaccgctgttgagatccagttcgatgtaacccactcgtgcacccaactgatcttcagcatcttttactttcaccagcgtttctgggtgagcaaaaacaggaaggcaaaatgccgcaaaaaagggaataagggcgacacggaaatgttgaatactcatactcttcctttttcaatattattgaagcatttatcagggttattgtctcatgagcggatacatatttgaatgtatttagaaaaataaacaaataggggttccgcgcacatttccccgaaaagtgccacctgacgtctaagaaaccattattatcatgacattaacctataaaaataggcgtatcacgaggccctttcgtctcgcgcgtttcggtgatgacggtgaaaacctctgacacatgcagctcccggagacggtcacagcttgtctgtaagcggatgccgggagcagacaagcccgtcagggcgcgtcagcgggtgttggcgggtgtcggggctggcttaactatgcggcatcagagcagattgtactgagagtgcaccatatgcggtgtgaaataccgcacagatgcgtaaggagaaaataccgcatcaggcgccattcgccattcaggctgcgcaactgttgggaagggcgatcggtgcgggcctcttcgctattacgccagctggcgaaagggggatgtgctgcaaggcgattaagttgggtaacgccagggttttcccagtcacgacgttgtaaaacgacggccagtgaattc

SEQ ID NO: 17 - DNA, 11681 bp, Artificial Sequence
  Synthetic: TL20d-r7SK/sh734-rGbGM
ggccgcctcggccaaacagcccttgagtttaccactccctatcagtgatagagaaaagtgaaagtcgagtttaccactccctatcagtgatagagaaaagtgaaagtcgagtttaccactccctatcagtgatagagaaaagtgaaagtcgagtttaccactccctatcagtgatagagaaaagtgaaagtcgagtttaccagtccctatcagtgatagagaaaagtgaaagtcgagtttaccactccctatcagtgatagagaaaagtgaaagtcgagtttaccactccctatcagtgatagagaaaagtgaaagtcgagctcgccatgggaggcgtggcctgggcgggactggggagtggcgagccctcagatcctgcatataagcagctgctttttgcctgtactgggtctctctggttagaccagatctgagcctgggagctctctggctaactagggaacccactgcttaagcctcaataaagcttgccttgagtgcttcaagtagtgtgtgcccgtctgttgtgtgactctggtaactagagatccctcagacccttttagtcagtgtggaaaatctctagcagtggcgcccgaacagggacttgaaagcgaaagggaaaccagaggagctctctcgacgcaggactcggcttgctgaagcgcgcacggcaagaggcgaggggcggcgactggtgagtacgccaaaaattttgactagcggaggctagaaggagagagatgggtgcgagagcgtcagtattaagcgggggagaattagatcgcgatgggaaaaaattcggttaaggccagggggaaagaaaaaatataaattaaaacatatagtatgggcaagcagggagctagaacgattcgcagttaatactggcctgttagaaacatcagaaggctgtagacaaatactgggacagctacaaccatcccttcagacaggatcagaagaacttagatcattatataatacagtagcaaccctctattgtgtgcatcaaaggatagagataaaagacaccaaggaagctttagacaagatagaggaagagcaaaacaaaagtaagaaaaaagcacagcaagcagcaggatcttcagacctggaaattccctacaatccccaaagtcaaggagtagtagaatctatgaataaagaattaaagaaaattataggacaggtaagagatcaggctgaacatcttaagacagcagtacaaatggcagtattcatccacaattttaaaagaaaaggggggattggggggtacagtgcaggggaaagaatagtagacataatagcaacagacatacaaactaaagaattacaaaaacaaattacaaaaattcaaaattttcgggtttattacagggacagcagaaatccactttggaaaggaccagcaaagctcctctggaaaggtgaaggggcagtagtaatacaagataatagtgacataaaagtagtgccaagaagaaaagcaaagatcattagggattatggaaaacagatggcaggtgatgattgtgtggcaagtagacaggatgaggattagaacatggaaaagtttagtaaaacaccataaggaggagatatgagggacaattggagaagtgaattatataaatataaagtagtaaaaattgaaccattaggagtagcacccaccaaggcaaagagaagagtggtgcagagagaaaaaagagcagtgggaataggagctttgttccttgggttcttgggagcagcaggaagcactatgggcgcagcgtcaatgacgctgacggtacaggccagacaattattgtctggtatagtgcagcagcagaacaatttgctgagggctattgaggcgcaacagcatctgttgcaactcacagtctggggcatcaagcagctccaggcaagaatcctggctgtggaaagatacctaaaggatcaacagctcctggggatttggggttgctctggaaaactcatttgcaccactgctgtgccttggaatgctagttggagtaataaatctctggaacagatttggaatcacacgacctggatggagtgggacagagaaattaacaattacacaagcttaatacactccttaattgaagaatcgcaaaaccagcaagaaaagaatgaacaagaattattggaattagataaatgggcaagtttgtggaattggtttaacataacaaattggctgtggtatataaaattattcataatgatagtaggaggcttggtaggtttaagaatagtttttgctgtactttctatagtgaatagagttaggcagggatattcaccattatcgtttcagacccacctcccaaccccgaggggaccgagctcaagcttcgaagcggccgcacaaaaaaggatatgcccttgactatgtcggacaaatagtcaagggcatatcctgaggtacccaggcggcgcacaagctatataaacctgaaggaaatctcaactttacacttaggtcaagttacttatcgtactagagcttcagcaggaaatttaactaaaatctaatttaaccagcatagcaaatatcatttattcccaaaatgctaaagtttgagataaacggacttgatttccggctgttttgacactatccagaatgccttgcagatgggtggggcatgctaaatactgcacgtcgatacgcgtggggatcctctagagtcgagctcgcgaggatcatcaccggtgctagccggagccagaagcaccataagggacatgataagggagccagcagacctctgatctcttcctgaatgctaatcttaaacatcctgaggaagaatgggacttccatttggggtgggcctatgatagggtaataagacagtagtgaatatcaagctacaaaaagccccctttcaaattcttctcagtcctaacttttcatactaagcccagtccttccaaagcagactgtgaaagagtgatagttccgggagactagcaccggctagccgagcttggaacactttcccttcattaagaaccatccttgctactcagctgcaatcaatccagcccccaggtcttcactgaaccttttcccatctcttccaaaacatctgtttctgagaagtcctgtcctatagaggtctttcttcccaccggatttctcctacaccatttactcccacttgcagaactcccgtgtacaagtgtctttactgcttttatttgctcaacaaaatgcacatctcatataaaaataaatgaggagcatgcacacaccacaaacacaaacaggcatgcagaaatacacatacacacttccctcaatataaaccctttgtggctcatatatttaaaaagatgtaaaaaaaagagctgaagaaaatcatgtgtgatctctcagcagaatagatttattatttgtattgcttgcagaataaagcctatccttgaaagctctgaatcatgggcaagaggctcagtggtatctggaggacagggcactggccactgcagtcaccatcttctgccaggaagcctgcacctcaggggtgaattctttgccaaagtgaatggccagcacggtgaccagcacgttgcccaggagctgtgggaggaagataagaggtatgaacatgattagcaaaagggcctagcttggactcagaataatccagccttatcccaaccataaaataaaagcagaatggtagctggattgtagctgctattagcaatatgaaacctcttacatcagttacaatttatatgcagaaatatttatatgcagaaatattgctattgccttaacccagaaattatcactgttattctttagaatggtgcaaagaggcatgatacattgtatcattattgccctgaaagaaagagattagggaaagtattagaaataagataaacaaaaaagtatattaaaagaagaaagcattttttaaaattacaaatgcaaaattaccctgatttggtcaatatgtgtaccctgttacttctccccttcctatgacatgaacttaaccatagaaaagaaggggaaagaaaacatcaagggtcccatagactcaccttgaagttctcaggatccacatgcagcttgtcacagtgcagttcactcagctgggcaaaggtgcccttgagatcatccaggtgctttatggcatctcccaaggaagtcagcaccttcttgccatgtgccttgactttggggttgcccatgatggcagaggcagaggacaggttgccaaagctgtcaaagaacctctgggtccatgggtagacaaccaggagcctgtgagattgacaagaacagtttgacagtcagaaggtgccacaaatcctgagaagcaacctggacttttgccaggcacagggtccttccttccctcccttgtcctggtcaccagagcctaccttcccagggtttctcctccagcatcttccacattcaccttgtcccacaggcttgtgatagtagccttgtcctcctctgtgaaatgacccatggtgtctgtttgaggttgctagtgaacacagttgtgtcagaagcaaatgtaagcaatagatggctctgccctgacttttatgcccagccctggctcctgccctccctgctcctgggagtagattggccaaccctagggtgtggctccacagggtgaggtctaagtgatgacagccgtacctgtccttggctcttctggcactggcttaggagttggacttcaaaccctcagccctccctctaagatatatctcttggccccataccatcagtacaaattgctactaaaaacatcctcctttgcaagtgtatttacgacggtatcgatgtatgtgagcatgtgtcctctaacagcacaggccttttgccacctagctgtccaggggtgccttaaaatggcaaacaaggtttgttttcttttcctgttttcatgccttcctcttccatatccttgtttcatattaatacatgtgtatagatcctaaaaatctatacacatgtattaataaagcctgattctgccgcttctaggtatagaggccacctgcaagataaatatttgattcacaataactaatcattctatggcaattgataacaacaaatatatatatatatatatatatacgtatatgtgtatatatatatatatattcaggaaataatatattctagaatatgtcacattctgtctcaggcatccattttctttatgatgccgtttgaggtggagttttagtcaggtggtcagcttctccttttttttgccatctgccctgtaagcatcctgctggggacccagataggagtcatcactctaggctgagaacatctgggcacacaccctaagcctcagcatgactcatcatgactcagcattgctgtgcttgagccagaaggtttgcttagaaggttacacagaaccagaaggcgggggtggggcactgaccccgacaggggcctggccagaactgctcatgcttggactatgggaggtcactaatggagacacacagaaatgtaacaggaactaagggaattccggtgccctgcttaggagcttaatctttaatgaaagctaagctttcattaaaaaaagtctaaccagctgcattcgactttgactgcagcagctggttagaaggttctactggaggagggtcccagcccattgctaaattaacatcaggctctgagactggcagtatatctctaacagtggttgatgctatcttctggaacttgcctgctacattgagaccactgacccatacataggaagcccatagctctgtcctgaactgttaggccactggtccagagagtgtgcatctcctttgatcctcataataaccctatgagatagacacaattattactcttactttatagatgatgatcctgaaaacataggagtcaaggcacttgcccctagctgggggtataggggagcagtcccatgtagtagtagaatgaaaaatgctgctatgctgtgcctcccccacctttcccatgtctgccctctactcatggtctatctctcctggctcctgggagtcatggactccacccagcaccaccaacctgacctaaccacctatctgagcctgccagcctataacccatctgggccctgatagctggtggccagccctgaccccaccccaccctccctggaacctctgatagacacatctggcacaccagctcgcaaagtcaccgtgagggtcttgtgtttgctgagtcaaaattccttgaaatccaagtccttagagactcctgctcccaaatttacagtcatagacttcttcatggctgtctcctttatccacagaatgattcctttgcttcattgccccatccatctgatcctcctcatcagtgcagcacagggcccatgagcagtagctgcagagtctcacataggtctggcactgcctctgacatgtccgaccttaggcaaatgcttgactcttctgagctcggatcccttgagctcaggaggtcaaggctgcagtgagacatgatcttgccactgcactccagcctggacagcagagtgaaaccttgcctcacgaaacagaatacaaaaacaaacaaacaaaaaactgctccgcaatgcgcttccttgatgctctaccacataggtctgggtactttgtacacattatctcattgctgttcataattgttagattaattttgtaatattgatattattcctagaaagctgaggcctcaagatgataacttttattttctggacttgtaatagctttctcttgtattcaccatgttgtaactttcttagagtagtaacaatataaagttattgtgagtttttgcaaacacagcaaacacaacgacccatatagacattgatgtgaaattgtctattgtcaatttatgggaaaacaagtatgtactttttctactaagccattgaaacaggaataacagaacaagattgaaagaatacattttccgaaattacttgagtattatacaaagacaagcacgtggacctgggaggagggttattgtccatgactggtgtgtggagacaaatgcaggtttataatagatgggatggcatctagcgcaatgactttgccatcacttttagagagctcttgggggccccagtacacaagaggggacgcagggtatatgtagacatctcattctttttcttagtgtgagaataagaatagccatgacctgagtttatagacaatgagcccttttctctctcccactcagcagctatgagatggcttgccctgcctctctactaggctgactcactccaaggcccagcaatgggcagggctctgtcagggctttgatagcactatctgcagagccagggccgagaaggggtggactccagagactctccctcccattcccgagcagggtttgcttatttatgcatttaaatgatatatttattttaaaagaaataacaggagactgcccagccctggctgtgacatggaaactatgtagaatattttgggttccatttttttttccttctttcagttagaggaaaaggggctcactgcacatacactagacagaaagtcaggagctttgaatccaagcctgatcatttccatgtcatactgagaaagtccccacccttctctgagcctcagtttctctttttataagtaggagtctggagtaaatgatttccaatggctctcatttcaatacaaaatttccgtttattaaatgcatgagcttccgttactccaagactgagaaggaaattgaacctgagactcattgactggcaagatgtccccagaggctctcattcagcaataaaattctcaccttcacccaggcccactagtgtcagatttgcatgcgttaacgcggccgcatcgatgccgtagtacctttaagaccaatgacttacaaggcagctgtagatcttagccactttttaaaagaaaaggggggactggaagggctaattcactcccaaagaagacaagatagatctgctttttgcctgtactgggtctctctggttagaccagatctgagcctgggagctctctggctaactagggaacccactgcttaagcctcaataaagcttcagctgctcgagctagcagatctttttccctctgccaaaaattatggggacatcatgaagccccttgagcatctgacttctggctaataaaggaaatttattttcattgcaatagtgtgttggaattttttgtgtctctcactcggaaggacatatgggagggcaaatcatttaaaacatcagaatgagtatttggtttagagtttggcaacatatgcccatatgctggctgccatgaacaaaggttggctataaagaggtcatcagtatatgaaacagccccctgctgtccattccttattccatagaaaagccttgacttgaggttagattttttttatattttgttttgtgttatttttttctttaacatccctaaaattttccttacatgttttactagccagatttttcctcctctcctgactactcccagtcatagctgtccctcttctcttatggagatccctcgacctgcagcccaagcttggcgtaatcatggtcatagctgtttcctgtgtgaaattgttatccgctcacaattccacacaacatacgagccggaagcataaagtgtaaagcctggggtgcctaatgagtgagctaactcacattaattgcgttgcgctcactgcccgctttccagtcgggaaacctgtcgtgccagcggatccgcatctcaattagtcagcaaccatagtcccgcccctaactccgcccatcccgcccctaactccgcccagttccgcccattctccgccccatggctgactaattttttttatttatgcagaggccgaggccgcctcggcctctgagctattccagaagtagtgaggaggcttttttggaggcctaggcttttgcaaaaagctgtcgactgcagaggcctgcatgcaagcttggcgtaatcatggtcatagctgtttcctgtgtgaaattgttatccgctcacaattccacacaacatacgagccggaagcataaagtgtaaagcctggggtgcctaatgagtgagctaactcacattaattgcgttgcgctcactgcccgctttccagtcgggaaacctgtcgtgccagctgcattaatgaatcggccaacgcgcggggagaggcggtttgcgtattgggcgctcttccgcttcctcgctcactgactcgctgcgctcggtcgttcggctgcggcgagcggtatcagctcactcaaaggcggtaatacggttatccacagaatcaggggataacgcaggaaagaacatgtgagcaaaaggccagcaaaaggccaggaaccgtaaaaaggccgcgttgctggcgtttttccataggctccgcccccctgacgagcatcacaaaaatcgacgctcaagtcagaggtggcgaaacccgacaggactataaagataccaggcgtttccccctggaagctccctcgtgcgctctcctgttccgaccctgccgcttaccggatacctgtccgcctttctcccttcgggaagcgtggcgctttctcatagctcacgctgtaggtatctcagttcggtgtaggtcgttcgctccaagctgggctgtgtgcacgaaccccccgttcagcccgaccgctgcgccttatccggtaactatcgtcttgagtccaacccggtaagacacgacttatcgccactggcagcagccactggtaacaggattagcagagcgaggtatgtaggcggtgctacagagttcttgaagtggtggcctaactacggctacactagaagaacagtatttggtatctgcgctctgctgaagccagttaccttcggaaaaagagttggtagctcttgatccggcaaacaaaccaccgctggtagcggtggtttttttgtttgcaagcagcagattacgcgcagaaaaaaaggatctcaagaagatcctttgatcttttctacggggtctgacgctcagtggaacgaaaactcacgttaagggattttggtcatgagattatcaaaaaggatcttcacctagatccttttaaattaaaaatgaagttttaaatcaatctaaagtatatatgagtaaacttggtctgacagttaccaatgcttaatcagtgaggcacctatctcagcgatctgtctatttcgttcatccatagttgcctgactccccgtcgtgtagataactacgatacgggagggcttaccatctggccccagtgctgcaatgataccgcgagacccacgctcaccggctccagatttatcagcaataaaccagccagccggaagggccgagcgcagaagtggtcctgcaactttatccgcctccatccagtctattaattgttgccgggaagctagagtaagtagttcgccagttaatagtttgcgcaacgttgttgccattgctacaggcatcgtggtgtcacgctcgtcgtttggtatggcttcattcagctccggttcccaacgatcaaggcgagttacatgatcccccatgttgtgcaaaaaagcggttagctccttcggtcctccgatcgttgtcagaagtaagttggccgcagtgttatcactcatggttatggcagcactgcataattctcttactgtcatgccatccgtaagatgcttttctgtgactggtgagtactcaaccaagtcattctgagaatagtgtatgcggcgaccgagttgctcttgcccggcgtcaatacgggataataccgcgccacatagcagaactttaaaagtgctcatcattggaaaacgttcttcggggcgaaaactctcaaggatcttaccgctgttgagatccagttcgatgtaacccactcgtgcacccaactgatcttcagcatcttttactttcaccagcgtttctgggtgagcaaaaacaggaaggcaaaatgccgcaaaaaagggaataagggcgacacggaaatgttgaatactcatactcttcctttttcaatattattgaagcatttatcagggttattgtctcatgagcggatacatatttgaatgtatttagaaaaataaacaaataggggttccgcgcacatttccccgaaaagtgccacctgacgtctaagaaaccattattatcatgacattaacctataaaaataggcgtatcacgaggccctttcgtctcgcgcgtttcggtgatgacggtgaaaacctctgacacatgcagctcccggagacggtcacagcttgtctgtaagcggatgccgggagcagacaagcccgtcagggcgcgtcagcgggtgttggcgggtgtcggggctggcttaactatgcggcatcagagcagattgtactgagagtgcaccatatgcggtgtgaaataccgcacagatgcgtaaggagaaaataccgcatcaggcgccattcgccattcaggctgcgcaactgttgggaagggcgatcggtgcgggcctcttcgctattacgccagctggcgaaagggggatgtgctgcaaggcgattaagttgggtaacgccagggttttcccagtcacgacgttgtaaaacgacggccagtgaattc

SEQ ID NO: 18 - DNA, 11369 bp, Artificial Sequence
  Synthetic: TL20d-GbGM
ggccgcctcggccaaacagcccttgagtttaccactccctatcagtgatagagaaaagtgaaagtcgagtttaccactccctatcagtgatagagaaaagtgaaagtcgagtttaccactccctatcagtgatagagaaaagtgaaagtcgagtttaccactccctatcagtgatagagaaaagtgaaagtcgagtttaccagtccctatcagtgatagagaaaagtgaaagtcgagtttaccactccctatcagtgatagagaaaagtgaaagtcgagtttaccactccctatcagtgatagagaaaagtgaaagtcgagctcgccatgggaggcgtggcctgggcgggactggggagtggcgagccctcagatcctgcatataagcagctgctttttgcctgtactgggtctctctggttagaccagatctgagcctgggagctctctggctaactagggaacccactgcttaagcctcaataaagcttgccttgagtgcttcaagtagtgtgtgcccgtctgttgtgtgactctggtaactagagatccctcagacccttttagtcagtgtggaaaatctctagcagtggcgcccgaacagggacttgaaagcgaaagggaaaccagaggagctctctcgacgcaggactcggcttgctgaagcgcgcacggcaagaggcgaggggcggcgactggtgagtacgccaaaaattttgactagcggaggctagaaggagagagatgggtgcgagagcgtcagtattaagcgggggagaattagatcgcgatgggaaaaaattcggttaaggccagggggaaagaaaaaatataaattaaaacatatagtatgggcaagcagggagctagaacgattcgcagttaatactggcctgttagaaacatcagaaggctgtagacaaatactgggacagctacaaccatcccttcagacaggatcagaagaacttagatcattatataatacagtagcaaccctctattgtgtgcatcaaaggatagagataaaagacaccaaggaagctttagacaagatagaggaagagcaaaacaaaagtaagaaaaaagcacagcaagcagcaggatcttcagacctggaaattccctacaatccccaaagtcaaggagtagtagaatctatgaataaagaattaaagaaaattataggacaggtaagagatcaggctgaacatcttaagacagcagtacaaatggcagtattcatccacaattttaaaagaaaaggggggattggggggtacagtgcaggggaaagaatagtagacataatagcaacagacatacaaactaaagaattacaaaaacaaattacaaaaattcaaaattttcgggtttattacagggacagcagaaatccactttggaaaggaccagcaaagctcctctggaaaggtgaaggggcagtagtaatacaagataatagtgacataaaagtagtgccaagaagaaaagcaaagatcattagggattatggaaaacagatggcaggtgatgattgtgtggcaagtagacaggatgaggattagaacatggaaaagtttagtaaaacaccataaggaggagatatgagggacaattggagaagtgaattatataaatataaagtagtaaaaattgaaccattaggagtagcacccaccaaggcaaagagaagagtggtgcagagagaaaaaagagcagtgggaataggagctttgttccttgggttcttgggagcagcaggaagcactatgggcgcagcgtcaatgacgctgacggtacaggccagacaattattgtctggtatagtgcagcagcagaacaatttgctgagggctattgaggcgcaacagcatctgttgcaactcacagtctggggcatcaagcagctccaggcaagaatcctggctgtggaaagatacctaaaggatcaacagctcctggggatttggggttgctctggaaaactcatttgcaccactgctgtgccttggaatgctagttggagtaataaatctctggaacagatttggaatcacacgacctggatggagtgggacagagaaattaacaattacacaagcttaatacactccttaattgaagaatcgcaaaaccagcaagaaaagaatgaacaagaattattggaattagataaatgggcaagtttgtggaattggtttaacataacaaattggctgtggtatataaaattattcataatgatagtaggaggcttggtaggtttaagaatagtttttgctgtactttctatagtgaatagagttaggcagggatattcaccattatcgtttcagacccacctcccaaccccgaggggaccgagctcaagcttcgaacgcgtggggatcctctagagtcgagctcgcgaggatcatcaccggtgctagccggagccagaagcaccataagggacatgataagggagccagcagacctctgatctcttcctgaatgctaatcttaaacatcctgaggaagaatgggacttccatttggggtgggcctatgatagggtaataagacagtagtgaatatcaagctacaaaaagccccctttcaaattcttctcagtcctaacttttcatactaagcccagtccttccaaagcagactgtgaaagagtgatagttccgggagactagcaccggctagccgagcttggaacactttcccttcattaagaaccatccttgctactcagctgcaatcaatccagcccccaggtcttcactgaaccttttcccatctcttccaaaacatctgtttctgagaagtcctgtcctatagaggtctttcttcccaccggatttctcctacaccatttactcccacttgcagaactcccgtgtacaagtgtctttactgcttttatttgctcaacaaaatgcacatctcatataaaaataaatgaggagcatgcacacaccacaaacacaaacaggcatgcagaaatacacatacacacttccctcaatataaaccctttgtggctcatatatttaaaaagatgtaaaaaaaagagctgaagaaaatcatgtgtgatctctcagcagaatagatttattatttgtattgcttgcagaataaagcctatccttgaaagctctgaatcatgggcaagaggctcagtggtatctggaggacagggcactggccactgcagtcaccatcttctgccaggaagcctgcacctcaggggtgaattctttgccaaagtgaatggccagcacggtgaccagcacgttgcccaggagctgtgggaggaagataagaggtatgaacatgattagcaaaagggcctagcttggactcagaataatccagccttatcccaaccataaaataaaagcagaatggtagctggattgtagctgctattagcaatatgaaacctcttacatcagttacaatttatatgcagaaatatttatatgcagaaatattgctattgccttaacccagaaattatcactgttattctttagaatggtgcaaagaggcatgatacattgtatcattattgccctgaaagaaagagattagggaaagtattagaaataagataaacaaaaaagtatattaaaagaagaaagcattttttaaaattacaaatgcaaaattaccctgatttggtcaatatgtgtaccctgttacttctccccttcctatgacatgaacttaaccatagaaaagaaggggaaagaaaacatcaagggtcccatagactcaccttgaagttctcaggatccacatgcagcttgtcacagtgcagttcactcagctgggcaaaggtgcccttgagatcatccaggtgctttatggcatctcccaaggaagtcagcaccttcttgccatgtgccttgactttggggttgcccatgatggcagaggcagaggacaggttgccaaagctgtcaaagaacctctgggtccatgggtagacaaccaggagcctgtgagattgacaagaacagtttgacagtcagaaggtgccacaaatcctgagaagcaacctggacttttgccaggcacagggtccttccttccctcccttgtcctggtcaccagagcctaccttcccagggtttctcctccagcatcttccacattcaccttgtcccacaggcttgtgatagtagccttgtcctcctctgtgaaatgacccatggtgtctgtttgaggttgctagtgaacacagttgtgtcagaagcaaatgtaagcaatagatggctctgccctgacttttatgcccagccctggctcctgccctccctgctcctgggagtagattggccaaccctagggtgtggctccacagggtgaggtctaagtgatgacagccgtacctgtccttggctcttctggcactggcttaggagttggacttcaaaccctcagccctccctctaagatatatctcttggccccataccatcagtacaaattgctactaaaaacatcctcctttgcaagtgtatttacgacggtatcgatgtatgtgagcatgtgtcctctaacagcacaggccttttgccacctagctgtccaggggtgccttaaaatggcaaacaaggtttgttttcttttcctgttttcatgccttcctcttccatatccttgtttcatattaatacatgtgtatagatcctaaaaatctatacacatgtattaataaagcctgattctgccgcttctaggtatagaggccacctgcaagataaatatttgattcacaataactaatcattctatggcaattgataacaacaaatatatatatatatatatatatacgtatatgtgtatatatatatatatattcaggaaataatatattctagaatatgtcacattctgtctcaggcatccattttctttatgatgccgtttgaggtggagttttagtcaggtggtcagcttctccttttttttgccatctgccctgtaagcatcctgctggggacccagataggagtcatcactctaggctgagaacatctgggcacacaccctaagcctcagcatgactcatcatgactcagcattgctgtgcttgagccagaaggtttgcttagaaggttacacagaaccagaaggcgggggtggggcactgaccccgacaggggcctggccagaactgctcatgcttggactatgggaggtcactaatggagacacacagaaatgtaacaggaactaagggaattccggtgccctgcttaggagcttaatctttaatgaaagctaagctttcattaaaaaaagtctaaccagctgcattcgactttgactgcagcagctggttagaaggttctactggaggagggtcccagcccattgctaaattaacatcaggctctgagactggcagtatatctctaacagtggttgatgctatcttctggaacttgcctgctacattgagaccactgacccatacataggaagcccatagctctgtcctgaactgttaggccactggtccagagagtgtgcatctcctttgatcctcataataaccctatgagatagacacaattattactcttactttatagatgatgatcctgaaaacataggagtcaaggcacttgcccctagctgggggtataggggagcagtcccatgtagtagtagaatgaaaaatgctgctatgctgtgcctcccccacctttcccatgtctgccctctactcatggtctatctctcctggctcctgggagtcatggactccacccagcaccaccaacctgacctaaccacctatctgagcctgccagcctataacccatctgggccctgatagctggtggccagccctgaccccaccccaccctccctggaacctctgatagacacatctggcacaccagctcgcaaagtcaccgtgagggtcttgtgtttgctgagtcaaaattccttgaaatccaagtccttagagactcctgctcccaaatttacagtcatagacttcttcatggctgtctcctttatccacagaatgattcctttgcttcattgccccatccatctgatcctcctcatcagtgcagcacagggcccatgagcagtagctgcagagtctcacataggtctggcactgcctctgacatgtccgaccttaggcaaatgcttgactcttctgagctcggatcccttgagctcaggaggtcaaggctgcagtgagacatgatcttgccactgcactccagcctggacagcagagtgaaaccttgcctcacgaaacagaatacaaaaacaaacaaacaaaaaactgctccgcaatgcgcttccttgatgctctaccacataggtctgggtactttgtacacattatctcattgctgttcataattgttagattaattttgtaatattgatattattcctagaaagctgaggcctcaagatgataacttttattttctggacttgtaatagctttctcttgtattcaccatgttgtaactttcttagagtagtaacaatataaagttattgtgagtttttgcaaacacagcaaacacaacgacccatatagacattgatgtgaaattgtctattgtcaatttatgggaaaacaagtatgtactttttctactaagccattgaaacaggaataacagaacaagattgaaagaatacattttccgaaattacttgagtattatacaaagacaagcacgtggacctgggaggagggttattgtccatgactggtgtgtggagacaaatgcaggtttataatagatgggatggcatctagcgcaatgactttgccatcacttttagagagctcttgggggccccagtacacaagaggggacgcagggtatatgtagacatctcattctttttcttagtgtgagaataagaatagccatgacctgagtttatagacaatgagcccttttctctctcccactcagcagctatgagatggcttgccctgcctctctactaggctgactcactccaaggcccagcaatgggcagggctctgtcagggctttgatagcactatctgcagagccagggccgagaaggggtggactccagagactctccctcccattcccgagcagggtttgcttatttatgcatttaaatgatatatttattttaaaagaaataacaggagactgcccagccctggctgtgacatggaaactatgtagaatattttgggttccatttttttttccttctttcagttagaggaaaaggggctcactgcacatacactagacagaaagtcaggagctttgaatccaagcctgatcatttccatgtcatactgagaaagtccccacccttctctgagcctcagtttctctttttataagtaggagtctggagtaaatgatttccaatggctctcatttcaatacaaaatttccgtttattaaatgcatgagcttccgttactccaagactgagaaggaaattgaacctgagactcattgactggcaagatgtccccagaggctctcattcagcaataaaattctcaccttcacccaggcccactagtgtcagatttgcatgcgttaacgcggccgcatcgatgccgtagtacctttaagaccaatgacttacaaggcagctgtagatcttagccactttttaaaagaaaaggggggactggaagggctaattcactcccaaagaagacaagatagatctgctttttgcctgtactgggtctctctggttagaccagatctgagcctgggagctctctggctaactagggaacccactgcttaagcctcaataaagcttcagctgctcgagctagcagatctttttccctctgccaaaaattatggggacatcatgaagccccttgagcatctgacttctggctaataaaggaaatttattttcattgcaatagtgtgttggaattttttgtgtctctcactcggaaggacatatgggagggcaaatcatttaaaacatcagaatgagtatttggtttagagtttggcaacatatgcccatatgctggctgccatgaacaaaggttggctataaagaggtcatcagtatatgaaacagccccctgctgtccattccttattccatagaaaagccttgacttgaggttagattttttttatattttgttttgtgttatttttttctttaacatccctaaaattttccttacatgttttactagccagatttttcctcctctcctgactactcccagtcatagctgtccctcttctcttatggagatccctcgacctgcagcccaagcttggcgtaatcatggtcatagctgtttcctgtgtgaaattgttatccgctcacaattccacacaacatacgagccggaagcataaagtgtaaagcctggggtgcctaatgagtgagctaactcacattaattgcgttgcgctcactgcccgctttccagtcgggaaacctgtcgtgccagcggatccgcatctcaattagtcagcaaccatagtcccgcccctaactccgcccatcccgcccctaactccgcccagttccgcccattctccgccccatggctgactaattttttttatttatgcagaggccgaggccgcctcggcctctgagctattccagaagtagtgaggaggcttttttggaggcctaggcttttgcaaaaagctgtcgactgcagaggcctgcatgcaagcttggcgtaatcatggtcatagctgtttcctgtgtgaaattgttatccgctcacaattccacacaacatacgagccggaagcataaagtgtaaagcctggggtgcctaatgagtgagctaactcacattaattgcgttgcgctcactgcccgctttccagtcgggaaacctgtcgtgccagctgcattaatgaatcggccaacgcgcggggagaggcggtttgcgtattgggcgctcttccgcttcctcgctcactgactcgctgcgctcggtcgttcggctgcggcgagcggtatcagctcactcaaaggcggtaatacggttatccacagaatcaggggataacgcaggaaagaacatgtgagcaaaaggccagcaaaaggccaggaaccgtaaaaaggccgcgttgctggcgtttttccataggctccgcccccctgacgagcatcacaaaaatcgacgctcaagtcagaggtggcgaaacccgacaggactataaagataccaggcgtttccccctggaagctccctcgtgcgctctcctgttccgaccctgccgcttaccggatacctgtccgcctttctcccttcgggaagcgtggcgctttctcatagctcacgctgtaggtatctcagttcggtgtaggtcgttcgctccaagctgggctgtgtgcacgaaccccccgttcagcccgaccgctgcgccttatccggtaactatcgtcttgagtccaacccggtaagacacgacttatcgccactggcagcagccactggtaacaggattagcagagcgaggtatgtaggcggtgctacagagttcttgaagtggtggcctaactacggctacactagaagaacagtatttggtatctgcgctctgctgaagccagttaccttcggaaaaagagttggtagctcttgatccggcaaacaaaccaccgctggtagcggtggtttttttgtttgcaagcagcagattacgcgcagaaaaaaaggatctcaagaagatcctttgatcttttctacggggtctgacgctcagtggaacgaaaactcacgttaagggattttggtcatgagattatcaaaaaggatcttcacctagatccttttaaattaaaaatgaagttttaaatcaatctaaagtatatatgagtaaacttggtctgacagttaccaatgcttaatcagtgaggcacctatctcagcgatctgtctatttcgttcatccatagttgcctgactccccgtcgtgtagataactacgatacgggagggcttaccatctggccccagtgctgcaatgataccgcgagacccacgctcaccggctccagatttatcagcaataaaccagccagccggaagggccgagcgcagaagtggtcctgcaactttatccgcctccatccagtctattaattgttgccgggaagctagagtaagtagttcgccagttaatagtttgcgcaacgttgttgccattgctacaggcatcgtggtgtcacgctcgtcgtttggtatggcttcattcagctccggttcccaacgatcaaggcgagttacatgatcccccatgttgtgcaaaaaagcggttagctccttcggtcctccgatcgttgtcagaagtaagttggccgcagtgttatcactcatggttatggcagcactgcataattctcttactgtcatgccatccgtaagatgcttttctgtgactggtgagtactcaaccaagtcattctgagaatagtgtatgcggcgaccgagttgctcttgcccggcgtcaatacgggataataccgcgccacatagcagaactttaaaagtgctcatcattggaaaacgttcttcggggcgaaaactctcaaggatcttaccgctgttgagatccagttcgatgtaacccactcgtgcacccaactgatcttcagcatcttttactttcaccagcgtttctgggtgagcaaaaacaggaaggcaaaatgccgcaaaaaagggaataagggcgacacggaaatgttgaatactcatactcttcctttttcaatattattgaagcatttatcagggttattgtctcatgagcggatacatatttgaatgtatttagaaaaataaacaaataggggttccgcgcacatttccccgaaaagtgccacctgacgtctaagaaaccattattatcatgacattaacctataaaaataggcgtatcacgaggccctttcgtctcgcgcgtttcggtgatgacggtgaaaacctctgacacatgcagctcccggagacggtcacagcttgtctgtaagcggatgccgggagcagacaagcccgtcagggcgcgtcagcgggtgttggcgggtgtcggggctggcttaactatgcggcatcagagcagattgtactgagagtgcaccatatgcggtgtgaaataccgcacagatgcgtaaggagaaaataccgcatcaggcgccattcgccattcaggctgcgcaactgttgggaagggcgatcggtgcgggcctcttcgctattacgccagctggcgaaagggggatgtgctgcaaggcgattaagttgggtaacgccagggttttcccagtcacgacgttgtaaaacgacggccagtgaattc

SEQ ID NO: 19 - DNA, 11671 bp, Artificial Sequence
  Synthetic: TL20d-rGbGM-7SKM1/sh734
ggccgcctcggccaaacagcccttgagtttaccactccctatcagtgatagagaaaagtgaaagtcgagtttaccactccctatcagtgatagagaaaagtgaaagtcgagtttaccactccctatcagtgatagagaaaagtgaaagtcgagtttaccactccctatcagtgatagagaaaagtgaaagtcgagtttaccagtccctatcagtgatagagaaaagtgaaagtcgagtttaccactccctatcagtgatagagaaaagtgaaagtcgagtttaccactccctatcagtgatagagaaaagtgaaagtcgagctcgccatgggaggcgtggcctgggcgggactggggagtggcgagccctcagatcctgcatataagcagctgctttttgcctgtactgggtctctctggttagaccagatctgagcctgggagctctctggctaactagggaacccactgcttaagcctcaataaagcttgccttgagtgcttcaagtagtgtgtgcccgtctgttgtgtgactctggtaactagagatccctcagacccttttagtcagtgtggaaaatctctagcagtggcgcccgaacagggacttgaaagcgaaagggaaaccagaggagctctctcgacgcaggactcggcttgctgaagcgcgcacggcaagaggcgaggggcggcgactggtgagtacgccaaaaattttgactagcggaggctagaaggagagagatgggtgcgagagcgtcagtattaagcgggggagaattagatcgcgatgggaaaaaattcggttaaggccagggggaaagaaaaaatataaattaaaacatatagtatgggcaagcagggagctagaacgattcgcagttaatactggcctgttagaaacatcagaaggctgtagacaaatactgggacagctacaaccatcccttcagacaggatcagaagaacttagatcattatataatacagtagcaaccctctattgtgtgcatcaaaggatagagataaaagacaccaaggaagctttagacaagatagaggaagagcaaaacaaaagtaagaaaaaagcacagcaagcagcaggatcttcagacctggaaattccctacaatccccaaagtcaaggagtagtagaatctatgaataaagaattaaagaaaattataggacaggtaagagatcaggctgaacatcttaagacagcagtacaaatggcagtattcatccacaattttaaaagaaaaggggggattggggggtacagtgcaggggaaagaatagtagacataatagcaacagacatacaaactaaagaattacaaaaacaaattacaaaaattcaaaattttcgggtttattacagggacagcagaaatccactttggaaaggaccagcaaagctcctctggaaaggtgaaggggcagtagtaatacaagataatagtgacataaaagtagtgccaagaagaaaagcaaagatcattagggattatggaaaacagatggcaggtgatgattgtgtggcaagtagacaggatgaggattagaacatggaaaagtttagtaaaacaccataaggaggagatatgagggacaattggagaagtgaattatataaatataaagtagtaaaaattgaaccattaggagtagcacccaccaaggcaaagagaagagtggtgcagagagaaaaaagagcagtgggaataggagctttgttccttgggttcttgggagcagcaggaagcactatgggcgcagcgtcaatgacgctgacggtacaggccagacaattattgtctggtatagtgcagcagcagaacaatttgctgagggctattgaggcgcaacagcatctgttgcaactcacagtctggggcatcaagcagctccaggcaagaatcctggctgtggaaagatacctaaaggatcaacagctcctggggatttggggttgctctggaaaactcatttgcaccactgctgtgccttggaatgctagttggagtaataaatctctggaacagatttggaatcacacgacctggatggagtgggacagagaaattaacaattacacaagcttaatacactccttaattgaagaatcgcaaaaccagcaagaaaagaatgaacaagaattattggaattagataaatgggcaagtttgtggaattggtttaacataacaaattggctgtggtatataaaattattcataatgatagtaggaggcttggtaggtttaagaatagtttttgctgtactttctatagtgaatagagttaggcagggatattcaccattatcgtttcagacccacctcccaaccccgaggggaccgagctcaagcttcgaacgcgtggggatcctctagagtcgagctcgcgaggatcatcaccggtgctagccggagccagaagcaccataagggacatgataagggagccagcagacctctgatctcttcctgaatgctaatcttaaacatcctgaggaagaatgggacttccatttggggtgggcctatgatagggtaataagacagtagtgaatatcaagctacaaaaagccccctttcaaattcttctcagtcctaacttttcatactaagcccagtccttccaaagcagactgtgaaagagtgatagttccgggagactagcaccggctagccgagcttggaacactttcccttcattaagaaccatccttgctactcagctgcaatcaatccagcccccaggtcttcactgaaccttttcccatctcttccaaaacatctgtttctgagaagtcctgtcctatagaggtctttcttcccaccggatttctcctacaccatttactcccacttgcagaactcccgtgtacaagtgtctttactgcttttatttgctcaacaaaatgcacatctcatataaaaataaatgaggagcatgcacacaccacaaacacaaacaggcatgcagaaatacacatacacacttccctcaatataaaccctttgtggctcatatatttaaaaagatgtaaaaaaaagagctgaagaaaatcatgtgtgatctctcagcagaatagatttattatttgtattgcttgcagaataaagcctatccttgaaagctctgaatcatgggcaagaggctcagtggtatctggaggacagggcactggccactgcagtcaccatcttctgccaggaagcctgcacctcaggggtgaattctttgccaaagtgaatggccagcacggtgaccagcacgttgcccaggagctgtgggaggaagataagaggtatgaacatgattagcaaaagggcctagcttggactcagaataatccagccttatcccaaccataaaataaaagcagaatggtagctggattgtagctgctattagcaatatgaaacctcttacatcagttacaatttatatgcagaaatatttatatgcagaaatattgctattgccttaacccagaaattatcactgttattctttagaatggtgcaaagaggcatgatacattgtatcattattgccctgaaagaaagagattagggaaagtattagaaataagataaacaaaaaagtatattaaaagaagaaagcattttttaaaattacaaatgcaaaattaccctgatttggtcaatatgtgtaccctgttacttctccccttcctatgacatgaacttaaccatagaaaagaaggggaaagaaaacatcaagggtcccatagactcaccttgaagttctcaggatccacatgcagcttgtcacagtgcagttcactcagctgggcaaaggtgcccttgagatcatccaggtgctttatggcatctcccaaggaagtcagcaccttcttgccatgtgccttgactttggggttgcccatgatggcagaggcagaggacaggttgccaaagctgtcaaagaacctctgggtccatgggtagacaaccaggagcctgtgagattgacaagaacagtttgacagtcagaaggtgccacaaatcctgagaagcaacctggacttttgccaggcacagggtccttccttccctcccttgtcctggtcaccagagcctaccttcccagggtttctcctccagcatcttccacattcaccttgtcccacaggcttgtgatagtagccttgtcctcctctgtgaaatgacccatggtgtctgtttgaggttgctagtgaacacagttgtgtcagaagcaaatgtaagcaatagatggctctgccctgacttttatgcccagccctggctcctgccctccctgctcctgggagtagattggccaaccctagggtgtggctccacagggtgaggtctaagtgatgacagccgtacctgtccttggctcttctggcactggcttaggagttggacttcaaaccctcagccctccctctaagatatatctcttggccccataccatcagtacaaattgctactaaaaacatcctcctttgcaagtgtatttacgacggtatcgatgtatgtgagcatgtgtcctctaacagcacaggccttttgccacctagctgtccaggggtgccttaaaatggcaaacaaggtttgttttcttttcctgttttcatgccttcctcttccatatccttgtttcatattaatacatgtgtatagatcctaaaaatctatacacatgtattaataaagcctgattctgccgcttctaggtatagaggccacctgcaagataaatatttgattcacaataactaatcattctatggcaattgataacaacaaatatatatatatatatatatatacgtatatgtgtatatatatatatatattcaggaaataatatattctagaatatgtcacattctgtctcaggcatccattttctttatgatgccgtttgaggtggagttttagtcaggtggtcagcttctccttttttttgccatctgccctgtaagcatcctgctggggacccagataggagtcatcactctaggctgagaacatctgggcacacaccctaagcctcagcatgactcatcatgactcagcattgctgtgcttgagccagaaggtttgcttagaaggttacacagaaccagaaggcgggggtggggcactgaccccgacaggggcctggccagaactgctcatgcttggactatgggaggtcactaatggagacacacagaaatgtaacaggaactaagggaattccggtgccctgcttaggagcttaatctttaatgaaagctaagctttcattaaaaaaagtctaaccagctgcattcgactttgactgcagcagctggttagaaggttctactggaggagggtcccagcccattgctaaattaacatcaggctctgagactggcagtatatctctaacagtggttgatgctatcttctggaacttgcctgctacattgagaccactgacccatacataggaagcccatagctctgtcctgaactgttaggccactggtccagagagtgtgcatctcctttgatcctcataataaccctatgagatagacacaattattactcttactttatagatgatgatcctgaaaacataggagtcaaggcacttgcccctagctgggggtataggggagcagtcccatgtagtagtagaatgaaaaatgctgctatgctgtgcctcccccacctttcccatgtctgccctctactcatggtctatctctcctggctcctgggagtcatggactccacccagcaccaccaacctgacctaaccacctatctgagcctgccagcctataacccatctgggccctgatagctggtggccagccctgaccccaccccaccctccctggaacctctgatagacacatctggcacaccagctcgcaaagtcaccgtgagggtcttgtgtttgctgagtcaaaattccttgaaatccaagtccttagagactcctgctcccaaatttacagtcatagacttcttcatggctgtctcctttatccacagaatgattcctttgcttcattgccccatccatctgatcctcctcatcagtgcagcacagggcccatgagcagtagctgcagagtctcacataggtctggcactgcctctgacatgtccgaccttaggcaaatgcttgactcttctgagctcggatcccttgagctcaggaggtcaaggctgcagtgagacatgatcttgccactgcactccagcctggacagcagagtgaaaccttgcctcacgaaacagaatacaaaaacaaacaaacaaaaaactgctccgcaatgcgcttccttgatgctctaccacataggtctgggtactttgtacacattatctcattgctgttcataattgttagattaattttgtaatattgatattattcctagaaagctgaggcctcaagatgataacttttattttctggacttgtaatagctttctcttgtattcaccatgttgtaactttcttagagtagtaacaatataaagttattgtgagtttttgcaaacacagcaaacacaacgacccatatagacattgatgtgaaattgtctattgtcaatttatgggaaaacaagtatgtactttttctactaagccattgaaacaggaataacagaacaagattgaaagaatacattttccgaaattacttgagtattatacaaagacaagcacgtggacctgggaggagggttattgtccatgactggtgtgtggagacaaatgcaggtttataatagatgggatggcatctagcgcaatgactttgccatcacttttagagagctcttgggggccccagtacacaagaggggacgcagggtatatgtagacatctcattctttttcttagtgtgagaataagaatagccatgacctgagtttatagacaatgagcccttttctctctcccactcagcagctatgagatggcttgccctgcctctctactaggctgactcactccaaggcccagcaatgggcagggctctgtcagggctttgatagcactatctgcagagccagggccgagaaggggtggactccagagactctccctcccattcccgagcagggtttgcttatttatgcatttaaatgatatatttattttaaaagaaataacaggagactgcccagccctggctgtgacatggaaactatgtagaatattttgggttccatttttttttccttctttcagttagaggaaaaggggctcactgcacatacactagacagaaagtcaggagctttgaatccaagcctgatcatttccatgtcatactgagaaagtccccacccttctctgagcctcagtttctctttttataagtaggagtctggagtaaatgatttccaatggctctcatttcaatacaaaatttccgtttattaaatgcatgagcttccgttactccaagactgagaaggaaattgaacctgagactcattgactggcaagatgtccccagaggctctcattcagcaataaaattctcaccttcacccaggcccactagtgtcagatttgcatgcgttcgcgttcgacgtgcagtcgggctactgccccacccatagtaccggcattctggatagtgtcaaaacagccggaaatcaagtccgtttatctcaaactttagcattttgggaataaatgatatttgctatgctggttaaattagattttagttaaatttcctgctgaagctctagtacgataagtaacttgacctaagtgtaaagttgagatttccttcaggtttatatagcttgtgcgccgcctgggtacctcaggatatgcccttgactatttgtccgacatagtcaagggcatatccttttttgcggccgcatcgatgccgtagtacctttaagaccaatgacttacaaggcagctgtagatcttagccactttttaaaagaaaaggggggactggaagggctaattcactcccaaagaagacaagatagatctgctttttgcctgtactgggtctctctggttagaccagatctgagcctgggagctctctggctaactagggaacccactgcttaagcctcaataaagcttcagctgctcgagctagcagatctttttccctctgccaaaaattatggggacatcatgaagccccttgagcatctgacttctggctaataaaggaaatttattttcattgcaatagtgtgttggaattttttgtgtctctcactcggaaggacatatgggagggcaaatcatttaaaacatcagaatgagtatttggtttagagtttggcaacatatgcccatatgctggctgccatgaacaaaggttggctataaagaggtcatcagtatatgaaacagccccctgctgtccattccttattccatagaaaagccttgacttgaggttagattttttttatattttgttttgtgttatttttttctttaacatccctaaaattttccttacatgttttactagccagatttttcctcctctcctgactactcccagtcatagctgtccctcttctcttatggagatccctcgacctgcagcccaagcttggcgtaatcatggtcatagctgtttcctgtgtgaaattgttatccgctcacaattccacacaacatacgagccggaagcataaagtgtaaagcctggggtgcctaatgagtgagctaactcacattaattgcgttgcgctcactgcccgctttccagtcgggaaacctgtcgtgccagcggatccgcatctcaattagtcagcaaccatagtcccgcccctaactccgcccatcccgcccctaactccgcccagttccgcccattctccgccccatggctgactaattttttttatttatgcagaggccgaggccgcctcggcctctgagctattccagaagtagtgaggaggcttttttggaggcctaggcttttgcaaaaagctgtcgactgcagaggcctgcatgcaagcttggcgtaatcatggtcatagctgtttcctgtgtgaaattgttatccgctcacaattccacacaacatacgagccggaagcataaagtgtaaagcctggggtgcctaatgagtgagctaactcacattaattgcgttgcgctcactgcccgctttccagtcgggaaacctgtcgtgccagctgcattaatgaatcggccaacgcgcggggagaggcggtttgcgtattgggcgctcttccgcttcctcgctcactgactcgctgcgctcggtcgttcggctgcggcgagcggtatcagctcactcaaaggcggtaatacggttatccacagaatcaggggataacgcaggaaagaacatgtgagcaaaaggccagcaaaaggccaggaaccgtaaaaaggccgcgttgctggcgtttttccataggctccgcccccctgacgagcatcacaaaaatcgacgctcaagtcagaggtggcgaaacccgacaggactataaagataccaggcgtttccccctggaagctccctcgtgcgctctcctgttccgaccctgccgcttaccggatacctgtccgcctttctcccttcgggaagcgtggcgctttctcatagctcacgctgtaggtatctcagttcggtgtaggtcgttcgctccaagctgggctgtgtgcacgaaccccccgttcagcccgaccgctgcgccttatccggtaactatcgtcttgagtccaacccggtaagacacgacttatcgccactggcagcagccactggtaacaggattagcagagcgaggtatgtaggcggtgctacagagttcttgaagtggtggcctaactacggctacactagaagaacagtatttggtatctgcgctctgctgaagccagttaccttcggaaaaagagttggtagctcttgatccggcaaacaaaccaccgctggtagcggtggtttttttgtttgcaagcagcagattacgcgcagaaaaaaaggatctcaagaagatcctttgatcttttctacggggtctgacgctcagtggaacgaaaactcacgttaagggattttggtcatgagattatcaaaaaggatcttcacctagatccttttaaattaaaaatgaagttttaaatcaatctaaagtatatatgagtaaacttggtctgacagttaccaatgcttaatcagtgaggcacctatctcagcgatctgtctatttcgttcatccatagttgcctgactccccgtcgtgtagataactacgatacgggagggcttaccatctggccccagtgctgcaatgataccgcgagacccacgctcaccggctccagatttatcagcaataaaccagccagccggaagggccgagcgcagaagtggtcctgcaactttatccgcctccatccagtctattaattgttgccgggaagctagagtaagtagttcgccagttaatagtttgcgcaacgttgttgccattgctacaggcatcgtggtgtcacgctcgtcgtttggtatggcttcattcagctccggttcccaacgatcaaggcgagttacatgatcccccatgttgtgcaaaaaagcggttagctccttcggtcctccgatcgttgtcagaagtaagttggccgcagtgttatcactcatggttatggcagcactgcataattctcttactgtcatgccatccgtaagatgcttttctgtgactggtgagtactcaaccaagtcattctgagaatagtgtatgcggcgaccgagttgctcttgcccggcgtcaatacgggataataccgcgccacatagcagaactttaaaagtgctcatcattggaaaacgttcttcggggcgaaaactctcaaggatcttaccgctgttgagatccagttcgatgtaacccactcgtgcacccaactgatcttcagcatcttttactttcaccagcgtttctgggtgagcaaaaacaggaaggcaaaatgccgcaaaaaagggaataagggcgacacggaaatgttgaatactcatactcttcctttttcaatattattgaagcatttatcagggttattgtctcatgagcggatacatatttgaatgtatttagaaaaataaacaaataggggttccgcgcacatttccccgaaaagtgccacctgacgtctaagaaaccattattatcatgacattaacctataaaaataggcgtatcacgaggccctttcgtctcgcgcgtttcggtgatgacggtgaaaacctctgacacatgcagctcccggagacggtcacagcttgtctgtaagcggatgccgggagcagacaagcccgtcagggcgcgtcagcgggtgttggcgggtgtcggggctggcttaactatgcggcatcagagcagattgtactgagagtgcaccatatgcggtgtgaaataccgcacagatgcgtaaggagaaaataccgcatcaggcgccattcgccattcaggctgcgcaactgttgggaagggcgatcggtgcgggcctcttcgctattacgccagctggcgaaagggggatgtgctgcaaggcgattaagttgggtaacgccagggttttcccagtcacgacgttgtaaaacgacggccagtgaattc

SEQ ID NO: 20 - DNA, 11674 bp, Artificial Sequence
  Synthetic: TL20d-rGbGM-7SK/sh734
ggccgcctcggccaaacagcccttgagtttaccactccctatcagtgatagagaaaagtgaaagtcgagtttaccactccctatcagtgatagagaaaagtgaaagtcgagtttaccactccctatcagtgatagagaaaagtgaaagtcgagtttaccactccctatcagtgatagagaaaagtgaaagtcgagtttaccagtccctatcagtgatagagaaaagtgaaagtcgagtttaccactccctatcagtgatagagaaaagtgaaagtcgagtttaccactccctatcagtgatagagaaaagtgaaagtcgagctcgccatgggaggcgtggcctgggcgggactggggagtggcgagccctcagatcctgcatataagcagctgctttttgcctgtactgggtctctctggttagaccagatctgagcctgggagctctctggctaactagggaacccactgcttaagcctcaataaagcttgccttgagtgcttcaagtagtgtgtgcccgtctgttgtgtgactctggtaactagagatccctcagacccttttagtcagtgtggaaaatctctagcagtggcgcccgaacagggacttgaaagcgaaagggaaaccagaggagctctctcgacgcaggactcggcttgctgaagcgcgcacggcaagaggcgaggggcggcgactggtgagtacgccaaaaattttgactagcggaggctagaaggagagagatgggtgcgagagcgtcagtattaagcgggggagaattagatcgcgatgggaaaaaattcggttaaggccagggggaaagaaaaaatataaattaaaacatatagtatgggcaagcagggagctagaacgattcgcagttaatactggcctgttagaaacatcagaaggctgtagacaaatactgggacagctacaaccatcccttcagacaggatcagaagaacttagatcattatataatacagtagcaaccctctattgtgtgcatcaaaggatagagataaaagacaccaaggaagctttagacaagatagaggaagagcaaaacaaaagtaagaaaaaagcacagcaagcagcaggatcttcagacctggaaattccctacaatccccaaagtcaaggagtagtagaatctatgaataaagaattaaagaaaattataggacaggtaagagatcaggctgaacatcttaagacagcagtacaaatggcagtattcatccacaattttaaaagaaaaggggggattggggggtacagtgcaggggaaagaatagtagacataatagcaacagacatacaaactaaagaattacaaaaacaaattacaaaaattcaaaattttcgggtttattacagggacagcagaaatccactttggaaaggaccagcaaagctcctctggaaaggtgaaggggcagtagtaatacaagataatagtgacataaaagtagtgccaagaagaaaagcaaagatcattagggattatggaaaacagatggcaggtgatgattgtgtggcaagtagacaggatgaggattagaacatggaaaagtttagtaaaacaccataaggaggagatatgagggacaattggagaagtgaattatataaatataaagtagtaaaaattgaaccattaggagtagcacccaccaaggcaaagagaagagtggtgcagagagaaaaaagagcagtgggaataggagctttgttccttgggttcttgggagcagcaggaagcactatgggcgcagcgtcaatgacgctgacggtacaggccagacaattattgtctggtatagtgcagcagcagaacaatttgctgagggctattgaggcgcaacagcatctgttgcaactcacagtctggggcatcaagcagctccaggcaagaatcctggctgtggaaagatacctaaaggatcaacagctcctggggatttggggttgctctggaaaactcatttgcaccactgctgtgccttggaatgctagttggagtaataaatctctggaacagatttggaatcacacgacctggatggagtgggacagagaaattaacaattacacaagcttaatacactccttaattgaagaatcgcaaaaccagcaagaaaagaatgaacaagaattattggaattagataaatgggcaagtttgtggaattggtttaacataacaaattggctgtggtatataaaattattcataatgatagtaggaggcttggtaggtttaagaatagtttttgctgtactttctatagtgaatagagttaggcagggatattcaccattatcgtttcagacccacctcccaaccccgaggggaccgagctcaagcttcgaacgcgtggggatcctctagagtcgagctcgcgaggatcatcaccggtgctagccggagccagaagcaccataagggacatgataagggagccagcagacctctgatctcttcctgaatgctaatcttaaacatcctgaggaagaatgggacttccatttggggtgggcctatgatagggtaataagacagtagtgaatatcaagctacaaaaagccccctttcaaattcttctcagtcctaacttttcatactaagcccagtccttccaaagcagactgtgaaagagtgatagttccgggagactagcaccggctagccgagcttggaacactttcccttcattaagaaccatccttgctactcagctgcaatcaatccagcccccaggtcttcactgaaccttttcccatctcttccaaaacatctgtttctgagaagtcctgtcctatagaggtctttcttcccaccggatttctcctacaccatttactcccacttgcagaactcccgtgtacaagtgtctttactgcttttatttgctcaacaaaatgcacatctcatataaaaataaatgaggagcatgcacacaccacaaacacaaacaggcatgcagaaatacacatacacacttccctcaatataaaccctttgtggctcatatatttaaaaagatgtaaaaaaaagagctgaagaaaatcatgtgtgatctctcagcagaatagatttattatttgtattgcttgcagaataaagcctatccttgaaagctctgaatcatgggcaagaggctcagtggtatctggaggacagggcactggccactgcagtcaccatcttctgccaggaagcctgcacctcaggggtgaattctttgccaaagtgaatggccagcacggtgaccagcacgttgcccaggagctgtgggaggaagataagaggtatgaacatgattagcaaaagggcctagcttggactcagaataatccagccttatcccaaccataaaataaaagcagaatggtagctggattgtagctgctattagcaatatgaaacctcttacatcagttacaatttatatgcagaaatatttatatgcagaaatattgctattgccttaacccagaaattatcactgttattctttagaatggtgcaaagaggcatgatacattgtatcattattgccctgaaagaaagagattagggaaagtattagaaataagataaacaaaaaagtatattaaaagaagaaagcattttttaaaattacaaatgcaaaattaccctgatttggtcaatatgtgtaccctgttacttctccccttcctatgacatgaacttaaccatagaaaagaaggggaaagaaaacatcaagggtcccatagactcaccttgaagttctcaggatccacatgcagcttgtcacagtgcagttcactcagctgggcaaaggtgcccttgagatcatccaggtgctttatggcatctcccaaggaagtcagcaccttcttgccatgtgccttgactttggggttgcccatgatggcagaggcagaggacaggttgccaaagctgtcaaagaacctctgggtccatgggtagacaaccaggagcctgtgagattgacaagaacagtttgacagtcagaaggtgccacaaatcctgagaagcaacctggacttttgccaggcacagggtccttccttccctcccttgtcctggtcaccagagcctaccttcccagggtttctcctccagcatcttccacattcaccttgtcccacaggcttgtgatagtagccttgtcctcctctgtgaaatgacccatggtgtctgtttgaggttgctagtgaacacagttgtgtcagaagcaaatgtaagcaatagatggctctgccctgacttttatgcccagccctggctcctgccctccctgctcctgggagtagattggccaaccctagggtgtggctccacagggtgaggtctaagtgatgacagccgtacctgtccttggctcttctggcactggcttaggagttggacttcaaaccctcagccctccctctaagatatatctcttggccccataccatcagtacaaattgctactaaaaacatcctcctttgcaagtgtatttacgacggtatcgatgtatgtgagcatgtgtcctctaacagcacaggccttttgccacctagctgtccaggggtgccttaaaatggcaaacaaggtttgttttcttttcctgttttcatgccttcctcttccatatccttgtttcatattaatacatgtgtatagatcctaaaaatctatacacatgtattaataaagcctgattctgccgcttctaggtatagaggccacctgcaagataaatatttgattcacaataactaatcattctatggcaattgataacaacaaatatatatatatatatatatatacgtatatgtgtatatatatatatatattcaggaaataatatattctagaatatgtcacattctgtctcaggcatccattttctttatgatgccgtttgaggtggagttttagtcaggtggtcagcttctccttttttttgccatctgccctgtaagcatcctgctggggacccagataggagtcatcactctaggctgagaacatctgggcacacaccctaagcctcagcatgactcatcatgactcagcattgctgtgcttgagccagaaggtttgcttagaaggttacacagaaccagaaggcgggggtggggcactgaccccgacaggggcctggccagaactgctcatgcttggactatgggaggtcactaatggagacacacagaaatgtaacaggaactaagggaattccggtgccctgcttaggagcttaatctttaatgaaagctaagctttcattaaaaaaagtctaaccagctgcattcgactttgactgcagcagctggttagaaggttctactggaggagggtcccagcccattgctaaattaacatcaggctctgagactggcagtatatctctaacagtggttgatgctatcttctggaacttgcctgctacattgagaccactgacccatacataggaagcccatagctctgtcctgaactgttaggccactggtccagagagtgtgcatctcctttgatcctcataataaccctatgagatagacacaattattactcttactttatagatgatgatcctgaaaacataggagtcaaggcacttgcccctagctgggggtataggggagcagtcccatgtagtagtagaatgaaaaatgctgctatgctgtgcctcccccacctttcccatgtctgccctctactcatggtctatctctcctggctcctgggagtcatggactccacccagcaccaccaacctgacctaaccacctatctgagcctgccagcctataacccatctgggccctgatagctggtggccagccctgaccccaccccaccctccctggaacctctgatagacacatctggcacaccagctcgcaaagtcaccgtgagggtcttgtgtttgctgagtcaaaattccttgaaatccaagtccttagagactcctgctcccaaatttacagtcatagacttcttcatggctgtctcctttatccacagaatgattcctttgcttcattgccccatccatctgatcctcctcatcagtgcagcacagggcccatgagcagtagctgcagagtctcacataggtctggcactgcctctgacatgtccgaccttaggcaaatgcttgactcttctgagctcggatcccttgagctcaggaggtcaaggctgcagtgagacatgatcttgccactgcactccagcctggacagcagagtgaaaccttgcctcacgaaacagaatacaaaaacaaacaaacaaaaaactgctccgcaatgcgcttccttgatgctctaccacataggtctgggtactttgtacacattatctcattgctgttcataattgttagattaattttgtaatattgatattattcctagaaagctgaggcctcaagatgataacttttattttctggacttgtaatagctttctcttgtattcaccatgttgtaactttcttagagtagtaacaatataaagttattgtgagtttttgcaaacacagcaaacacaacgacccatatagacattgatgtgaaattgtctattgtcaatttatgggaaaacaagtatgtactttttctactaagccattgaaacaggaataacagaacaagattgaaagaatacattttccgaaattacttgagtattatacaaagacaagcacgtggacctgggaggagggttattgtccatgactggtgtgtggagacaaatgcaggtttataatagatgggatggcatctagcgcaatgactttgccatcacttttagagagctcttgggggccccagtacacaagaggggacgcagggtatatgtagacatctcattctttttcttagtgtgagaataagaatagccatgacctgagtttatagacaatgagcccttttctctctcccactcagcagctatgagatggcttgccctgcctctctactaggctgactcactccaaggcccagcaatgggcagggctctgtcagggctttgatagcactatctgcagagccagggccgagaaggggtggactccagagactctccctcccattcccgagcagggtttgcttatttatgcatttaaatgatatatttattttaaaagaaataacaggagactgcccagccctggctgtgacatggaaactatgtagaatattttgggttccatttttttttccttctttcagttagaggaaaaggggctcactgcacatacactagacagaaagtcaggagctttgaatccaagcctgatcatttccatgtcatactgagaaagtccccacccttctctgagcctcagtttctctttttataagtaggagtctggagtaaatgatttccaatggctctcatttcaatacaaaatttccgtttattaaatgcatgagcttccgttactccaagactgagaaggaaattgaacctgagactcattgactggcaagatgtccccagaggctctcattcagcaataaaattctcaccttcacccaggcccactagtgtcagatttgcatgcgttcgcgtatcgacgtgcagtatttagcatgccccacccatctgcaaggcattctggatagtgtcaaaacagccggaaatcaagtccgtttatctcaaactttagcattttgggaataaatgatatttgctatgctggttaaattagattttagttaaatttcctgctgaagctctagtacgataagtaacttgacctaagtgtaaagttgagatttccttcaggtttatatagcttgtgcgccgcctgggtacctcaggatatgcccttgactatttgtccgacatagtcaagggcatatccttttttgtgcggccgcatcgatgccgtagtacctttaagaccaatgacttacaaggcagctgtagatcttagccactttttaaaagaaaaggggggactggaagggctaattcactcccaaagaagacaagatagatctgctttttgcctgtactgggtctctctggttagaccagatctgagcctgggagctctctggctaactagggaacccactgcttaagcctcaataaagcttcagctgctcgagctagcagatctttttccctctgccaaaaattatggggacatcatgaagccccttgagcatctgacttctggctaataaaggaaatttattttcattgcaatagtgtgttggaattttttgtgtctctcactcggaaggacatatgggagggcaaatcatttaaaacatcagaatgagtatttggtttagagtttggcaacatatgcccatatgctggctgccatgaacaaaggttggctataaagaggtcatcagtatatgaaacagccccctgctgtccattccttattccatagaaaagccttgacttgaggttagattttttttatattttgttttgtgttatttttttctttaacatccctaaaattttccttacatgttttactagccagatttttcctcctctcctgactactcccagtcatagctgtccctcttctcttatggagatccctcgacctgcagcccaagcttggcgtaatcatggtcatagctgtttcctgtgtgaaattgttatccgctcacaattccacacaacatacgagccggaagcataaagtgtaaagcctggggtgcctaatgagtgagctaactcacattaattgcgttgcgctcactgcccgctttccagtcgggaaacctgtcgtgccagcggatccgcatctcaattagtcagcaaccatagtcccgcccctaactccgcccatcccgcccctaactccgcccagttccgcccattctccgccccatggctgactaattttttttatttatgcagaggccgaggccgcctcggcctctgagctattccagaagtagtgaggaggcttttttggaggcctaggcttttgcaaaaagctgtcgactgcagaggcctgcatgcaagcttggcgtaatcatggtcatagctgtttcctgtgtgaaattgttatccgctcacaattccacacaacatacgagccggaagcataaagtgtaaagcctggggtgcctaatgagtgagctaactcacattaattgcgttgcgctcactgcccgctttccagtcgggaaacctgtcgtgccagctgcattaatgaatcggccaacgcgcggggagaggcggtttgcgtattgggcgctcttccgcttcctcgctcactgactcgctgcgctcggtcgttcggctgcggcgagcggtatcagctcactcaaaggcggtaatacggttatccacagaatcaggggataacgcaggaaagaacatgtgagcaaaaggccagcaaaaggccaggaaccgtaaaaaggccgcgttgctggcgtttttccataggctccgcccccctgacgagcatcacaaaaatcgacgctcaagtcagaggtggcgaaacccgacaggactataaagataccaggcgtttccccctggaagctccctcgtgcgctctcctgttccgaccctgccgcttaccggatacctgtccgcctttctcccttcgggaagcgtggcgctttctcatagctcacgctgtaggtatctcagttcggtgtaggtcgttcgctccaagctgggctgtgtgcacgaaccccccgttcagcccgaccgctgcgccttatccggtaactatcgtcttgagtccaacccggtaagacacgacttatcgccactggcagcagccactggtaacaggattagcagagcgaggtatgtaggcggtgctacagagttcttgaagtggtggcctaactacggctacactagaagaacagtatttggtatctgcgctctgctgaagccagttaccttcggaaaaagagttggtagctcttgatccggcaaacaaaccaccgctggtagcggtggtttttttgtttgcaagcagcagattacgcgcagaaaaaaaggatctcaagaagatcctttgatcttttctacggggtctgacgctcagtggaacgaaaactcacgttaagggattttggtcatgagattatcaaaaaggatcttcacctagatccttttaaattaaaaatgaagttttaaatcaatctaaagtatatatgagtaaacttggtctgacagttaccaatgcttaatcagtgaggcacctatctcagcgatctgtctatttcgttcatccatagttgcctgactccccgtcgtgtagataactacgatacgggagggcttaccatctggccccagtgctgcaatgataccgcgagacccacgctcaccggctccagatttatcagcaataaaccagccagccggaagggccgagcgcagaagtggtcctgcaactttatccgcctccatccagtctattaattgttgccgggaagctagagtaagtagttcgccagttaatagtttgcgcaacgttgttgccattgctacaggcatcgtggtgtcacgctcgtcgtttggtatggcttcattcagctccggttcccaacgatcaaggcgagttacatgatcccccatgttgtgcaaaaaagcggttagctccttcggtcctccgatcgttgtcagaagtaagttggccgcagtgttatcactcatggttatggcagcactgcataattctcttactgtcatgccatccgtaagatgcttttctgtgactggtgagtactcaaccaagtcattctgagaatagtgtatgcggcgaccgagttgctcttgcccggcgtcaatacgggataataccgcgccacatagcagaactttaaaagtgctcatcattggaaaacgttcttcggggcgaaaactctcaaggatcttaccgctgttgagatccagttcgatgtaacccactcgtgcacccaactgatcttcagcatcttttactttcaccagcgtttctgggtgagcaaaaacaggaaggcaaaatgccgcaaaaaagggaataagggcgacacggaaatgttgaatactcatactcttcctttttcaatattattgaagcatttatcagggttattgtctcatgagcggatacatatttgaatgtatttagaaaaataaacaaataggggttccgcgcacatttccccgaaaagtgccacctgacgtctaagaaaccattattatcatgacattaacctataaaaataggcgtatcacgaggccctttcgtctcgcgcgtttcggtgatgacggtgaaaacctctgacacatgcagctcccggagacggtcacagcttgtctgtaagcggatgccgggagcagacaagcccgtcagggcgcgtcagcgggtgttggcgggtgtcggggctggcttaactatgcggcatcagagcagattgtactgagagtgcaccatatgcggtgtgaaataccgcacagatgcgtaaggagaaaataccgcatcaggcgccattcgccattcaggctgcgcaactgttgggaagggcgatcggtgcgggcctcttcgctattacgccagctggcgaaagggggatgtgctgcaaggcgattaagttgggtaacgccagggttttcccagtcacgacgttgtaaaacgacggccagtgaattc

SEQ ID NO: 21 - DNA, 11671 bp, Artificial Sequence
  Synthetic: TL20d-rGbGM-r7SKM1/sh734
ggccgcctcggccaaacagcccttgagtttaccactccctatcagtgatagagaaaagtgaaagtcgagtttaccactccctatcagtgatagagaaaagtgaaagtcgagtttaccactccctatcagtgatagagaaaagtgaaagtcgagtttaccactccctatcagtgatagagaaaagtgaaagtcgagtttaccagtccctatcagtgatagagaaaagtgaaagtcgagtttaccactccctatcagtgatagagaaaagtgaaagtcgagtttaccactccctatcagtgatagagaaaagtgaaagtcgagctcgccatgggaggcgtggcctgggcgggactggggagtggcgagccctcagatcctgcatataagcagctgctttttgcctgtactgggtctctctggttagaccagatctgagcctgggagctctctggctaactagggaacccactgcttaagcctcaataaagcttgccttgagtgcttcaagtagtgtgtgcccgtctgttgtgtgactctggtaactagagatccctcagacccttttagtcagtgtggaaaatctctagcagtggcgcccgaacagggacttgaaagcgaaagggaaaccagaggagctctctcgacgcaggactcggcttgctgaagcgcgcacggcaagaggcgaggggcggcgactggtgagtacgccaaaaattttgactagcggaggctagaaggagagagatgggtgcgagagcgtcagtattaagcgggggagaattagatcgcgatgggaaaaaattcggttaaggccagggggaaagaaaaaatataaattaaaacatatagtatgggcaagcagggagctagaacgattcgcagttaatactggcctgttagaaacatcagaaggctgtagacaaatactgggacagctacaaccatcccttcagacaggatcagaagaacttagatcattatataatacagtagcaaccctctattgtgtgcatcaaaggatagagataaaagacaccaaggaagctttagacaagatagaggaagagcaaaacaaaagtaagaaaaaagcacagcaagcagcaggatcttcagacctggaaattccctacaatccccaaagtcaaggagtagtagaatctatgaataaagaattaaagaaaattataggacaggtaagagatcaggctgaacatcttaagacagcagtacaaatggcagtattcatccacaattttaaaagaaaaggggggattggggggtacagtgcaggggaaagaatagtagacataatagcaacagacatacaaactaaagaattacaaaaacaaattacaaaaattcaaaattttcgggtttattacagggacagcagaaatccactttggaaaggaccagcaaagctcctctggaaaggtgaaggggcagtagtaatacaagataatagtgacataaaagtagtgccaagaagaaaagcaaagatcattagggattatggaaaacagatggcaggtgatgattgtgtggcaagtagacaggatgaggattagaacatggaaaagtttagtaaaacaccataaggaggagatatgagggacaattggagaagtgaattatataaatataaagtagtaaaaattgaaccattaggagtagcacccaccaaggcaaagagaagagtggtgcagagagaaaaaagagcagtgggaataggagctttgttccttgggttcttgggagcagcaggaagcactatgggcgcagcgtcaatgacgctgacggtacaggccagacaattattgtctggtatagtgcagcagcagaacaatttgctgagggctattgaggcgcaacagcatctgttgcaactcacagtctggggcatcaagcagctccaggcaagaatcctggctgtggaaagatacctaaaggatcaacagctcctggggatttggggttgctctggaaaactcatttgcaccactgctgtgccttggaatgctagttggagtaataaatctctggaacagatttggaatcacacgacctggatggagtgggacagagaaattaacaattacacaagcttaatacactccttaattgaagaatcgcaaaaccagcaagaaaagaatgaacaagaattattggaattagataaatgggcaagtttgtggaattggtttaacataacaaattggctgtggtatataaaattattcataatgatagtaggaggcttggtaggtttaagaatagtttttgctgtactttctatagtgaatagagttaggcagggatattcaccattatcgtttcagacccacctcccaaccccgaggggaccgagctcaagcttcgaacgcgtggggatcctctagagtcgagctcgcgaggatcatcaccggtgctagccggagccagaagcaccataagggacatgataagggagccagcagacctctgatctcttcctgaatgctaatcttaaacatcctgaggaagaatgggacttccatttggggtgggcctatgatagggtaataagacagtagtgaatatcaagctacaaaaagccccctttcaaattcttctcagtcctaacttttcatactaagcccagtccttccaaagcagactgtgaaagagtgatagttccgggagactagcaccggctagccgagcttggaacactttcccttcattaagaaccatccttgctactcagctgcaatcaatccagcccccaggtcttcactgaaccttttcccatctcttccaaaacatctgtttctgagaagtcctgtcctatagaggtctttcttcccaccggatttctcctacaccatttactcccacttgcagaactcccgtgtacaagtgtctttactgcttttatttgctcaacaaaatgcacatctcatataaaaataaatgaggagcatgcacacaccacaaacacaaacaggcatgcagaaatacacatacacacttccctcaatataaaccctttgtggctcatatatttaaaaagatgtaaaaaaaagagctgaagaaaatcatgtgtgatctctcagcagaatagatttattatttgtattgcttgcagaataaagcctatccttgaaagctctgaatcatgggcaagaggctcagtggtatctggaggacagggcactggccactgcagtcaccatcttctgccaggaagcctgcacctcaggggtgaattctttgccaaagtgaatggccagcacggtgaccagcacgttgcccaggagctgtgggaggaagataagaggtatgaacatgattagcaaaagggcctagcttggactcagaataatccagccttatcccaaccataaaataaaagcagaatggtagctggattgtagctgctattagcaatatgaaacctcttacatcagttacaatttatatgcagaaatatttatatgcagaaatattgctattgccttaacccagaaattatcactgttattctttagaatggtgcaaagaggcatgatacattgtatcattattgccctgaaagaaagagattagggaaagtattagaaataagataaacaaaaaagtatattaaaagaagaaagcattttttaaaattacaaatgcaaaattaccctgatttggtcaatatgtgtaccctgttacttctccccttcctatgacatgaacttaaccatagaaaagaaggggaaagaaaacatcaagggtcccatagactcaccttgaagttctcaggatccacatgcagcttgtcacagtgcagttcactcagctgggcaaaggtgcccttgagatcatccaggtgctttatggcatctcccaaggaagtcagcaccttcttgccatgtgccttgactttggggttgcccatgatggcagaggcagaggacaggttgccaaagctgtcaaagaacctctgggtccatgggtagacaaccaggagcctgtgagattgacaagaacagtttgacagtcagaaggtgccacaaatcctgagaagcaacctggacttttgccaggcacagggtccttccttccctcccttgtcctggtcaccagagcctaccttcccagggtttctcctccagcatcttccacattcaccttgtcccacaggcttgtgatagtagccttgtcctcctctgtgaaatgacccatggtgtctgtttgaggttgctagtgaacacagttgtgtcagaagcaaatgtaagcaatagatggctctgccctgacttttatgcccagccctggctcctgccctccctgctcctgggagtagattggccaaccctagggtgtggctccacagggtgaggtctaagtgatgacagccgtacctgtccttggctcttctggcactggcttaggagttggacttcaaaccctcagccctccctctaagatatatctcttggccccataccatcagtacaaattgctactaaaaacatcctcctttgcaagtgtatttacgacggtatcgatgtatgtgagcatgtgtcctctaacagcacaggccttttgccacctagctgtccaggggtgccttaaaatggcaaacaaggtttgttttcttttcctgttttcatgccttcctcttccatatccttgtttcatattaatacatgtgtatagatcctaaaaatctatacacatgtattaataaagcctgattctgccgcttctaggtatagaggccacctgcaagataaatatttgattcacaataactaatcattctatggcaattgataacaacaaatatatatatatatatatatatacgtatatgtgtatatatatatatatattcaggaaataatatattctagaatatgtcacattctgtctcaggcatccattttctttatgatgccgtttgaggtggagttttagtcaggtggtcagcttctccttttttttgccatctgccctgtaagcatcctgctggggacccagataggagtcatcactctaggctgagaacatctgggcacacaccctaagcctcagcatgactcatcatgactcagcattgctgtgcttgagccagaaggtttgcttagaaggttacacagaaccagaaggcgggggtggggcactgaccccgacaggggcctggccagaactgctcatgcttggactatgggaggtcactaatggagacacacagaaatgtaacaggaactaagggaattccggtgccctgcttaggagcttaatctttaatgaaagctaagctttcattaaaaaaagtctaaccagctgcattcgactttgactgcagcagctggttagaaggttctactggaggagggtcccagcccattgctaaattaacatcaggctctgagactggcagtatatctctaacagtggttgatgctatcttctggaacttgcctgctacattgagaccactgacccatacataggaagcccatagctctgtcctgaactgttaggccactggtccagagagtgtgcatctcctttgatcctcataataaccctatgagatagacacaattattactcttactttatagatgatgatcctgaaaacataggagtcaaggcacttgcccctagctgggggtataggggagcagtcccatgtagtagtagaatgaaaaatgctgctatgctgtgcctcccccacctttcccatgtctgccctctactcatggtctatctctcctggctcctgggagtcatggactccacccagcaccaccaacctgacctaaccacctatctgagcctgccagcctataacccatctgggccctgatagctggtggccagccctgaccccaccccaccctccctggaacctctgatagacacatctggcacaccagctcgcaaagtcaccgtgagggtcttgtgtttgctgagtcaaaattccttgaaatccaagtccttagagactcctgctcccaaatttacagtcatagacttcttcatggctgtctcctttatccacagaatgattcctttgcttcattgccccatccatctgatcctcctcatcagtgcagcacagggcccatgagcagtagctgcagagtctcacataggtctggcactgcctctgacatgtccgaccttaggcaaatgcttgactcttctgagctcggatcccttgagctcaggaggtcaaggctgcagtgagacatgatcttgccactgcactccagcctggacagcagagtgaaaccttgcctcacgaaacagaatacaaaaacaaacaaacaaaaaactgctccgcaatgcgcttccttgatgctctaccacataggtctgggtactttgtacacattatctcattgctgttcataattgttagattaattttgtaatattgatattattcctagaaagctgaggcctcaagatgataacttttattttctggacttgtaatagctttctcttgtattcaccatgttgtaactttcttagagtagtaacaatataaagttattgtgagtttttgcaaacacagcaaacacaacgacccatatagacattgatgtgaaattgtctattgtcaatttatgggaaaacaagtatgtactttttctactaagccattgaaacaggaataacagaacaagattgaaagaatacattttccgaaattacttgagtattatacaaagacaagcacgtggacctgggaggagggttattgtccatgactggtgtgtggagacaaatgcaggtttataatagatgggatggcatctagcgcaatgactttgccatcacttttagagagctcttgggggccccagtacacaagaggggacgcagggtatatgtagacatctcattctttttcttagtgtgagaataagaatagccatgacctgagtttatagacaatgagcccttttctctctcccactcagcagctatgagatggcttgccctgcctctctactaggctgactcactccaaggcccagcaatgggcagggctctgtcagggctttgatagcactatctgcagagccagggccgagaaggggtggactccagagactctccctcccattcccgagcagggtttgcttatttatgcatttaaatgatatatttattttaaaagaaataacaggagactgcccagccctggctgtgacatggaaactatgtagaatattttgggttccatttttttttccttctttcagttagaggaaaaggggctcactgcacatacactagacagaaagtcaggagctttgaatccaagcctgatcatttccatgtcatactgagaaagtccccacccttctctgagcctcagtttctctttttataagtaggagtctggagtaaatgatttccaatggctctcatttcaatacaaaatttccgtttattaaatgcatgagcttccgttactccaagactgagaaggaaattgaacctgagactcattgactggcaagatgtccccagaggctctcattcagcaataaaattctcaccttcacccaggcccactagtgtcagatttgcatgcgttcgcgtaaaaaaggatatgcccttgactatgtcggacaaatagtcaagggcatatcctgaggtacccaggcggcgcacaagctatataaacctgaaggaaatctcaactttacacttaggtcaagttacttatcgtactagagcttcagcaggaaatttaactaaaatctaatttaaccagcatagcaaatatcatttattcccaaaatgctaaagtttgagataaacggacttgatttccggctgttttgacactatccagaatgccggtactatgggtggggcagtagcccgactgcacgtcgagcggccgcatcgatgccgtagtacctttaagaccaatgacttacaaggcagctgtagatcttagccactttttaaaagaaaaggggggactggaagggctaattcactcccaaagaagacaagatagatctgctttttgcctgtactgggtctctctggttagaccagatctgagcctgggagctctctggctaactagggaacccactgcttaagcctcaataaagcttcagctgctcgagctagcagatctttttccctctgccaaaaattatggggacatcatgaagccccttgagcatctgacttctggctaataaaggaaatttattttcattgcaatagtgtgttggaattttttgtgtctctcactcggaaggacatatgggagggcaaatcatttaaaacatcagaatgagtatttggtttagagtttggcaacatatgcccatatgctggctgccatgaacaaaggttggctataaagaggtcatcagtatatgaaacagccccctgctgtccattccttattccatagaaaagccttgacttgaggttagattttttttatattttgttttgtgttatttttttctttaacatccctaaaattttccttacatgttttactagccagatttttcctcctctcctgactactcccagtcatagctgtccctcttctcttatggagatccctcgacctgcagcccaagcttggcgtaatcatggtcatagctgtttcctgtgtgaaattgttatccgctcacaattccacacaacatacgagccggaagcataaagtgtaaagcctggggtgcctaatgagtgagctaactcacattaattgcgttgcgctcactgcccgctttccagtcgggaaacctgtcgtgccagcggatccgcatctcaattagtcagcaaccatagtcccgcccctaactccgcccatcccgcccctaactccgcccagttccgcccattctccgccccatggctgactaattttttttatttatgcagaggccgaggccgcctcggcctctgagctattccagaagtagtgaggaggcttttttggaggcctaggcttttgcaaaaagctgtcgactgcagaggcctgcatgcaagcttggcgtaatcatggtcatagctgtttcctgtgtgaaattgttatccgctcacaattccacacaacatacgagccggaagcataaagtgtaaagcctggggtgcctaatgagtgagctaactcacattaattgcgttgcgctcactgcccgctttccagtcgggaaacctgtcgtgccagctgcattaatgaatcggccaacgcgcggggagaggcggtttgcgtattgggcgctcttccgcttcctcgctcactgactcgctgcgctcggtcgttcggctgcggcgagcggtatcagctcactcaaaggcggtaatacggttatccacagaatcaggggataacgcaggaaagaacatgtgagcaaaaggccagcaaaaggccaggaaccgtaaaaaggccgcgttgctggcgtttttccataggctccgcccccctgacgagcatcacaaaaatcgacgctcaagtcagaggtggcgaaacccgacaggactataaagataccaggcgtttccccctggaagctccctcgtgcgctctcctgttccgaccctgccgcttaccggatacctgtccgcctttctcccttcgggaagcgtggcgctttctcatagctcacgctgtaggtatctcagttcggtgtaggtcgttcgctccaagctgggctgtgtgcacgaaccccccgttcagcccgaccgctgcgccttatccggtaactatcgtcttgagtccaacccggtaagacacgacttatcgccactggcagcagccactggtaacaggattagcagagcgaggtatgtaggcggtgctacagagttcttgaagtggtggcctaactacggctacactagaagaacagtatttggtatctgcgctctgctgaagccagttaccttcggaaaaagagttggtagctcttgatccggcaaacaaaccaccgctggtagcggtggtttttttgtttgcaagcagcagattacgcgcagaaaaaaaggatctcaagaagatcctttgatcttttctacggggtctgacgctcagtggaacgaaaactcacgttaagggattttggtcatgagattatcaaaaaggatcttcacctagatccttttaaattaaaaatgaagttttaaatcaatctaaagtatatatgagtaaacttggtctgacagttaccaatgcttaatcagtgaggcacctatctcagcgatctgtctatttcgttcatccatagttgcctgactccccgtcgtgtagataactacgatacgggagggcttaccatctggccccagtgctgcaatgataccgcgagacccacgctcaccggctccagatttatcagcaataaaccagccagccggaagggccgagcgcagaagtggtcctgcaactttatccgcctccatccagtctattaattgttgccgggaagctagagtaagtagttcgccagttaatagtttgcgcaacgttgttgccattgctacaggcatcgtggtgtcacgctcgtcgtttggtatggcttcattcagctccggttcccaacgatcaaggcgagttacatgatcccccatgttgtgcaaaaaagcggttagctccttcggtcctccgatcgttgtcagaagtaagttggccgcagtgttatcactcatggttatggcagcactgcataattctcttactgtcatgccatccgtaagatgcttttctgtgactggtgagtactcaaccaagtcattctgagaatagtgtatgcggcgaccgagttgctcttgcccggcgtcaatacgggataataccgcgccacatagcagaactttaaaagtgctcatcattggaaaacgttcttcggggcgaaaactctcaaggatcttaccgctgttgagatccagttcgatgtaacccactcgtgcacccaactgatcttcagcatcttttactttcaccagcgtttctgggtgagcaaaaacaggaaggcaaaatgccgcaaaaaagggaataagggcgacacggaaatgttgaatactcatactcttcctttttcaatattattgaagcatttatcagggttattgtctcatgagcggatacatatttgaatgtatttagaaaaataaacaaataggggttccgcgcacatttccccgaaaagtgccacctgacgtctaagaaaccattattatcatgacattaacctataaaaataggcgtatcacgaggccctttcgtctcgcgcgtttcggtgatgacggtgaaaacctctgacacatgcagctcccggagacggtcacagcttgtctgtaagcggatgccgggagcagacaagcccgtcagggcgcgtcagcgggtgttggcgggtgtcggggctggcttaactatgcggcatcagagcagattgtactgagagtgcaccatatgcggtgtgaaataccgcacagatgcgtaaggagaaaataccgcatcaggcgccattcgccattcaggctgcgcaactgttgggaagggcgatcggtgcgggcctcttcgctattacgccagctggcgaaagggggatgtgctgcaaggcgattaagttgggtaacgccagggttttcccagtcacgacgttgtaaaacgacggccagtgaattc

SEQ ID NO: 22 - DNA, 11674 bp, Artificial Sequence
  Synthetic: TL20d-rGbGM-r7SK/sh734
ggccgcctcggccaaacagcccttgagtttaccactccctatcagtgatagagaaaagtgaaagtcgagtttaccactccctatcagtgatagagaaaagtgaaagtcgagtttaccactccctatcagtgatagagaaaagtgaaagtcgagtttaccactccctatcagtgatagagaaaagtgaaagtcgagtttaccagtccctatcagtgatagagaaaagtgaaagtcgagtttaccactccctatcagtgatagagaaaagtgaaagtcgagtttaccactccctatcagtgatagagaaaagtgaaagtcgagctcgccatgggaggcgtggcctgggcgggactggggagtggcgagccctcagatcctgcatataagcagctgctttttgcctgtactgggtctctctggttagaccagatctgagcctgggagctctctggctaactagggaacccactgcttaagcctcaataaagcttgccttgagtgcttcaagtagtgtgtgcccgtctgttgtgtgactctggtaactagagatccctcagacccttttagtcagtgtggaaaatctctagcagtggcgcccgaacagggacttgaaagcgaaagggaaaccagaggagctctctcgacgcaggactcggcttgctgaagcgcgcacggcaagaggcgaggggcggcgactggtgagtacgccaaaaattttgactagcggaggctagaaggagagagatgggtgcgagagcgtcagtattaagcgggggagaattagatcgcgatgggaaaaaattcggttaaggccagggggaaagaaaaaatataaattaaaacatatagtatgggcaagcagggagctagaacgattcgcagttaatactggcctgttagaaacatcagaaggctgtagacaaatactgggacagctacaaccatcccttcagacaggatcagaagaacttagatcattatataatacagtagcaaccctctattgtgtgcatcaaaggatagagataaaagacaccaaggaagctttagacaagatagaggaagagcaaaacaaaagtaagaaaaaagcacagcaagcagcaggatcttcagacctggaaattccctacaatccccaaagtcaaggagtagtagaatctatgaataaagaattaaagaaaattataggacaggtaagagatcaggctgaacatcttaagacagcagtacaaatggcagtattcatccacaattttaaaagaaaaggggggattggggggtacagtgcaggggaaagaatagtagacataatagcaacagacatacaaactaaagaattacaaaaacaaattacaaaaattcaaaattttcgggtttattacagggacagcagaaatccactttggaaaggaccagcaaagctcctctggaaaggtgaaggggcagtagtaatacaagataatagtgacataaaagtagtgccaagaagaaaagcaaagatcattagggattatggaaaacagatggcaggtgatgattgtgtggcaagtagacaggatgaggattagaacatggaaaagtttagtaaaacaccataaggaggagatatgagggacaattggagaagtgaattatataaatataaagtagtaaaaattgaaccattaggagtagcacccaccaaggcaaagagaagagtggtgcagagagaaaaaagagcagtgggaataggagctttgttccttgggttcttgggagcagcaggaagcactatgggcgcagcgtcaatgacgctgacggtacaggccagacaattattgtctggtatagtgcagcagcagaacaatttgctgagggctattgaggcgcaacagcatctgttgcaactcacagtctggggcatcaagcagctccaggcaagaatcctggctgtggaaagatacctaaaggatcaacagctcctggggatttggggttgctctggaaaactcatttgcaccactgctgtgccttggaatgctagttggagtaataaatctctggaacagatttggaatcacacgacctggatggagtgggacagagaaattaacaattacacaagcttaatacactccttaattgaagaatcgcaaaaccagcaagaaaagaatgaacaagaattattggaattagataaatgggcaagtttgtggaattggtttaacataacaaattggctgtggtatataaaattattcataatgatagtaggaggcttggtaggtttaagaatagtttttgctgtactttctatagtgaatagagttaggcagggatattcaccattatcgtttcagacccacctcccaaccccgaggggaccgagctcaagcttcgaacgcgtggggatcctctagagtcgagctcgcgaggatcatcaccggtgctagccggagccagaagcaccataagggacatgataagggagccagcagacctctgatctcttcctgaatgctaatcttaaacatcctgaggaagaatgggacttccatttggggtgggcctatgatagggtaataagacagtagtgaatatcaagctacaaaaagccccctttcaaattcttctcagtcctaacttttcatactaagcccagtccttccaaagcagactgtgaaagagtgatagttccgggagactagcaccggctagccgagcttggaacactttcccttcattaagaaccatccttgctactcagctgcaatcaatccagcccccaggtcttcactgaaccttttcccatctcttccaaaacatctgtttctgagaagtcctgtcctatagaggtctttcttcccaccggatttctcctacaccatttactcccacttgcagaactcccgtgtacaagtgtctttactgcttttatttgctcaacaaaatgcacatctcatataaaaataaatgaggagcatgcacacaccacaaacacaaacaggcatgcagaaatacacatacacacttccctcaatataaaccctttgtggctcatatatttaaaaagatgtaaaaaaaagagctgaagaaaatcatgtgtgatctctcagcagaatagatttattatttgtattgcttgcagaataaagcctatccttgaaagctctgaatcatgggcaagaggctcagtggtatctggaggacagggcactggccactgcagtcaccatcttctgccaggaagcctgcacctcaggggtgaattctttgccaaagtgaatggccagcacggtgaccagcacgttgcccaggagctgtgggaggaagataagaggtatgaacatgattagcaaaagggcctagcttggactcagaataatccagccttatcccaaccataaaataaaagcagaatggtagctggattgtagctgctattagcaatatgaaacctcttacatcagttacaatttatatgcagaaatatttatatgcagaaatattgctattgccttaacccagaaattatcactgttattctttagaatggtgcaaagaggcatgatacattgtatcattattgccctgaaagaaagagattagggaaagtattagaaataagataaacaaaaaagtatattaaaagaagaaagcattttttaaaattacaaatgcaaaattaccctgatttggtcaatatgtgtaccctgttacttctccccttcctatgacatgaacttaaccatagaaaagaaggggaaagaaaacatcaagggtcccatagactcaccttgaagttctcaggatccacatgcagcttgtcacagtgcagttcactcagctgggcaaaggtgcccttgagatcatccaggtgctttatggcatctcccaaggaagtcagcaccttcttgccatgtgccttgactttggggttgcccatgatggcagaggcagaggacaggttgccaaagctgtcaaagaacctctgggtccatgggtagacaaccaggagcctgtgagattgacaagaacagtttgacagtcagaaggtgccacaaatcctgagaagcaacctggacttttgccaggcacagggtccttccttccctcccttgtcctggtcaccagagcctaccttcccagggtttctcctccagcatcttccacattcaccttgtcccacaggcttgtgatagtagccttgtcctcctctgtgaaatgacccatggtgtctgtttgaggttgctagtgaacacagttgtgtcagaagcaaatgtaagcaatagatggctctgccctgacttttatgcccagccctggctcctgccctccctgctcctgggagtagattggccaaccctagggtgtggctccacagggtgaggtctaagtgatgacagccgtacctgtccttggctcttctggcactggcttaggagttggacttcaaaccctcagccctccctctaagatatatctcttggccccataccatcagtacaaattgctactaaaaacatcctcctttgcaagtgtatttacgacggtatcgatgtatgtgagcatgtgtcctctaacagcacaggccttttgccacctagctgtccaggggtgccttaaaatggcaaacaaggtttgttttcttttcctgttttcatgccttcctcttccatatccttgtttcatattaatacatgtgtatagatcctaaaaatctatacacatgtattaataaagcctgattctgccgcttctaggtatagaggccacctgcaagataaatatttgattcacaataactaatcattctatggcaattgataacaacaaatatatatatatatatatatatacgtatatgtgtatatatatatatatattcaggaaataatatattctagaatatgtcacattctgtctcaggcatccattttctttatgatgccgtttgaggtggagttttagtcaggtggtcagcttctccttttttttgccatctgccctgtaagcatcctgctggggacccagataggagtcatcactctaggctgagaacatctgggcacacaccctaagcctcagcatgactcatcatgactcagcattgctgtgcttgagccagaaggtttgcttagaaggttacacagaaccagaaggcgggggtggggcactgaccccgacaggggcctggccagaactgctcatgcttggactatgggaggtcactaatggagacacacagaaatgtaacaggaactaagggaattccggtgccctgcttaggagcttaatctttaatgaaagctaagctttcattaaaaaaagtctaaccagctgcattcgactttgactgcagcagctggttagaaggttctactggaggagggtcccagcccattgctaaattaacatcaggctctgagactggcagtatatctctaacagtggttgatgctatcttctggaacttgcctgctacattgagaccactgacccatacataggaagcccatagctctgtcctgaactgttaggccactggtccagagagtgtgcatctcctttgatcctcataataaccctatgagatagacacaattattactcttactttatagatgatgatcctgaaaacataggagtcaaggcacttgcccctagctgggggtataggggagcagtcccatgtagtagtagaatgaaaaatgctgctatgctgtgcctcccccacctttcccatgtctgccctctactcatggtctatctctcctggctcctgggagtcatggactccacccagcaccaccaacctgacctaaccacctatctgagcctgccagcctataacccatctgggccctgatagctggtggccagccctgaccccaccccaccctccctggaacctctgatagacacatctggcacaccagctcgcaaagtcaccgtgagggtcttgtgtttgctgagtcaaaattccttgaaatccaagtccttagagactcctgctcccaaatttacagtcatagacttcttcatggctgtctcctttatccacagaatgattcctttgcttcattgccccatccatctgatcctcctcatcagtgcagcacagggcccatgagcagtagctgcagagtctcacataggtctggcactgcctctgacatgtccgaccttaggcaaatgcttgactcttctgagctcggatcccttgagctcaggaggtcaaggctgcagtgagacatgatcttgccactgcactccagcctggacagcagagtgaaaccttgcctcacgaaacagaatacaaaaacaaacaaacaaaaaactgctccgcaatgcgcttccttgatgctctaccacataggtctgggtactttgtacacattatctcattgctgttcataattgttagattaattttgtaatattgatattattcctagaaagctgaggcctcaagatgataacttttattttctggacttgtaatagctttctcttgtattcaccatgttgtaactttcttagagtagtaacaatataaagttattgtgagtttttgcaaacacagcaaacacaacgacccatatagacattgatgtgaaattgtctattgtcaatttatgggaaaacaagtatgtactttttctactaagccattgaaacaggaataacagaacaagattgaaagaatacattttccgaaattacttgagtattatacaaagacaagcacgtggacctgggaggagggttattgtccatgactggtgtgtggagacaaatgcaggtttataatagatgggatggcatctagcgcaatgactttgccatcacttttagagagctcttgggggccccagtacacaagaggggacgcagggtatatgtagacatctcattctttttcttagtgtgagaataagaatagccatgacctgagtttatagacaatgagcccttttctctctcccactcagcagctatgagatggcttgccctgcctctctactaggctgactcactccaaggcccagcaatgggcagggctctgtcagggctttgatagcactatctgcagagccagggccgagaaggggtggactccagagactctccctcccattcccgagcagggtttgcttatttatgcatttaaatgatatatttattttaaaagaaataacaggagactgcccagccctggctgtgacatggaaactatgtagaatattttgggttccatttttttttccttctttcagttagaggaaaaggggctcactgcacatacactagacagaaagtcaggagctttgaatccaagcctgatcatttccatgtcatactgagaaagtccccacccttctctgagcctcagtttctctttttataagtaggagtctggagtaaatgatttccaatggctctcatttcaatacaaaatttccgtttattaaatgcatgagcttccgttactccaagactgagaaggaaattgaacctgagactcattgactggcaagatgtccccagaggctctcattcagcaataaaattctcaccttcacccaggcccactagtgtcagatttgcatgcgttcgcgtacaaaaaaggatatgcccttgactatgtcggacaaatagtcaagggcatatcctgaggtacccaggcggcgcacaagctatataaacctgaaggaaatctcaactttacacttaggtcaagttacttatcgtactagagcttcagcaggaaatttaactaaaatctaatttaaccagcatagcaaatatcatttattcccaaaatgctaaagtttgagataaacggacttgatttccggctgttttgacactatccagaatgccttgcagatgggtggggcatgctaaatactgcacgtcgatgcggccgcatcgatgccgtagtacctttaagaccaatgacttacaaggcagctgtagatcttagccactttttaaaagaaaaggggggactggaagggctaattcactcccaaagaagacaagatagatctgctttttgcctgtactgggtctctctggttagaccagatctgagcctgggagctctctggctaactagggaacccactgcttaagcctcaataaagcttcagctgctcgagctagcagatctttttccctctgccaaaaattatggggacatcatgaagccccttgagcatctgacttctggctaataaaggaaatttattttcattgcaatagtgtgttggaattttttgtgtctctcactcggaaggacatatgggagggcaaatcatttaaaacatcagaatgagtatttggtttagagtttggcaacatatgcccatatgctggctgccatgaacaaaggttggctataaagaggtcatcagtatatgaaacagccccctgctgtccattccttattccatagaaaagccttgacttgaggttagattttttttatattttgttttgtgttatttttttctttaacatccctaaaattttccttacatgttttactagccagatttttcctcctctcctgactactcccagtcatagctgtccctcttctcttatggagatccctcgacctgcagcccaagcttggcgtaatcatggtcatagctgtttcctgtgtgaaattgttatccgctcacaattccacacaacatacgagccggaagcataaagtgtaaagcctggggtgcctaatgagtgagctaactcacattaattgcgttgcgctcactgcccgctttccagtcgggaaacctgtcgtgccagcggatccgcatctcaattagtcagcaaccatagtcccgcccctaactccgcccatcccgcccctaactccgcccagttccgcccattctccgccccatggctgactaattttttttatttatgcagaggccgaggccgcctcggcctctgagctattccagaagtagtgaggaggcttttttggaggcctaggcttttgcaaaaagctgtcgactgcagaggcctgcatgcaagcttggcgtaatcatggtcatagctgtttcctgtgtgaaattgttatccgctcacaattccacacaacatacgagccggaagcataaagtgtaaagcctggggtgcctaatgagtgagctaactcacattaattgcgttgcgctcactgcccgctttccagtcgggaaacctgtcgtgccagctgcattaatgaatcggccaacgcgcggggagaggcggtttgcgtattgggcgctcttccgcttcctcgctcactgactcgctgcgctcggtcgttcggctgcggcgagcggtatcagctcactcaaaggcggtaatacggttatccacagaatcaggggataacgcaggaaagaacatgtgagcaaaaggccagcaaaaggccaggaaccgtaaaaaggccgcgttgctggcgtttttccataggctccgcccccctgacgagcatcacaaaaatcgacgctcaagtcagaggtggcgaaacccgacaggactataaagataccaggcgtttccccctggaagctccctcgtgcgctctcctgttccgaccctgccgcttaccggatacctgtccgcctttctcccttcgggaagcgtggcgctttctcatagctcacgctgtaggtatctcagttcggtgtaggtcgttcgctccaagctgggctgtgtgcacgaaccccccgttcagcccgaccgctgcgccttatccggtaactatcgtcttgagtccaacccggtaagacacgacttatcgccactggcagcagccactggtaacaggattagcagagcgaggtatgtaggcggtgctacagagttcttgaagtggtggcctaactacggctacactagaagaacagtatttggtatctgcgctctgctgaagccagttaccttcggaaaaagagttggtagctcttgatccggcaaacaaaccaccgctggtagcggtggtttttttgtttgcaagcagcagattacgcgcagaaaaaaaggatctcaagaagatcctttgatcttttctacggggtctgacgctcagtggaacgaaaactcacgttaagggattttggtcatgagattatcaaaaaggatcttcacctagatccttttaaattaaaaatgaagttttaaatcaatctaaagtatatatgagtaaacttggtctgacagttaccaatgcttaatcagtgaggcacctatctcagcgatctgtctatttcgttcatccatagttgcctgactccccgtcgtgtagataactacgatacgggagggcttaccatctggccccagtgctgcaatgataccgcgagacccacgctcaccggctccagatttatcagcaataaaccagccagccggaagggccgagcgcagaagtggtcctgcaactttatccgcctccatccagtctattaattgttgccgggaagctagagtaagtagttcgccagttaatagtttgcgcaacgttgttgccattgctacaggcatcgtggtgtcacgctcgtcgtttggtatggcttcattcagctccggttcccaacgatcaaggcgagttacatgatcccccatgttgtgcaaaaaagcggttagctccttcggtcctccgatcgttgtcagaagtaagttggccgcagtgttatcactcatggttatggcagcactgcataattctcttactgtcatgccatccgtaagatgcttttctgtgactggtgagtactcaaccaagtcattctgagaatagtgtatgcggcgaccgagttgctcttgcccggcgtcaatacgggataataccgcgccacatagcagaactttaaaagtgctcatcattggaaaacgttcttcggggcgaaaactctcaaggatcttaccgctgttgagatccagttcgatgtaacccactcgtgcacccaactgatcttcagcatcttttactttcaccagcgtttctgggtgagcaaaaacaggaaggcaaaatgccgcaaaaaagggaataagggcgacacggaaatgttgaatactcatactcttcctttttcaatattattgaagcatttatcagggttattgtctcatgagcggatacatatttgaatgtatttagaaaaataaacaaataggggttccgcgcacatttccccgaaaagtgccacctgacgtctaagaaaccattattatcatgacattaacctataaaaataggcgtatcacgaggccctttcgtctcgcgcgtttcggtgatgacggtgaaaacctctgacacatgcagctcccggagacggtcacagcttgtctgtaagcggatgccgggagcagacaagcccgtcagggcgcgtcagcgggtgttggcgggtgtcggggctggcttaactatgcggcatcagagcagattgtactgagagtgcaccatatgcggtgtgaaataccgcacagatgcgtaaggagaaaataccgcatcaggcgccattcgccattcaggctgcgcaactgttgggaagggcgatcggtgcgggcctcttcgctattacgccagctggcgaaagggggatgtgctgcaaggcgattaagttgggtaacgccagggttttcccagtcacgacgttgtaaaacgacggccagtgaattc

SEQ ID NO: 23 - RNA, 111 nt, Artificial Sequence
  Synthetic: miRNA734 de novo (RNA form)
acccguacauauuuuuguguagcucuaguuuauagucaagggcauauccuuguguuuuuuuugaaggauaugcccuugacuauaaacuagcgcuacacuuuuucgucuugu

SEQ ID NO: 24 - RNA, 111 nt, Artificial Sequence
  Synthetic: miRNA211 de novo (RNA form)
acccguacauauuuuuguguagcucuaguuauaaaucaaggucauaaccuuguguuuuuuuugaagguuaugaccuugauuuauaacuagcgcuacacuuuuucgucuugu

SEQ ID NO: 25 - DNA, 166 bp, Artificial Sequence
  Synthetic: miRNA211-3G
ccggatcaacgccctaggtttatgtttggatgaactgacatacgcgtatccgtcttttaaatcaaggtcataaccgtagtgaaatatatattaaacaggttatgaccttgatttaaaatacggtaacgcggaattcgcaactattttatcaattttttgcgtcgac

SEQ ID NO: 26 - DNA, 166 bp, Artificial Sequence
  Synthetic: miRNA734-3G
ccggatcaacgccctaggtttatgtttggatgaactgacatacgcgtatccgtcttatagtcaagggcatatcctgtagtgaaatatatattaaacaaggatatgcccttgactataatacggtaacgcggaattcgcaactattttatcaattttttgcgtcgac

SEQ ID NO: 27 - DNA, 56 bp, Artificial Sequence
  Synthetic: shHPRT 616
gcaggcagtataatccaaatacctgacccatatttggattatactgcctgcttttt

SEQ ID NO: 28 - DNA, 55 bp, Artificial Sequence
  Synthetic: shHPRT 211
ggttatgaccttgatttatacctgacccatattaaatcaaggtcataaccttttt

SEQ ID NO: 29 - DNA, 56 bp, Artificial Sequence
  Synthetic: shHPRT 734.1
gggatatgcccttgactaatacctgacccatattagtcaagggcatatcccttttt

SEQ ID NO: 30 - DNA, 52 bp, Artificial Sequence
  Synthetic: shHPRT 734
aggatatgcccttgactatttgtccgacatagtcaagggcatatcctttttt

SEQ ID NO: 31 - RNA, 51 nt, Artificial Sequence
  Synthetic: Modified sh734
aggauaugcccuugacuaugcccugacccagcauagucaagggcauauccu

SEQ ID NO: 32 - DNA, 248 bp, Homo sapiens
  misc_feature: Homo sapiens cell-line HEK-293 7SK RNA promoter region
tcgacgtgcagtatttagcatgccccacccatctgcaaggcattctggatagtgtcaaaacagccggaaatcaagtccgtttatctcaaactttagcattttgggaataaatgatatttgctatgctggttaaattagattttagttaaatttcctgctgaagctctagtacgataagtaacttgacctaagtgtaaagttgagatttccttcaggtttatatagcttgtgcgccgcctgggtacctc

SEQ ID NO: 33 - DNA, 248 bp, Homo sapiens
  misc_feature: Homo sapiens cell-line HEK-293 7SK RNA promoter region with mutation 1
tcgacgtgcagtcgggctactgccccacccatagtaccggcattctggatagtgtcaaaacagccggaaatcaagtccgtttatctcaaactttagcattttgggaataaatgatatttgctatgctggttaaattagattttagttaaatttcctgctgaagctctagtacgataagtaacttgacctaagtgtaaagttgagatttccttcaggtttatatagcttgtgcgccgcctgggtacctc

SEQ ID NO: 34 - RNA, 9 nt, Artificial Sequence
  Synthetic: hsa-miR-22 loop sequence
ccugaccca

SEQ ID NO: 35 - DNA, 9 bp, Artificial Sequence
  Synthetic: Hairpin loop sequence of sh734 (5 to 3)
ttgtccgac

SEQ ID NO: 36 - DNA, 483 bp, Artificial Sequence
  Synthetic: EF1a-miRNA734-Denovo-SV40 polyA
ggatatcggctccggtgcccgtcagtgggcagagcgcacatcgcccacagtccccgagaagttggggggaggggtcggcaattgaaccggtgcctagagaaggtggcgcggggtaaactgggaaagtgatgtcgtgtactggctccgcctttttcccgagggtgggggagaaccgtatataagtgcagtagtcgccgtgaacgttcttttcgcaacgggtttgccgccagaacacaggatgacccgtacatatttttgtgtagctctagttataaatcaaggtcataaccttgtgttttttttgaaggttatgaccttgatttataactagcgctacactttttcgtcttgttagaacttgtttattgcagcttataatggttacaaataaagcaatagcatcacaaatttcacaaataaagcatttttttcactgcattctagttgtggtttgtccaaactcatcaatgtatcttatcatct

SEQ ID NO: 37 - DNA, 483 bp, Artificial Sequence
  Synthetic: EF1a-miRNA211-Denovo-SV40 polyA
ggatatcggctccggtgcccgtcagtgggcagagcgcacatcgcccacagtccccgagaagttggggggaggggtcggcaattgaaccggtgcctagagaaggtggcgcggggtaaactgggaaagtgatgtcgtgtactggctccgcctttttcccgagggtgggggagaaccgtatataagtgcagtagtcgccgtgaacgttcttttcgcaacgggtttgccgccagaacacaggatgacccgtacatatttttgtgtagctctagtttatagtcaagggcatatccttgtgttttttttgaaggatatgcccttgactataaactagcgctacactttttcgtcttgttagaacttgtttattgcagcttataatggttacaaataaagcaatagcatcacaaatttcacaaataaagcatttttttcactgcattctagttgtggtttgtccaaactcatcaatgtatcttatcatct

SEQ ID NO: 38 - DNA, 537 bp, Artificial Sequence
  Synthetic: EF1a-miRNA734-3G-SV40 polyA
ggatatcggctccggtgcccgtcagtgggcagagcgcacatcgcccacagtccccgagaagttggggggaggggtcggcaattgaaccggtgcctagagaaggtggcgcggggtaaactgggaaagtgatgtcgtgtactggctccgcctttttcccgagggtgggggagaaccgtatataagtgcagtagtcgccgtgaacgttcttttcgcaacgggtttgccgccagaacacaggatgccggatcaacgccctaggtttatgtttggatgaactgacatacgcgtatccgtcttatagtcaagggcatatccagtagtgaaatatatattaaactggatatgcccttgactataatacggtaacgcggaattcgcaactattttatcaattttttgcgtcgactagaacttgtttattgcagcttataatggttacaaataaagcaatagcatcacaaatttcacaaataaagcatttttttcactgcattctagttgtggtttgtccaaactcatcaatgtatcttatcatct

SEQ ID NO: 39 - DNA, 696 bp, Artificial Sequence
  Synthetic: EF1a-miRNA211-3G-SV40 polyA
ggatatcggctccggtgcccgtcagtgggcagagcgcacatcgcccacagtccccgagaagttggggggaggggtcggcaattgaaccggtgcctagagaaggtggcgcggggtaaactgggaaagtgatgtcgtgtactggctccgcctttttcccgagggtgggggagaaccgtatataagtgcagtagtcgccgtgaacgttcttttcgcaacgggtttgccgccagaacacaggccggatcaacgccctaggtttatgtttggatgaactgacatacgcgtatccgtctataaatcaaggtcataacctgtagtgaaatatatattaaacaaggttatgaccttgatttattacggtaacgcggaattcgcaactattttatcaattttttgcgtcgacccggatcaacgccctaggtttatgtttggatgaactgacatacgcgtatccgtctataaatcaaggtcataacctgtagtgaaatatatattaaacaaggttatgaccttgatttattacggtaacgcggaattcgcaactattttatcaattttttgcgtcgacaacttgtttattgcagcttataatggttacaaataaagcaatagcatcacaaatttcacaaataaagcatttttttcactgcattctagttgtggtttgtccaaactcatcaatgtatcttatcatct

SEQ ID NO: 40 - DNA, 809 bp, Artificial Sequence
  Synthetic: Left Arm 150-EF1a-miRNA734-Denovo-SV40 polyA-Right Arm 150
gcttcttctctggaatcttcttcatcatcctcctgacaatcgataggtacctggctgtcgtccatgctgtgtttgctttaaaagccaggacggtcacctttggggtggtgacaagtgtgatcacttgggtggtggctgtgtttgcgtctcaagcttttcgaagcggccgcggatatcggctccggtgcccgtcagtgggcagagcgcacatcgcccacagtccccgagaagttggggggaggggtcggcaattgaaccggtgcctagagaaggtggcgcggggtaaactgggaaagtgatgtcgtgtactggctccgcctttttcccgagggtgggggagaaccgtatataagtgcagtagtcgccgtgaacgttcttttcgcaacgggtttgccgccagaacacaggatgacccgtacatatttttgtgtagctctagttataaatcaaggtcataaccttgtgttttttttgaaggttatgaccttgatttataactagcgctacactttttcgtcttgttagaacttgtttattgcagcttataatggttacaaataaagcaatagcatcacaaatttcacaaataaagcatttttttcactgcattctagttgtggtttgtccaaactcatcaatgtatcttatcatctacgcgtccaggaatcatctttaccagatctcaaaaagaaggtcttcattacacctgcagctctcattttccatacagtcagtatcaattctggaagaatttccagacattaaagatagtcatcttggggctggtcctgccgctgcttgtcatggtc

SEQ ID NO: 41 - DNA, 809 bp, Artificial Sequence
  Synthetic: miRNA211-Denovo
gcttcttctctggaatcttcttcatcatcctcctgacaatcgataggtacctggctgtcgtccatgctgtgtttgctttaaaagccaggacggtcacctttggggtggtgacaagtgtgatcacttgggtggtggctgtgtttgcgtctcaagcttttcgaagcggccgcggatatcggctccggtgcccgtcagtgggcagagcgcacatcgcccacagtccccgagaagttggggggaggggtcggcaattgaaccggtgcctagagaaggtggcgcggggtaaactgggaaagtgatgtcgtgtactggctccgcctttttcccgagggtgggggagaaccgtatataagtgcagtagtcgccgtgaacgttcttttcgcaacgggtttgccgccagaacacaggatgacccgtacatatttttgtgtagctctagtttatagtcaagggcatatccttgtgttttttttgaaggatatgcccttgactataaactagcgctacactttttcgtcttgttagaacttgtttattgcagcttataatggttacaaataaagcaatagcatcacaaatttcacaaataaagcatttttttcactgcattctagttgtggtttgtccaaactcatcaatgtatcttatcatctacgcgtccaggaatcatctttaccagatctcaaaaagaaggtcttcattacacctgcagctctcattttccatacagtcagtatcaattctggaagaatttccagacattaaagatagtcatcttggggctggtcctgccgctgcttgtcatggtc

SEQ ID NO: 42 - DNA, 863 bp, Artificial Sequence
  Synthetic: miRNA734-3G
gcttcttctctggaatcttcttcatcatcctcctgacaatcgataggtacctggctgtcgtccatgctgtgtttgctttaaaagccaggacggtcacctttggggtggtgacaagtgtgatcacttgggtggtggctgtgtttgcgtctcaagcttttcgaagcggccgcggatatcggctccggtgcccgtcagtgggcagagcgcacatcgcccacagtccccgagaagttggggggaggggtcggcaattgaaccggtgcctagagaaggtggcgcggggtaaactgggaaagtgatgtcgtgtactggctccgcctttttcccgagggtgggggagaaccgtatataagtgcagtagtcgccgtgaacgttcttttcgcaacgggtttgccgccagaacacaggatgccggatcaacgccctaggtttatgtttggatgaactgacatacgcgtatccgtcttatagtcaagggcatatccagtagtgaaatatatattaaactggatatgcccttgactataatacggtaacgcggaattcgcaactattttatcaattttttgcgtcgactagaacttgtttattgcagcttataatggttacaaataaagcaatagcatcacaaatttcacaaataaagcatttttttcactgcattctagttgtggtttgtccaaactcatcaatgtatcttatcatctacgcgtccaggaatcatctttaccagatctcaaaaagaaggtcttcattacacctgcagctctcattttccatacagtcagtatcaattctggaagaatttccagacattaaagatagtcatcttggggctggtcctgccgctgcttgtcatggtc

SEQ ID NO: 43 - DNA, 1022 bp, Artificial Sequence
  Synthetic: miRNA211-3G
gcttcttctctggaatcttcttcatcatcctcctgacaatcgataggtacctggctgtcgtccatgctgtgtttgctttaaaagccaggacggtcacctttggggtggtgacaagtgtgatcacttgggtggtggctgtgtttgcgtctcaagcttttcgaagcggccgcggatatcggctccggtgcccgtcagtgggcagagcgcacatcgcccacagtccccgagaagttggggggaggggtcggcaattgaaccggtgcctagagaaggtggcgcggggtaaactgggaaagtgatgtcgtgtactggctccgcctttttcccgagggtgggggagaaccgtatataagtgcagtagtcgccgtgaacgttcttttcgcaacgggtttgccgccagaacacaggccggatcaacgccctaggtttatgtttggatgaactgacatacgcgtatccgtctataaatcaaggtcataacctgtagtgaaatatatattaaacaaggttatgaccttgatttattacggtaacgcggaattcgcaactattttatcaattttttgcgtcgacccggatcaacgccctaggtttatgtttggatgaactgacatacgcgtatccgtctataaatcaaggtcataacctgtagtgaaatatatattaaacaaggttatgaccttgatttattacggtaacgcggaattcgcaactattttatcaattttttgcgtcgacaacttgtttattgcagcttataatggttacaaataaagcaatagcatcacaaatttcacaaataaagcatttttttcactgcattctagttgtggtttgtccaaactcatcaatgtatcttatcatctacgcgtccaggaatcatctttaccagatctcaaaaagaaggtcttcattacacctgcagctctcattttccatacagtcagtatcaattctggaagaatttccagacattaaagatagtcatcttggggctggtcctgccgctgcttgtcatggtc

SEQ ID NO: 44 - DNA, 20 bp, Artificial Sequence
  Synthetic: GbGM    F  5-3
tgacttccttgggagatgcc

SEQ ID NO: 45 - DNA, 20 bp, Artificial Sequence
  Synthetic: GbGM    R  5-3
caaagtgaatggccagcacg

SEQ ID NO: 46 - DNA, 20 bp, Artificial Sequence
  Synthetic: Probe     5- 3
agctcctgggcaacgtgctg

SEQ ID NO: 47 - DNA, 6565 bp, Artificial Sequence
  Synthetic: PTL20c
ggccgcctcggccaaacagcccttgagtttaccactccctatcagtgatagagaaaagtgaaagtcgagtttaccactccctatcagtgatagagaaaagtgaaagtcgagtttaccactccctatcagtgatagagaaaagtgaaagtcgagtttaccactccctatcagtgatagagaaaagtgaaagtcgagtttaccagtccctatcagtgatagagaaaagtgaaagtcgagtttaccactccctatcagtgatagagaaaagtgaaagtcgagtttaccactccctatcagtgatagagaaaagtgaaagtcgagctcgccatgggaggcgtggcctgggcgggactggggagtggcgagccctcagatcctgcatataagcagctgctttttgcctgtactgggtctctctggttagaccagatctgagcctgggagctctctggctaactagggaacccactgcttaagcctcaataaagcttgccttgagtgcttcaagtagtgtgtgcccgtctgttgtgtgactctggtaactagagatccctcagacccttttagtcagtgtggaaaatctctagcagtggcgcccgaacagggacttgaaagcgaaagggaaaccagaggagctctctcgacgcaggactcggcttgctgaagcgcgcacggcaagaggcgaggggcggcgactggtgagtacgccaaaaattttgactagcggaggctagaaggagagagatgggtgcgagagcgtcagtattaagcgggggagaattagatcgcgatgggaaaaaattcggttaaggccagggggaaagaaaaaatataaattaaaacatatagtatgggcaagcagggagctagaacgattcgcagttaatactggcctgttagaaacatcagaaggctgtagacaaatactgggacagctacaaccatcccttcagacaggatcagaagaacttagatcattatataatacagtagcaaccctctattgtgtgcatcaaaggatagagataaaagacaccaaggaagctttagacaagatagaggaagagcaaaacaaaagtaagaaaaaagcacagcaagcagcaggatcttcagacctggaaattccctacaatccccaaagtcaaggagtagtagaatctatgaataaagaattaaagaaaattataggacaggtaagagatcaggctgaacatcttaagacagcagtacaaatggcagtattcatccacaattttaaaagaaaaggggggattggggggtacagtgcaggggaaagaatagtagacataatagcaacagacatacaaactaaagaattacaaaaacaaattacaaaaattcaaaattttcgggtttattacagggacagcagaaatccactttggaaaggaccagcaaagctcctctggaaaggtgaaggggcagtagtaatacaagataatagtgacataaaagtagtgccaagaagaaaagcaaagatcattagggattatggaaaacagatggcaggtgatgattgtgtggcaagtagacaggatgaggattagaacatggaaaagtttagtaaaacaccataaggaggagatatgagggacaattggagaagtgaattatataaatataaagtagtaaaaattgaaccattaggagtagcacccaccaaggcaaagagaagagtggtgcagagagaaaaaagagcagtgggaataggagctttgttccttgggttcttgggagcagcaggaagcactatgggcgcagcgtcaatgacgctgacggtacaggccagacaattattgtctggtatagtgcagcagcagaacaatttgctgagggctattgaggcgcaacagcatctgttgcaactcacagtctggggcatcaagcagctccaggcaagaatcctggctgtggaaagatacctaaaggatcaacagctcctggggatttggggttgctctggaaaactcatttgcaccactgctgtgccttggaatgctagttggagtaataaatctctggaacagatttggaatcacacgacctggatggagtgggacagagaaattaacaattacacaagcttaatacactccttaattgaagaatcgcaaaaccagcaagaaaagaatgaacaagaattattggaattagataaatgggcaagtttgtggaattggtttaacataacaaattggctgtggtatataaaattattcataatgatagtaggaggcttggtaggtttaagaatagtttttgctgtactttctatagtgaatagagttaggcagggatattcaccattatcgtttcagacccacctcccaaccccgaggggaccgagctcaagcttcgaacgcgtgcggccgcatcgatgccgtagtacctttaagaccaatgacttacaaggcagctgtagatcttagccactttttaaaagaaaaggggggactggaagggctaattcactcccaaagaagacaagatccctgcaggcattcaaggccaggctggatgtggctctgggcagcctgggctgctggttgatgaccctgcacatagcagggggttggatctggatgagcactgtgctcctttgcaacccaggccgttctatgattctgtcattctaaatctctctttcagcctaaagctttttccccgtatccccccaggtgtctgcaggctcaaagagcagcgagaagcgttcagaggaaagcgatcccgtgccaccttccccgtgcccgggctgtccccgcacgctgccggctcggggatgcggggggagcgccggaccggagcggagccccgggcggctcgctgctgccccctagcgggggagggacgtaattacatccctgggggctttgggggggggctgtccccgtgagctccccagatctgctttttgcctgtactgggtctctctggttagaccagatctgagcctgggagctctctggctaactagggaacccactgcttaagcctcaataaagcttcagctgctcgagctagcagatctttttccctctgccaaaaattatggggacatcatgaagccccttgagcatctgacttctggctaataaaggaaatttattttcattgcaatagtgtgttggaattttttgtgtctctcactcggaaggacatatgggagggcaaatcatttaaaacatcagaatgagtatttggtttagagtttggcaacatatgcccatatgctggctgccatgaacaaaggttggctataaagaggtcatcagtatatgaaacagccccctgctgtccattccttattccatagaaaagccttgacttgaggttagattttttttatattttgttttgtgttatttttttctttaacatccctaaaattttccttacatgttttactagccagatttttcctcctctcctgactactcccagtcatagctgtccctcttctcttatggagatccctcgacctgcagcccaagcttggcgtaatcatggtcatagctgtttcctgtgtgaaattgttatccgctcacaattccacacaacatacgagccggaagcataaagtgtaaagcctggggtgcctaatgagtgagctaactcacattaattgcgttgcgctcactgcccgctttccagtcgggaaacctgtcgtgccagcggatccgcatctcaattagtcagcaaccatagtcccgcccctaactccgcccatcccgcccctaactccgcccagttccgcccattctccgccccatggctgactaattttttttatttatgcagaggccgaggccgcctcggcctctgagctattccagaagtagtgaggaggcttttttggaggcctaggcttttgcaaaaagctgtcgactgcagaggcctgcatgcaagcttggcgtaatcatggtcatagctgtttcctgtgtgaaattgttatccgctcacaattccacacaacatacgagccggaagcataaagtgtaaagcctggggtgcctaatgagtgagctaactcacattaattgcgttgcgctcactgcccgctttccagtcgggaaacctgtcgtgccagctgcattaatgaatcggccaacgcgcggggagaggcggtttgcgtattgggcgctcttccgcttcctcgctcactgactcgctgcgctcggtcgttcggctgcggcgagcggtatcagctcactcaaaggcggtaatacggttatccacagaatcaggggataacgcaggaaagaacatgtgagcaaaaggccagcaaaaggccaggaaccgtaaaaaggccgcgttgctggcgtttttccataggctccgcccccctgacgagcatcacaaaaatcgacgctcaagtcagaggtggcgaaacccgacaggactataaagataccaggcgtttccccctggaagctccctcgtgcgctctcctgttccgaccctgccgcttaccggatacctgtccgcctttctcccttcgggaagcgtggcgctttctcatagctcacgctgtaggtatctcagttcggtgtaggtcgttcgctccaagctgggctgtgtgcacgaaccccccgttcagcccgaccgctgcgccttatccggtaactatcgtcttgagtccaacccggtaagacacgacttatcgccactggcagcagccactggtaacaggattagcagagcgaggtatgtaggcggtgctacagagttcttgaagtggtggcctaactacggctacactagaagaacagtatttggtatctgcgctctgctgaagccagttaccttcggaaaaagagttggtagctcttgatccggcaaacaaaccaccgctggtagcggtggtttttttgtttgcaagcagcagattacgcgcagaaaaaaaggatctcaagaagatcctttgatcttttctacggggtctgacgctcagtggaacgaaaactcacgttaagggattttggtcatgagattatcaaaaaggatcttcacctagatccttttaaattaaaaatgaagttttaaatcaatctaaagtatatatgagtaaacttggtctgacagttaccaatgcttaatcagtgaggcacctatctcagcgatctgtctatttcgttcatccatagttgcctgactccccgtcgtgtagataactacgatacgggagggcttaccatctggccccagtgctgcaatgataccgcgagacccacgctcaccggctccagatttatcagcaataaaccagccagccggaagggccgagcgcagaagtggtcctgcaactttatccgcctccatccagtctattaattgttgccgggaagctagagtaagtagttcgccagttaatagtttgcgcaacgttgttgccattgctacaggcatcgtggtgtcacgctcgtcgtttggtatggcttcattcagctccggttcccaacgatcaaggcgagttacatgatcccccatgttgtgcaaaaaagcggttagctccttcggtcctccgatcgttgtcagaagtaagttggccgcagtgttatcactcatggttatggcagcactgcataattctcttactgtcatgccatccgtaagatgcttttctgtgactggtgagtactcaaccaagtcattctgagaatagtgtatgcggcgaccgagttgctcttgcccggcgtcaatacgggataataccgcgccacatagcagaactttaaaagtgctcatcattggaaaacgttcttcggggcgaaaactctcaaggatcttaccgctgttgagatccagttcgatgtaacccactcgtgcacccaactgatcttcagcatcttttactttcaccagcgtttctgggtgagcaaaaacaggaaggcaaaatgccgcaaaaaagggaataagggcgacacggaaatgttgaatactcatactcttcctttttcaatattattgaagcatttatcagggttattgtctcatgagcggatacatatttgaatgtatttagaaaaataaacaaataggggttccgcgcacatttccccgaaaagtgccacctgacgtctaagaaaccattattatcatgacattaacctataaaaataggcgtatcacgaggccctttcgtctcgcgcgtttcggtgatgacggtgaaaacctctgacacatgcagctcccggagacggtcacagcttgtctgtaagcggatgccgggagcagacaagcccgtcagggcgcgtcagcgggtgttggcgggtgtcggggctggcttaactatgcggcatcagagcagattgtactgagagtgcaccatatgcggtgtgaaataccgcacagatgcgtaaggagaaaataccgcatcaggcgccattcgccattcaggctgcgcaactgttgggaagggcgatcggtgcgggcctcttcgctattacgccagctggcgaaagggggatgtgctgcaaggcgattaagttgggtaacgccagggttttcccagtcacgacgttgtaaaacgacggccagtgaattc

SEQ ID NO: 48 - DNA, 3901 bp, Artificial Sequence
  Synthetic: PTL20c backbone including a 400bp cHS4 insulator
ggccgcctcggccaaacagcccttgagtttaccactccctatcagtgatagagaaaagtgaaagtcgagtttaccactccctatcagtgatagagaaaagtgaaagtcgagtttaccactccctatcagtgatagagaaaagtgaaagtcgagtttaccactccctatcagtgatagagaaaagtgaaagtcgagtttaccagtccctatcagtgatagagaaaagtgaaagtcgagtttaccactccctatcagtgatagagaaaagtgaaagtcgagtttaccactccctatcagtgatagagaaaagtgaaagtcgagctcgccatgggaggcgtggcctgggcgggactggggagtggcgagccctcagatcctgcatataagcagctgctttttgcctgtactgggtctctctggttagaccagatctgagcctgggagctctctggctaactagggaacccactgcttaagcctcaataaagcttgccttgagtgcttcaagtagtgtgtgcccgtctgttgtgtgactctggtaactagagatccctcagacccttttagtcagtgtggaaaatctctagcagtggcgcccgaacagggacttgaaagcgaaagggaaaccagaggagctctctcgacgcaggactcggcttgctgaagcgcgcacggcaagaggcgaggggcggcgactggtgagtacgccaaaaattttgactagcggaggctagaaggagagagatgggtgcgagagcgtcagtattaagcgggggagaattagatcgcgatgggaaaaaattcggttaaggccagggggaaagaaaaaatataaattaaaacatatagtatgggcaagcagggagctagaacgattcgcagttaatactggcctgttagaaacatcagaaggctgtagacaaatactgggacagctacaaccatcccttcagacaggatcagaagaacttagatcattatataatacagtagcaaccctctattgtgtgcatcaaaggatagagataaaagacaccaaggaagctttagacaagatagaggaagagcaaaacaaaagtaagaaaaaagcacagcaagcagcaggatcttcagacctggaaattccctacaatccccaaagtcaaggagtagtagaatctatgaataaagaattaaagaaaattataggacaggtaagagatcaggctgaacatcttaagacagcagtacaaatggcagtattcatccacaattttaaaagaaaaggggggattggggggtacagtgcaggggaaagaatagtagacataatagcaacagacatacaaactaaagaattacaaaaacaaattacaaaaattcaaaattttcgggtttattacagggacagcagaaatccactttggaaaggaccagcaaagctcctctggaaaggtgaaggggcagtagtaatacaagataatagtgacataaaagtagtgccaagaagaaaagcaaagatcattagggattatggaaaacagatggcaggtgatgattgtgtggcaagtagacaggatgaggattagaacatggaaaagtttagtaaaacaccataaggaggagatatgagggacaattggagaagtgaattatataaatataaagtagtaaaaattgaaccattaggagtagcacccaccaaggcaaagagaagagtggtgcagagagaaaaaagagcagtgggaataggagctttgttccttgggttcttgggagcagcaggaagcactatgggcgcagcgtcaatgacgctgacggtacaggccagacaattattgtctggtatagtgcagcagcagaacaatttgctgagggctattgaggcgcaacagcatctgttgcaactcacagtctggggcatcaagcagctccaggcaagaatcctggctgtggaaagatacctaaaggatcaacagctcctggggatttggggttgctctggaaaactcatttgcaccactgctgtgccttggaatgctagttggagtaataaatctctggaacagatttggaatcacacgacctggatggagtgggacagagaaattaacaattacacaagcttaatacactccttaattgaagaatcgcaaaaccagcaagaaaagaatgaacaagaattattggaattagataaatgggcaagtttgtggaattggtttaacataacaaattggctgtggtatataaaattattcataatgatagtaggaggcttggtaggtttaagaatagtttttgctgtactttctatagtgaatagagttaggcagggatattcaccattatcgtttcagacccacctcccaaccccgaggggaccgagctcaagcttcgaacgcgtgcggccgcatcgatgccgtagtacctttaagaccaatgacttacaaggcagctgtagatcttagccactttttaaaagaaaaggggggactggaagggctaattcactcccaaagaagacaagatccctgcaggcattcaaggccaggctggatgtggctctgggcagcctgggctgctggttgatgaccctgcacatagcagggggttggatctggatgagcactgtgctcctttgcaacccaggccgttctatgattctgtcattctaaatctctctttcagcctaaagctttttccccgtatccccccaggtgtctgcaggctcaaagagcagcgagaagcgttcagaggaaagcgatcccgtgccaccttccccgtgcccgggctgtccccgcacgctgccggctcggggatgcggggggagcgccggaccggagcggagccccgggcggctcgctgctgccccctagcgggggagggacgtaattacatccctgggggctttgggggggggctgtccccgtgagctccccagatctgctttttgcctgtactgggtctctctggttagaccagatctgagcctgggagctctctggctaactagggaacccactgcttaagcctcaataaagcttcagctgctcgagctagcagatctttttccctctgccaaaaattatggggacatcatgaagccccttgagcatctgacttctggctaataaaggaaatttattttcattgcaatagtgtgttggaattttttgtgtctctcactcggaaggacatatgggagggcaaatcatttaaaacatcagaatgagtatttggtttagagtttggcaacatatgcccatatgctggctgccatgaacaaaggttggctataaagaggtcatcagtatatgaaacagccccctgctgtccattccttattccatagaaaagccttgacttgaggttagattttttttatattttgttttgtgttatttttttctttaacatccctaaaattttccttacatgttttactagccagatttttcctcctctcctgactactcccagtcatagctgtccctcttctcttatggagatccctcgacctgcagcccaagcttggcgtaatcatggtcatagctgtttcctgtgtgaaattgttatccgctcacaattccacacaacatacgagccggaagcataaagtgtaaagcctggggtgcctaatgagtgagctaactcacattaattgcgttgcgctcactgcccgctttccagtcgggaaacctgtcgtgccagcggatccgcatctcaattagtcagcaaccatagtcccgcccctaactccgcccatcccgcccctaactccgcccagttccgcccattctccgccccatggctgactaattttttttatttatgcagaggccgaggccgcctcggcctctgagctattccagaagtagtgaggaggcttttttggaggcctaggcttttgcaaaaagct

SEQ ID NO: 49 - DNA, 412 bp, Artificial Sequence
  Synthetic: cHS4 insulator
atccctgcaggcattcaaggccaggctggatgtggctctgggcagcctgggctgctggttgatgaccctgcacatagcagggggttggatctggatgagcactgtgctcctttgcaacccaggccgttctatgattctgtcattctaaatctctctttcagcctaaagctttttccccgtatccccccaggtgtctgcaggctcaaagagcagcgagaagcgttcagaggaaagcgatcccgtgccaccttccccgtgcccgggctgtccccgcacgctgccggctcggggatgcggggggagcgccggaccggagcggagccccgggcggctcgctgctgccccctagcgggggagggacgtaattacatccctgggggctttgggggggggctgtccccgtgagctcccc

SEQ ID NO: 50 - DNA, 5221 bp, Artificial Sequence
  Synthetic: sGbGM vector cassette
ggagccagaagcaccataagggacatggggatcctctagagtcgagctcgcgaggatcatcaccggtgctagccgataagggagccagcagacctctgatctcttcctgaatgctaatcttaaacatcctgaggaagaatgggacttccatttggggtgggcctatgatagggtaataagacagtagtgaatatcaagctacaaaaagccccctttcaaattcttctcagtcctaacttttcatactaagcccagtccttccaaagcagactgtgaaagagtgatagttccgggagactagcaccggctagccgagcttggaacactttcccttcattaagaaccatccttgctactcagctgcaatcaatccagcccccaggtcttcactgaaccttttcccatctcttccaaaacatctgtttctgagaagtcctgtcctatagaggtctttcttcccaccggatttctcctacaccatttactcccacttgcagaactcccgtgtacaagtgtctttactgcttttatttgctcaacaaaatgcacatctcatataaaaataaatgaggagcatgcacacaccacaaacacaaacaggcatgcagaaatacacatacacacttccctcaatataaaccctttgtggctcatatatttaaaaagatgtaaaaaaaagagctgaagaaaatcatgtgtgatctctcagcagaatagatttattatttgtattgcttgcagaataaagcctatccttgaaagctctgaatcatgggcaagaggctcagtggtatctggaggacagggcactggccactgcagtcaccatcttctgccaggaagcctgcacctcaggggtgaattctttgccaaagtgaatggccagcacggtgaccagcacgttgcccaggagctgtgggaggaagataagaggtatgaacatgattagcaaaagggcctagcttggactcagaataatccagccttatcccaaccataaaataaaagcagaatggtagctggattgtagctgctattagcaatatgaaacctcttacatcagttacaatttatatgcagaaatatttatatgcagaaatattgctattgccttaacccagaaattatcactgttattctttagaatggtgcaaagaggcatgatacattgtatcattattgccctgaaagaaagagattagggaaagtattagaaataagataaacaaaaaagtatattaaaagaagaaagcattttttaaaattacaaatgcaaaattaccctgatttggtcaatatgtgtaccctgttacttctccccttcctatgacatgaacttaaccatagaaaagaaggggaaagaaaacatcaagggtcccatagactcaccttgaagttctcaggatccacatgcagcttgtcacagtgcagttcactcagctgggcaaaggtgcccttgagatcatccaggtgctttatggcatctcccaaggaagtcagcaccttcttgccatgtgccttgactttggggttgcccatgatggcagaggcagaggacaggttgccaaagctgtcaaagaacctctgggtccatgggtagacaaccaggagcctgtgagattgacaagaacagtttgacagtcagaaggtgccacaaatcctgagaagcaacctggacttttgccaggcacagggtccttccttccctcccttgtcctggtcaccagagcctaccttcccagggtttctcctccagcatcttccacattcaccttgtcccacaggcttgtgatagtagccttgtcctcctctgtgaaatgacccatggtgtctgtttgaggttgctagtgaacacagttgtgtcagaagcaaatgtaagcaatagatggctctgccctgacttttatgcccagccctggctcctgccctccctgctcctgggagtagattggccaaccctagggtgtggctccacagggtgaggtctaagtgatgacagccgtacctgtccttggctcttctggcactggcttaggagttggacttcaaaccctcagccctccctctaagatatatctcttggccccataccatcagtacaaattgctactaaaaacatcctcctttgcaagtgtatttacgacggtatcgatgtatgtgagcatgtgtcctctaacagcacaggccttttgccacctagctgtccaggggtgccttaaaatggcaaacaaggtttgttttcttttcctgttttcatgccttcctcttccatatccttgtttcatattaatacatgtgtatagatcctaaaaatctatacacatgtattaataaagcctgattctgccgcttctaggtatagaggccacctgcaagataaatatttgattcacaataactaatcattctatggcaattgataacaacaaatatatatatatatatatatatacgtatatgtgtatatatatatatatatatatatattcaggaaataatatattctagaatatgtcacattctgtctcaggcatccattttctttatgatgccgtttgaggtggagttttagtcaggtggtcagcttctccttttttttgccatctgccctgtaagcatcctgctggggacccagataggagtcatcactctaggctgagaacatctgggcacacaccctaagcctcagcatgactcatcatgactcagcattgctgtgcttgagccagaaggtttgcttagaaggttacacagaaccagaaggcgggggtggggcactgaccccgacaggggcctggccagaactgctcatgcttggactatgggaggtcactaatggagacacacagaaatgtaacaggaactaagggaattccggtgccctgcttaggagcttaatctttaatgaaagctaagctttcattaaaaaaagtctaaccagctgcattcgactttgactgcagcagctggttagaaggttctactggaggagggtcccagcccattgctaaattaacatcaggctctgagactggcagtatatctctaacagtggttgatgctatcttctggaacttgcctgctacattgagaccactgacccatacataggaagcccatagctctgtcctgaactgttaggccactggtccagagagtgtgcatctcctttgatcctcataataaccctatgagatagacacaattattactcttactttatagatgatgatcctgaaaacataggagtcaaggcacttgcccctagctgggggtataggggagcagtcccatgtagtagtagaatgaaaaatgctgctatgctgtgcctcccccacctttcccatgtctgccctctactcatggtctatctctcctggctcctgggagtcatggactccacccagcaccaccaacctgacctaaccacctatctgagcctgccagcctataacccatctgggccctgatagctggtggccagccctgaccccaccccaccctccctggaacctctgatagacacatctggcacaccagctcgcaaagtcaccgtgagggtcttgtgtttgctgagtcaaaattccttgaaatccaagtccttagagactcctgctcccaaatttacagtcatagacttcttcatggctgtctcctttatccacagaatgattcctttgcttcattgccccatccatctgatcctcctcatcagtgcagcacagggcccatgagcagtagctgcagagtctcacataggtctggcactgcctctgacatgtccgaccttaggcaaatgcttgactcttctgagctcggatcccttgagctcaggaggtcaaggctgcagtgagacatgatcttgccactgcactccagcctggacagcagagtgaaaccttgcctcacgaaacagaatacaaaaacaaacaaacaaaaaactgctccgcaatgcgcttccttgatgctctaccacataggtctgggtactttgtacacattatctcattgctgttcataattgttagattaattttgtaatattgatattattcctagaaagctgaggcctcaagatgataacttttattttctggacttgtaatagctttctcttgtattcaccatgttgtaactttcttagagtagtaacaatataaagttattgtgagtttttgcaaacacagcaaacacaacgacccatatagacattgatgtgaaattgtctattgtcaatttatgggaaaacaagtatgtactttttctactaagccattgaaacaggaataacagaacaagattgaaagaatacattttccgaaattacttgagtattatacaaagacaagcacgtggacctgggaggagggttattgtccatgactggtgtgtggagacaaatgcaggtttataatagatgggatggcatctagcgcaatgactttgccatcacttttagagagctcttgggggccccagtacacaagaggggacgcagggtatatgtagacatctcattctttttcttagtgtgagaataagaatagccatgacctgagtttatagacaatgagcccttttctctctcccactcagcagctatgagatggcttgccctgcctctctactaggctgactcactccaaggcccagcaatgggcagggctctgtcagggctttgatagcactatctgcagagccagggccgagaaggggtggactccagagactctccctcccattcccgagcagggtttgcttatttatgcatttaaatgatatatttattttaaaagaaataacaggagactgcccagccctggctgtgacatggaaactatgtagaatattttgggttccatttttttttccttctttcagttagaggaaaaggggctcactgcacatacactagacagaaagtcaggagctttgaatccaagcctgatcatttccatgtcatactgagaaagtccccacccttctctgagcctcagtttctctttttataagtaggagtctggagtaaatgatttccaatggctctcatttcaatacaaaatttccgtttattaaatgcatgagcttctgttactccaagactgagaaggaaattgaacctgagactcattgactggcaagatgtccccagaggctctcattcagcaataaaattctcaccttcacccaggcccactgagtgtcagatttgcatgcggat

SEQ ID NO: 51 - DNA, 100 bp, Artificial Sequence
  Synthetic: Exon 1 (HBG17101-7152; sGbGm reverse strand 1735-1834)
cttcccagggtttctcctccagcatcttccacattcaccttgtcccacaggcttgtgatagtagccttgtcctcctctgtgaaatgacccatggtgtctg

SEQ ID NO: 52 - DNA, 223 bp, Artificial Sequence
  Synthetic: Exon 2 (HBG17323-7545; sGbGm reverse strand 1612-1320)
cttgaagttctcaggatccacatgcagcttgtcacagtgcagttcactcagctgggcaaaggtgcccttgagatcatccaggtgctttatggcatctcccaaggaagtcagcaccttcttgccatgtgccttgactttggggttgcccatgatggcagaggcagaggacaggttgccaaagctgtcaaagaacctctgggtccatgggtagacaaccaggagc

SEQ ID NO: 53 - DNA, 216 bp, Artificial Sequence
  Synthetic: Exon 3 (HBG1 8412-8627; sGbGm reverse strand 698-913)
gtgatctctcagcagaatagatttattatttgtattgcttgcagaataaagcctatccttgaaagctctgaatcatgggcaagaggctcagtggtatctggaggacagggcactggccactgcagtcaccatcttctgccaggaagcctgcacctcaggggtgaattctttgccaaagtgaatggccagcacggtgaccagcacgttgcccaggag

SEQ ID NO: 54 - DNA, 303 bp, Artificial Sequence
  Synthetic: 7SK-sh734 Sequence cassette
atcgacgtgcagtatttagcatgccccacccatctgcaaggcattctggatagtgtcaaaacagccggaaatcaagtccgtttatctcaaactttagcattttgggaataaatgatatttgctatgctggttaaattagattttagttaaatttcctgctgaagctctagtacgataagtaacttgacctaagtgtaaagttgagatttccttcaggtttatatagcttgtgcgccgcctgggtacctcaggatatgcccttgactatttgtccgacatagtcaagggcatatccttttttgt

SEQ ID NO: 55 - DNA, 539 bp, Artificial Sequence
  Synthetic: sGbGm A gamma-globin sequence 5-3 complementary strand
cagacaccatgggtcatttcacagaggaggacaaggctactatcacaagcctgtgggacaaggtgaatgtggaagatgctggaggagaaaccctgggaaggctcctggttgtctacccatggacccagaggttctttgacagctttggcaacctgtcctctgcctctgccatcatgggcaaccccaaagtcaaggcacatggcaagaaggtgctgacttccttgggagatgccataaagcacctggatgatctcaagggcacctttgcccagctgagtgaactgcactgtgacaagctgcatgtggatcctgagaacttcaagctcctgggcaacgtgctggtcaccgtgctggccattcactttggcaaagaattcacccctgaggtgcaggcttcctggcagaagatggtgactgcagtggccagtgccctgtcctccagataccactgagcctcttgcccatgattcagagctttcaaggataggctttattctgcaagcaatacaaataataaatctattctgctgagagatcac

SEQ ID NO: 56 - DNA, 769 bp, Artificial Sequence
  Synthetic: REV response element (RRE)
aggaggagatatgagggacaattggagaagtgaattatataaatataaagtagtaaaaattgaaccattaggagtagcacccaccaaggcaaagagaagagtggtgcagagagaaaaaagagcagtgggaataggagctttgttccttgggttcttgggagcagcaggaagcactatgggcgcagcgtcaatgacgctgacggtacaggccagacaattattgtctggtatagtgcagcagcagaacaatttgctgagggctattgaggcgcaacagcatctgttgcaactcacagtctggggcatcaagcagctccaggcaagaatcctggctgtggaaagatacctaaaggatcaacagctcctggggatttggggttgctctggaaaactcatttgcaccactgctgtgccttggaatgctagttggagtaataaatctctggaacagatttggaatcacacgacctggatggagtgggacagagaaattaacaattacacaagcttaatacactccttaattgaagaatcgcaaaaccagcaagaaaagaatgaacaagaattattggaattagataaatgggcaagtttgtggaattggtttaacataacaaattggctgtggtatataaaattattcataatgatagtaggaggcttggtaggtttaagaatagtttttgctgtactttctatagtgaatagagttaggcagggatattcaccattatcgtttcagacccacctcccaaccccgaggggaccg

SEQ ID NO: 57 - DNA, 3055 bp, Artificial Sequence
  Synthetic: Locus Control Region
gtatgtgagcatgtgtcctctaacagcacaggccttttgccacctagctgtccaggggtgccttaaaatggcaaacaaggtttgttttcttttcctgttttcatgccttcctcttccatatccttgtttcatattaatacatgtgtatagatcctaaaaatctatacacatgtattaataaagcctgattctgccgcttctaggtatagaggccacctgcaagataaatatttgattcacaataactaatcattctatggcaattgataacaacaaatatatatatatatatatatatacgtatatgtgtatatatatatatatattcaggaaataatatattctagaatatgtcacattctgtctcaggcatccattttctttatgatgccgtttgaggtggagttttagtcaggtggtcagcttctccttttttttgccatctgccctgtaagcatcctgctggggacccagataggagtcatcactctaggctgagaacatctgggcacacaccctaagcctcagcatgactcatcatgactcagcattgctgtgcttgagccagaaggtttgcttagaaggttacacagaaccagaaggcgggggtggggcactgaccccgacaggggcctggccagaactgctcatgcttggactatgggaggtcactaatggagacacacagaaatgtaacaggaactaagggaattccggtgccctgcttaggagcttaatctttaatgaaagctaagctttcattaaaaaaagtctaaccagctgcattcgactttgactgcagcagctggttagaaggttctactggaggagggtcccagcccattgctaaattaacatcaggctctgagactggcagtatatctctaacagtggttgatgctatcttctggaacttgcctgctacattgagaccactgacccatacataggaagcccatagctctgtcctgaactgttaggccactggtccagagagtgtgcatctcctttgatcctcataataaccctatgagatagacacaattattactcttactttatagatgatgatcctgaaaacataggagtcaaggcacttgcccctagctgggggtataggggagcagtcccatgtagtagtagaatgaaaaatgctgctatgctgtgcctcccccacctttcccatgtctgccctctactcatggtctatctctcctggctcctgggagtcatggactccacccagcaccaccaacctgacctaaccacctatctgagcctgccagcctataacccatctgggccctgatagctggtggccagccctgaccccaccccaccctccctggaacctctgatagacacatctggcacaccagctcgcaaagtcaccgtgagggtcttgtgtttgctgagtcaaaattccttgaaatccaagtccttagagactcctgctcccaaatttacagtcatagacttcttcatggctgtctcctttatccacagaatgattcctttgcttcattgccccatccatctgatcctcctcatcagtgcagcacagggcccatgagcagtagctgcagagtctcacataggtctggcactgcctctgacatgtccgaccttaggcaaatgcttgactcttctgagctcggatcccttgagctcaggaggtcaaggctgcagtgagacatgatcttgccactgcactccagcctggacagcagagtgaaaccttgcctcacgaaacagaatacaaaaacaaacaaacaaaaaactgctccgcaatgcgcttccttgatgctctaccacataggtctgggtactttgtacacattatctcattgctgttcataattgttagattaattttgtaatattgatattattcctagaaagctgaggcctcaagatgataacttttattttctggacttgtaatagctttctcttgtattcaccatgttgtaactttcttagagtagtaacaatataaagttattgtgagtttttgcaaacacagcaaacacaacgacccatatagacattgatgtgaaattgtctattgtcaatttatgggaaaacaagtatgtactttttctactaagccattgaaacaggaataacagaacaagattgaaagaatacattttccgaaattacttgagtattatacaaagacaagcacgtggacctgggaggagggttattgtccatgactggtgtgtggagacaaatgcaggtttataatagatgggatggcatctagcgcaatgactttgccatcacttttagagagctcttgggggccccagtacacaagaggggacgcagggtatatgtagacatctcattctttttcttagtgtgagaataagaatagccatgacctgagtttatagacaatgagcccttttctctctcccactcagcagctatgagatggcttgccctgcctctctactaggctgactcactccaaggcccagcaatgggcagggctctgtcagggctttgatagcactatctgcagagccagggccgagaaggggtggactccagagactctccctcccattcccgagcagggtttgcttatttatgcatttaaatgatatatttattttaaaagaaataacaggagactgcccagccctggctgtgacatggaaactatgtagaatattttgggttccatttttttttccttctttcagttagaggaaaaggggctcactgcacatacactagacagaaagtcaggagctttgaatccaagcctgatcatttccatgtcatactgagaaagtccccacccttctctgagcctcagtttctctttttataagtaggagtctggagtaaatgatttccaatggctctcatttcaatacaaaatttccgtttattaaatgcatgagcttccgttactccaagactgagaaggaaattgaacctgagactcattgactggcaagatgtccccagaggctctcattcagcaataaaattctcaccttcacccaggcccactagtgtcagatttgcatgc

SEQ ID NO: 58 - DNA, 43 bp, Artificial Sequence
  Synthetic: Agosh 734 5-3
atagtcaagggcatatcctcaagaaggatatgcccttgactac

SEQ ID NO: 59 - DNA, 1435 bp, Homo sapiens
  misc_feature: Homo sapiens hypoxanthine phosphoribosyltransferase 1 (HPRT1), mRNA
ggcggggcctgcttctcctcagcttcaggcggctgcgacgagccctcaggcgaacctctcggctttcccgcgcggcgccgcctcttgctgcgcctccgcctcctcctctgctccgccaccggcttcctcctcctgagcagtcagcccgcgcgccggccggctccgttatggcgacccgcagccctggcgtcgtgattagtgatgatgaaccaggttatgaccttgatttattttgcatacctaatcattatgctgaggatttggaaagggtgtttattcctcatggactaattatggacaggactgaacgtcttgctcgagatgtgatgaaggagatgggaggccatcacattgtagccctctgtgtgctcaaggggggctataaattctttgctgacctgctggattacatcaaagcactgaatagaaatagtgatagatccattcctatgactgtagattttatcagactgaagagctattgtaatgaccagtcaacaggggacataaaagtaattggtggagatgatctctcaactttaactggaaagaatgtcttgattgtggaagatataattgacactggcaaaacaatgcagactttgctttccttggtcaggcagtataatccaaagatggtcaaggtcgcaagcttgctggtgaaaaggaccccacgaagtgttggatataagccagactttgttggatttgaaattccagacaagtttgttgtaggatatgcccttgactataatgaatacttcagggatttgaatcatgtttgtgtcattagtgaaactggaaaagcaaaatacaaagcctaagatgagagttcaagttgagtttggaaacatctggagtcctattgacatcgccagtaaaattatcaatgttctagttctgtggccatctgcttagtagagctttttgcatgtatcttctaagaattttatctgttttgtactttagaaatgtcagttgctgcattcctaaactgtttatttgcactatgagcctatagactatcagttccctttgggcggattgttgtttaacttgtaaatgaaaaaattctcttaaaccacagcactattgagtgaaacattgaactcatatctgtaagaaataaagagaagatatattagttttttaattggtattttaatttttatatatgcaggaaagaatagaagtgattgaatattgttaattataccaccgtgtgttagaaaagtaagaagcagtcaattttcacatcaaagacagcatctaagaagttttgttctgtcctggaattattttagtagtgtttcagtaatgttgactgtattttccaacttgttcaaattattaccagtgaatctttgtcagcagttcccttttaaatgcaaatcaataaattcccaaaaatttaaaaaaaaaaaaaaaaaaaaaa

SEQ ID NO: 60 - DNA, 42 bp, Artificial Sequence
  Synthetic: miRNA 451 hairpin sequence
aaaccgttaccattactgagtttagtaatggtaatggttctc

SEQ ID NO: 61 - DNA, 23 bp, Artificial Sequence
  Synthetic: sgRNA candidate for knock down of human HPRT
gttatggcgacccgcagccctgg

SEQ ID NO: 62 - DNA, 212 bp, Artificial Sequence
  Synthetic: left homology arm from target CCR5 gene region
gcttcttctctggaatcttcttcatcatcctcctgacaatcgataggtacctggctgtcgtccatgctgtgtttgctttaaaagccaggacggtcacctttggggtggtgacaagtgtgatcacttgggtggtggctgtgtttgcgtctcaagcttttcgaagcggccgcggatatcggctccggtgcccgtcagtgggcagagcgcacatc

SEQ ID NO: 63 - DNA, 221 bp, Artificial Sequence
  Synthetic: left homology arm from target CCR5 gene region
aaagcatttttttcactgcattctagttgtggtttgtccaaactcatcaatgtatcttatcatctacgcgtccaggaatcatctttaccagatctcaaaaagaaggtcttcattacacctgcagctctcattttccatacagtcagtatcaattctggaagaatttccagacattaaagatagtcatcttggggctggtcctgccgctgcttgtcatggtc

SEQ ID NO: 64 - DNA, 238 bp, Artificial Sequence
  Synthetic: EF1a promoter
ggatatcggctccggtgcccgtcagtgggcagagcgcacatcgcccacagtccccgagaagttggggggaggggtcggcaattgaaccggtgcctagagaaggtggcgcggggtaaactgggaaagtgatgtcgtgtactggctccgcctttttcccgagggtgggggagaaccgtatataagtgcagtagtcgccgtgaacgttcttttcgcaacgggtttgccgccagaacacagg

SEQ ID NO: 65 - DNA, 128 bp, Artificial Sequence
  Synthetic: SV40 promoter
aacttgtttattgcagcttataatggttacaaataaagcaatagcatcacaaatttcacaaataaagcatttttttcactgcattctagttgtggtttgtccaaactcatcaatgtatcttatcatct

SEQ ID NO: 66 - DNA, 87 bp, Artificial Sequence
  Synthetic: Beta globin promoter
ggtgtctgtttgaggttgctagtgaacacagttgtgtcagaagcaaatgtaagcaatagatggctctgccctgacttttatgcccag

SEQ ID NO: 67 - DNA, 111 bp, Artificial Sequence
  Synthetic: miRNA734 de novo (DNA form)
acccgtacatatttttgtgtagctctagtttatagtcaagggcatatccttgtgttttttttgaaggatatgcccttgactataaactagcgctacactttttcgtcttgt

SEQ ID NO: 68 - DNA, 111 bp, Artificial Sequence
  Synthetic: miRNA211 de novo (DNA form)
acccgtacatatttttgtgtagctctagttataaatcaaggtcataaccttgtgttttttttgaaggttatgaccttgatttataactagcgctacactttttcgtcttgt

SEQ ID NO: 69 - DNA, 23 bp, Artificial Sequence
  Synthetic: sgRNA candidate for knock down of human HPRT
gcgggtcgccataacggagccgg